European Patent Application EP 4 144 752 A1, published March 8, 2023. Title: VIRAL-LIKE PARTICLES FOR THE TREATMENT OR PREVENTION OF AN INFECTION BY A CORONAVIRIDAE VIRUS. Applicant: SORBONNE UNIVERSITE INSTITUT NATIONAL DE LA SANTE ET DE LA RECHERCHE MEDICALE ASSISTANCE PUBLIQUE - HOPITAUX DE PARIS CONSEJO NACIONAL DE INVESTIGACIONES CIENTIFICAS Y TECNICAS (CONICET) UNIVERSIDAD CATOLICA DE CORDOBA (UCC). The sequence listing filed with the application follows.

SEQUENCE LISTING (133 sequences)

SEQ ID NO: 1 - protein, 596 aa, Giardia
MLLIAFYLILSTFAVDCKNSGNSCEAGQCDTIGDTEICMQCNQGKVPINGICTAHSEEAVTNAGCKKNGGTNIEESDKVCGQCGNGYFLHKGGCYKIGEAPGNLICADEASNPGARTAGVCGACKDGYYKNSDAVATADSCIACEDANCATCGGAGENKCTKCIDGYFVGATGNEGGCIKCDATTGPNSYKGVAGCAKCEKPKNAGPAKCIECAADYLKTEADEQTSCVSEAVCREGKTHFPTTDSAGGNKKVCVSCGTTNNGGIENCGECTSKESAARAGTEITCTKCSSNNLSPLGDACLTDCPAGTYAVSGDSGSVCKPCHNTCAGCQTDDRETSCTACYPGYSLLYESNGATGRCVKECTGAFITNCADGQCTANVGGAKYCTQCKDGYAPIDGICTAVAAAGRDVSVCTATGGKCTACTGNYALLSGGCYNTQTLPGKSVCKAVANSNDGKCKTCANGQAPDPATNFCPLCDSTCAECSTKNDADACTKCFPGYYKTGNKCIKCTESSNNGKKIDGIPDCLSCEAPINTGPVICYVKTDGTSDDNSGNGGDSTNKSGLSTGAIAGISVAAFVVVAGLVGFLCWWFICRGKA

SEQ ID NO: 2 - protein, 713 aa, Giardia
MFGRFLLAIVILQLARTACTQEADDGKCKTCGVTIGQDTWCSECNGANYAPVNGQCVDVNAEGPSKTLCPQHSAGKCTQCGGNSFMYKDGCYSSGEGLPGHSLCLSSDGDGVCTEAAPGYFAPVGAANTEQSVIACGDTTGVTIAAGGNTYKGIADCAECSAPDATAGAEAGKVATCTKCGVSKYLKDNVCVDKAQCNSGSTNKFVAVDDSENGNKCVSCSDNLNGGVANCDTCSYDEQSKKIKCTKCTDNNYLKTTSEGTSCVQKDQCKDGFFPKDDSSAGNKCLPCNDSTDGIANCATCALVSGRSGAALVTCSACTDGYKPSADKTTCEAVSNCKTPGCKACSNEGKENEVCTDCDGSTYLTPTSQCIDSCAKIGNYYGATEGAKKLCKECTAANCKTCDDQGQCQACNDGFYKNGDACSPCHESCKTCSAGTASDCTECPTGKALRYGDDGTKGTCGEGCTTGTGAGACKTCGLTIDGASYCSECATTTEYPQNGVCAPKASRATPTCNDSPIQNGVCGTCADNYFKMNGGCYETVKYPGKTVCISAPNGGTCQKAADGYKLDSGTLTVCSEGCKECASSTDCTTCLDGYVKSASACTKCDASCETCNGAATTCKACATGYYKTASGEGACTSCESDSNGVTGIKGCLNCAPPPNNKGSVLCYLIKDSGSTNKSGLSTGAIAGISVAVIVVVGGLIGFLCWWFLCRGKA

SEQ ID NO: 3 - protein, 739 aa, Giardia
MFGSFVLAGVLVQIAWAGKATERAQEAQCADNTNCAAEACNVLIGGKLYCSRCNTGFVPINGQCADKEGATDKCKDGSGGDTADQTCGQCAEQTFMYKGGCYEAAQQPGQTMCQAADAGVCTQAAQGYFVPPGADASHQSVIPCGDEEEITVKNDKKYKGVLHCTRCNAPTEAADANAKAATCTACQADRYLKTAKDQATSCVTEQECTGTEGFFAKNGGTKTCEACAETCKTCKTEAAKCTSCKDDKPYLKKDNGSDTGTCVTEAECKTGNTHYPDDTEPKTCKTCAEGTSDGCATCEKGADGAVACKTCGNQKKVQPNKKGCVENCPSNSNDKKTPGTCECVEGYVPEEAGTGCTKKPDPPAAPCNTPGCKTCSEPKTSKEVCTECEDPKALTPTGQCIYGCEHLEGYYEGTSEGGKKACKKCEVENCLLCNENGQCETCKDGYYKKETACAKCDTSCKTCANGEPNGCTSCEAKKALSYEGEGNTGTCKSECKPGTNNCEKCELTVDGTAYCSKCKDANQFPQNGVCSAAAGKAITCTTKGTGVCDKCANGLLRMNGGCYETTKFPGKSVCEEAASAGDTCQVEAPGYHLNNNDLVTCSAGCKTCTSNTVCTECMDGYAKTDNKCTKCATGCATCAGSASNCDTCSTGYYKYKNACVSCTESNSDKTITGVANCANCAPPLNNKGSVLCYLVQSGENTNKSGLSAGAIAGIAVAVIIVVGGLVGFLCWWFMCRGKA

SEQ ID NO: 4 - protein, 617 aa, Giardia
MFEKIIFGIAILQVVWAATTCTEASSDPQTGQCATGKCDVWIGGSNFCSQCSTAAEHLVNGKCITTGEDAEGACTTKNDGTCTSCKAGFFLHRGGCYEMGSDIGLLVCNDRTATADKDGICIACHDGYFKNPASDADKTKESCIACNNTAGVDHNKGVQNCATCDAPKTPGQSSAEQTATCKSCVDGYYGTTSCQQCHADCRTCTGNGEDKCTSCKDTGKQYFKEGANSDGTGTCVDENGCGNTHFPIAEDKKCHLCGSVSEGGVADCKTCSKTGDSVKCLTCEGTKKPNEAGTGCFVCPMEHCEKCSKDNVCEACGSEKKLSPLGDACLDACPAGTRTDANVCNLCHESCASCSTNAETSCTACYPGYVLKRDETNAKGTCIKECTGDFMAHCKADGCSLNVGGSKYCDQCEEGYAPVDGVCTSIPATARDASGCKASGGKCTECGANYALLSGGCYNTQKLPGSSVCTAAQNKGQCQTCANGQSPAGGKCPACTEGCVKCAGSKETCTDCLAGYYKGAGDKCFKCTDSDKASSNAITGVENCISCAPPAGGNGPVTCYVTQQKADDGTGGDTGGDSTNRSGLSTGAIAGISVAVIVVVGGLVGFLCWWFICRGKA

SEQ ID NO: 5 - protein, 681 aa, Giardia
MLLTAFYIVVSSFAAPCQQDGDHIVTCQVNKCETVGSAEICTECKVGGVPVDGFCRPFGSIQAAAAGCTKADGAALDKMTATCEKCGDGYFLFMGGCYKTSLWSEVCTAASNGVCTTCNTKNGLFKNPAATVTPGNECILCSDATDRNGVMGVENCLKCTAPGGNTGAAACTACKAGFYGSGPCTKCHDDCATCSGAANNQCTSCKAGKYLKTDTNTCVDAGSCNGNTYADPVTRTCKDSAITDCTTCEYNPATGGPKCTACGNSKKVKTAIDGATTCVTVASECVDENHFKDDGNTMCVLCSDTSGSDPNKGVAQCKTCTKNGANKPECKTCLEGYVLKGSGADAICESCGNNCAVCTAANDISTCTGCLPGYFLKAEGGTKECVPCDDTAKGGREGCSLCSSNGGFKCTDCKANYRKQSNGDAGDDYTCVKTCEDPTVCGGTSGACDAIVIDANGKEHYYCSYCGETNKFPIDGLCTDNKGTNAGCTDHTCSYCAAGFFLYMGGCYKIDTVPGSYMCSKSTTAGVCDTPNANNRFFVVPKAISAEQSVLACGNPLGTIAGGNAYVGVEGCSQCTAPDARADGGMAVATCTACEDGKKPGKSGTGCVACPDANCKSCTMDDVCEECADGFSLDNGKCVSSGTNKSGLSTGAIAGISVAAIVVVGGLVGFLCWWFICRGKA

SEQ ID NO: 6 - protein, 547 aa, Giardia
MFYAFLLTGLALELVRAAQAGDECEEVASSEPNTCKACSAVVNGKKYCSQCNGGGSQSAPTDGVCSADNNECTRKQDGKCTQCANKSFMYKGGCYKDSQAPGNTMCETANAGVCTQAKEGYFLPPGTDNAHDSVVSCGDTTGVTLTGDKKYTGVAECVTCTQPGQLSIGGTKAAICTKCAADLYLKIDRGVMECVAESGCGEGFFPTIVDGVKKCAGCSEAGSGGIEDCELCIPRAPAPEAGVKVTCSKCHASKKVSPLKDECMDNCPAGTYDKQNVCTPCHSSCASCQTDDKETSCTACYPGHSLLYEANGATGRCVKECTGAFITNCADGQCTADVGGAKYCAQCKEGYAPIDGVCTAVKIGRDASVCTAASGKCTACTGAYALISGGCYGVAKLPGKAVCTAANNGECTTCANGQQPSGKVCPTCPAGCSKCTGSAPSQQCSECFPGYYKSGTKCVACDKDDGSIKGVPNCLSCKEPASSSGAVTCYLTQQKTDDGTGGDTGGDSMNKSGLSTGAIAGISVAAIVVVGGLIGFLCWWFICRGKA

SEQ ID NO: 7 - protein, 689 aa, Giardia
MLLTAFYIVLGSFAAPCQQDGDHIVTCQVNKCETVGSAEICTECKVGGVPVDGFCRPFGSIQAAAAGCTKADGAALDKMTATCEKCGDGYFLFMGGCYKTTDGPGSEICTKAEGGLCTECKTANGLFKNPATPQKPGSECILCHDATNRNGVMGVDNCLKCTAPGGNTGAATCTECMAGTYKKSDTECAACHSDCATCSGANQNQCTSCETGKYLKGTECVDKGTCNNNHYPDDTSMTCVACTVLDANCATCSFDSATAKGKCLTCNSNKIPRTTLDGTSTCVENSYAGCQGADNELFMKEDQSACLLCGDTKDVDNNNKGKEGCKTCTKSADGSPPTCTACLDGYFFEQSSNTCEACGANCVTCSAKTDETKCKTCKEGFFLAGTGEGKCISCENGNDSGYSGLAGCLSCTAPAAPGPASCNRCKIGYKLQGTTCVKTCEDTTACGGTSGACDAIVIDDKGNTKHYCSYCGDSGKFPIDGICTDSKGTNAGCTDHICSYCAQGYFLYMGGCYSTASPPGNYMCKTAEGGKCTAVNDGNRYFIVPEAKATDQSVLACSNPLGTLVGTDSAAKAYVGVLNCSQCKAPAALTEAGMTAAVCTSCDSGKKPNRDGSGCVTCSVGDCKSCVMDDVCGECSDGYSLEGGKCVSSGSNRSGLSTGAIAGISVAVIVVVGGLIGFLCWWFICRGKA

SEQ ID NO: 8 - protein, 732 aa, Giardia
MFGSFVLAGVLVQIAWAEKVAERAAQCADNTNCAAEACNVLIDGKLYCSKCKTELVGHAPVNGVCADVSSSKEICKINAEGKCTECAGQSFMYKGGCYQTSQAPGSSMCQAADAGKCTTAPESKAYFVVPEVDRKPTGQTVVSCGDATGVTLADKTYKGVDGCTKCEAPAPADASGAKAATCTACQADKYLKTTTDSATSCVTEKECTDAAGFFVDTTGGKKCSKCDPGCKTCKTEAAKCTSCKDDKPYLKKDAGDTGTCVTEADCKNGNTHYADDTEPKTCKTCAEGTSDGCATCEKSADGAVACKTCGNQKKVQPNKKGCIAKCPETVSAEKDGVCECVEGYVPDNAGTGCTKKSDPQCNTPGCKTCSEPKTSKEVCTECEDAKALTPTGQCIDNCGDLGGYYAGTNEGGKKACKKCEVENCLLCNGQGQCETCKDGYYKSGAACAKCDTSCKTCANGNSNGCTSCESSKALSYEGEGTGTCKPGCEPNANNCEKCELTVDGTAYCSKCKDASQFPQNGVCSAAAGKAITCTTQRDGVCNKCANGFLRMNGGCYETTKFPGKSVCKEVLQNGDTCQTLADGYKLDNGALTTCSAGCKTCTSNTVCTECMYGYAKTNNECKVCTTGCATCAGSTSNCDICSTGYYKSGSTCVSCTANTADGTITGVANCANCAPPLNDKGSVLCYLVQSGENTNKSGLSAGAIAGISVAVIIVVGGLVGFLCWWFMCRGKA

SEQ ID NO: 9 - protein, 681 aa, Giardia
MFQLIPLFMASALMAPCQPDGNHLTTCAHEKCETVGSAEICTECKVGGVPVDGFCRPFGSIQAAAAGCTKADGAALDKMTATCEKCGDGYFLFMGGCYKTSLWSEVCTAASNGVCTTCNTKNGLFKNPAATVTPGNECILCSDATDRNGVMGVENCLKCTAPGGNTGAAACTACKAGFYGSGPCTKCHDDCATCSGAANNQCTSCKAGKYLKTDTNTCVDAGSCNGNTYADPVTRTCKDSAITDCTTCEYNPATGGPKCTACGNSKKVKTAIDGATTCVTVASECVDENHFKDDGNTMCVLCSDTSGSDPNKGVAQCKTCTKNGANKPECKTCLEGYVLKGSGADAICESCGNNCAVCTAANDISTCTGCLPGYFLKAEGGTKECVPCDDTAKGGREGCSLCSSNGGFKCTDCKANYRKQSNGDAGDDYTCVKTCEDPTVCGGTSGACDAIVIDANGKEHYYCSYCGETNKFPIDGLCTDNKGTNAGCTDHTCSYCAAGFFLYMGGCYKIDTVPGSYMCSKSTTAGVCDTPNANNRFFVVPKAISAEQSVLACGNPLGTIAGGNAYVGVEGCSQCTAPDARADGGMAVATCTACEDGKKPGKSGTGCVACPDANCKSCTMDDVCEECADGFSLDNGKCVSSGTNKSGLSTGAIAGISVAAIVVVGGLVGFLCWWFICRGKA

SEQ ID NO: 10 - protein, 540 aa, Giardia
MFYAFLLTGLALELVRAAQAGDECEEVASSEPNTCKACSAVVNGKKYCSQCNGGGSQSAPTDGVCSADNNECTRKQDGKCTQCANKSFMYKGGCYKDSQAPGNTMCETANAGVCTQAKEGYFLPPGTDNAHDSVVSCGDTTGVTLTGDKKYTGVAECVTCTQPGQLSIGGTKAAICTKCAADLYLKIDRGVMECVAESGCGEGFFPTIVDGVKKCAGCSEAGSGGIEDCELCIPRAPAPEAGVKVTCSKCHASKKVSPLKDECMDNCPAGTYDKQNVCTPCHSSCASCQTDDKETSCTACYPGHSLLYEANGATGRCVKECTGAFITNCADGQCTADVGGAKYCAQCKEGYAPIDGVCTAVKIGRDASVCTAASGKCTACTGAYALISGGCYGVAKLPGKAVCTAANNGECTTCANGQQPSGKVCPTCPAGCSKCTGSAPSQQCSECFPGYYKSGTKCVACDKDDGSIKGVPNCLSCKEPASSSGAVTCYVKTDGTNNGGSMNKSGLSTGAIAGISVAVIAVVGGLVGFLCWWFICRGKA

SEQ ID NO: 11 - protein, 529 aa, Giardia
MLVGIGLIFAVALADACSPSIDGCAECDSTGKKCTKCDPNDPSNKKYLKDGACVTDAECTGAHDHYADSTDPTALVCKACGKNEKPNTAGNACFVCPDPNCRRCNEANKCADCATGKPQADGTCPAATPGCHSSCKECVSGANTSEDDKCLSCSGDNYLKVTNAAARSGVCVSASACTSDKTHFAKEVTDSNGSKKMCLSCSDATHGIADCKKCSSTASSAQTELALVCSDCGIKWLSPLGNACLEKCPAGTYSDRSADGISVCASCHSTCAECNGNAEATSCTACYPGSVLSKGNGGATGTCIPECTGRYAENCEAGQCTAVVGGSKYCSKCKAGFAPVDGVCVPITQRTIAGCNPGQDGTCTSCKDAYFKESGGCYQSTTYPGDKLCTTASQGKCTTCANGQAADNQGSCPACPDGCSKCTAGSSPQQCSECFPGYYLDAGKGCKKCSETSGNIQGIPNCVSCAPPTGGNGGPVTCYIKTDGANNGGSTNKSGLSTGAIAGISVAAIVVVGGLVGFLCWWFICRGKA

SEQ ID NO: 12 - protein, 687 aa, Giardia
MLLKITLTLAIALSACQEGTEATKCKTGKCIDIGGTQYCSECAVSTEAPVNGQCADASSNTAICKAHAGGKCTECDGDSFMYKGGCYETTNEPGQSMCKSTNNAGVCTAPNDSGKYFVPPDTDASHQSIVACGDTSGMRYQPDDSTDKAYNGVAGCETCTAPQQITDNTGTATATCTKCASNNIVKTDADETTCIAESECPTTKGFFVEDPGSGNQKKCTTCSPNCLSCTSAAEAACKSCTVETHFLGAEDGQVGKCVSCGDAATGSGDWKGVTGCAKCAKPEAAGAATCTECASDYLKTEAGATSCVERNRCTGGFFPNDDVDGKKQCVPCGDAAHKGIPNCRTCTESGGAVTCDACTEGNTPTTDKTACIPCSVDGCDSCNEENVCAKCATDKYLTSTGQCVDDCEALEGYYSDKSTNKCEKCSPACKMCTKTADQCSSCPAKKVLQYSSESNLDYGGSCVDECKAGMNGCAECGATIGEAKYCSKCSDAKQAPLNGNCTVSARAAASCKRVEEGACKECETGYFLLEGGCYQTTRQPGMQVCKTANGGSCQTCANELAASSGDCSTQTCHPSCKTCSAANDASKCKVCAAGYYKQSDENTAGKCDPCSQGNDKCTLCRYSTKFICLAKDSSDGDGTDTKPVDPPSSNKSGLSTGAIAGISVAAIVVVGGLVGFLCWWFICRGKA

SEQ ID NO: 13 - protein, 682 aa, Giardia
MLLAIFYFVISTLTAKCTTQTQTCEAEKCEMVGETEICTRCQTGKVPIDGKCVDATANANCKNASGDGDANQVCGKCIGANFFMYKGGCYDKEKVPGNTLCTTVSPDGVCSVAANEYFVPPNADATHDSVVSCSEETPIHLANNKQYIGVAGCATCSAPKAPGEDNTPKAATCTKCAAGFLHTPSEGLSSCEETCPEGYFGHTATAESKKTCKSCTGGSSEAPNVKGIGDCLKCMYNEASGNTLTCEKCSAQKKPSLDKTSCNDCTGQNCAFCSSSGGDCEGCDSGFILDGQNCVKSDCKTENCKACTNPKAANEVCTECISTHHLTPTSQCVQYCQALGNYYAGTNADNKKACKECTVANCKTCNDQGQCQTCNDGFYKNGDACSPCHESCKTCSAGTASDCTECPTGKALKYGNDGTKGTCGEGCTTGQGSGACKTCGLTIDGASYCSECDTQNEYPQNGICTSTTARTVATCKNSNVANGICSSCTNGFLRMNGGCYETTKFPGKSVCEGANADADTCKAPVPGYKVEAGKLVMCSKGCDTCSDATTCTKCGDGYTKIENSQTCTKCDSSCETCTGAATTCKVCATGYYKTALGESTCTSCENDSNGVIGVKGCLNCAPPSSSTGSVLCYLMKGENTGGSVNKSGLSTGAIAGISVAAVVVVAGLVGFLCWWFICRGKA

SEQ ID NO: 14 - protein, 1949 aa, Giardia
MLVGFLLVCVTVLAKHNEKTAQCDDGNGYQLQGDACVKGQANACPTLEGAGCETCDLSGGETCLTCKDKAQYVAANKKSCKAACTAPEEVIDPAAGSAKACKCDDGNGYQLQGDACVKGQANACPTLEGAGCETCDLSGGETCLTCKDKAQYVAANKKSCKAACTAPEEVIDPAAGSAKACKCDDGNGYQLQGDACVKGQANACPTLEGAGCETCDLSGGETCLTCKDKAQYVAANKKSCKAACTAPEEVIDPAAGSAKACKCDDGNGYQLQGDACVKGQANACPTLEGAGCETCDLSGGETCLTCKDKAQYVAANKKSCKAACTAPEEVIDPAAGSAKACKCDDGNGYQLQGDACVQAWTERGRTAAHTSRPGAGPGKRCRPAGGADGRTVATCQDRPGRGGGADGGGETCLTCKDKAQYVAANKKSCKAACTAPEEVIDPAAGSAKACKCDDGNGYQLQGDACVKGQANACPTLEGAGCETCDLSGGETCLTCKDKAQYVAANKKSCKAACTAPEEVIDPAAGSAKACKCDDGNGYQLQGDACVKGQANACPTLEGAGCETCDLSGGETCLTCKDKAQYVAANKKSCKAACTAPEEVIDPAAGSAKACKCDDGNGYQLQGDACVKGQANACPTLEGAGCETCDLSGGETCLTCKDKAQYVAANKKSCKAACTAPEEVIDPAAGSAKACKCDDGNGYQLQGDACVKGQANACPTLEGAGCETCDLSGGETCLTCKDKAQYVAANKKSCKAACTAPEEVIDPAAGSAKACKCDDGNGYQLQGDACVKGQANACPTLEGAGCETCDLSGGETCLTCKDKAQYVAANKKSCKAACTAPEEVIDPAAGSAKACKCDDGNGYQLQGDACVKGQANACPTLEGAGCETCDLSGGETCLTCKDKAQYVAANKKSCKAACTAPEEVIDPAAGSAKACKCDDGNGYQLQGDACVKGQANACPTLEGAGCETCDLSGGETCLTCKDKAQYVAANKKSCKAACTAPEEVIDPAAGSAKACKCDDGNGYQLQGDACVKGQANACPTLEGAGCETCDLSGGETCLTCKDKAQYVAANKKSCKAACTAPEEVIDPAAGSAKACKCDDGNGYQLQGDACVKGQANACPTLEGAGCETCDLSGGETCLTCKDKAQYVAANKKSCKAACTAPEEVIDPAAGSAKACKCDDGNGYQLQGDACVKGQANACPTLEGAGCETCDLSGGETCLTCKDKAQYVAANKKSCKAACTAPEEVIDPAAGSAKACKCDDGNGYQLQGDACVKGQANACPTLEGAGCETCDLSGGETCLTCKDKAQYVAANKKSCKAACTAPEEVIDPAAGSAKACKCDDGNGYQLQGDACVKGQANACPTLEGAGCETCDLSGGETCLTCKDKAQYVAANKKSCKAACTAPEEVIDPAAGSAKACKCDDGNGYQLQGDACVKGQANACPTLEGAGCETCDLSGGETCLTCKDKAQYVAANKKSCKAACTAPEEVIDPAAGSAKACKCDDGNGYQLQGDACVKGQANACPTLEGAGCETCDLSGGETCLTCKDKAQYVAANKKSCKAACTAPEEVIDPAAGSAKACKCDDGNGYQLQGDACVKGQANACPTLEGAGCETCDLSGGETCLTCKDKAQYVAANKKSCKAACTAPEEVIDPAAGSAKACKCDDGNGYQLQGDACVKGQANACPTLEGAGCETCDLSGGETCLTCKDKAQYVAANKKSCKAACTAPEEVIDPAAGSAKACKCDDGNGYQLQGDACVKGQANACPTLEGAGCETCDLSGGETCLTCKDKAQYVAANKKSCKAACTAPEEVIDPAAGSAKACKCDDGNGYQLQGDACVKGQANACPTLEGAGCETCDLSGGETCLTCKDKAQYVAANKKSCKAACTAPEEVIDPAAGSAKACKCDDGNGYQLQGDACVIPNTNKSSGLSTGAIAGIAVAAVIVVGGLVGFLCWWFLCRGKA

SEQ ID NO: 15 - protein, 926 aa, Giardia
MLLLVLCFLMSALAAQCKGHQHSNCATGWCRAVRGVEVCMRCKAGHVLIDGVCADNSVVYGAGSACQILNCKQCNADNTQCEQCEDGYTPSAGNTQCNEDAASACQILNCKQCNADNTQCEQCEDGYTPSAGNTQCNEDAASACQILNCKQCNADNTQCEQCEDGYTPSAGNTQCNEDAASACQILNCKQCNADNTQCEQCEDGYTPSAGNTQCNEDAASACQILNCKQCNADNTQCEQCEDGYTPSAGNTQCNEDAASACQILNCKQCNADNTQCEQCEDGYTPSAGNTQCNEDAASACQILNCKQCNADNTQCEQCEDGYTPSAGNTQCNEDAASACQILNCKQCNADNTQCEQCEDGYTPSAGNTQCNEDAASACQILNCKQCNADNTQCEQCEDGYTPSAGNTQCNEDAASACQILNCKQCNADNTQCEQCEDGYTPSAGNTQCNEDAASACQILNCKQCNADNTQCEQCEDGYTPSAGNTQCNEDAASACQILNCKQCNADNTQCEQCEDGYTPSAGNTQCNEDAASACQILNCKQCNADNTQCEQCEDGYTPSAGNTQCNEDAASACQILNCKQCNADNTQCEQCEDGYTPSAGNTQCNENPEARCNTPNCKTCDNPKTGNEICTKCNDGDYLTPTNQCAHDCTAISGYYGDTDKKCKPCSPECAECVGPANNQCSACPAGKALTYGGGDPAQGGTCGDACTADKNGCKVCGARIGGTDYCSQCSVGTQAPLNGVCTANARAQFCTQVTSGSCTSCSGGYFLKNGGCYQADRQPGKQICTLADSNGGCQACANGLPPSSSDVCPSCHFTCKTCSTADIANTCTTCATGYYMVGSGPNTCISCESDSGSVKGVAGCMSCAPPSSNTGSVLCYLMNGDSAGGSTNKSGLSTGAIAGISVAVIVVVGGLVGFLCWWFICRGKA

SEQ ID NO: 16 - protein, 419 aa, Giardia
MLLLVLCFLMSALAAQCKGHQHSNCATGWCRAVRGVEVCMRCKAGHVLIDGVCADNSVVYGAGSACQILNCKQCNADNTQCEQCEDGYTPSAGNTQCNENPEARCNTPNCKTCDNPKTGNEICTKCNDGDYLTPTNQCAHDCTAISGYYGDTDKKCKPCSPECAECVGPANNQCSACPAGKALTYGGGDPAQGGTCGDACTADKNGCKVCGARIGGTDYCSQCSVGTQAPLNGVCTANARAQFCTQVTSGSCTSCSGGYFLKNGGCYQADRQPGKQICTLADSNGGCQACANGLPPSSSDVCPSCHFTCKTCSTADIANTCTTCATGYYMVGSGPNTCISCESDSGSVKGVAGCMSCAPPSSNTGSVLCYLMNGDSAGGSTNKSGLSTGAIAGISVAVIVVVGGLVGFLCWWFICRGKA

SEQ ID NO: 17 - protein, 1621 aa, Giardia
MFDKLIFVSLALQLAWASQTASRAKASPASCNPQSPDATSCAPDSCNVVIEGQTFCSKCTGGKVPVNGECKAKGDAPLCTAGANAQEGTCTACTGAQRLYMGGCYDKCPYGNGADANTCADAPAGPASCNPQSPDATSCAPDSCNVVIEGQTFCSKCTGGKVPVNGECKAKGDAPLCTAGANAQEGTCTACTGAQRLYMGGCYDKCPYGNGADANTCADAPAGPASCNPQSPDATSCAPDSCNVVIEGQTFCSKCTGGKVPVNGECKAKGDAPLCTAGANAQEGTCTACTGAQRLYMGGCYDKCPYGNGADANTCADAPAGPASCNPQSPDATSCAPDSCNVVIEGQTFCSKCTGGKVPVNGECKAKGDAPLCTAGANAQEGTCTACTGAQRLYMGGCYDKCPYGNGADANTCADAPAGPASCNPQSPDATSCAPDSCNVVIEGQTFCSKCTGGKVPVNGECKAKGDAPLCTAGANAQEGTCTACTGAQRLYMGGCYDKCPYGNGADANTCADAPAGPASCNPQSPDATSCAPDSCNVVIEGQTFCSKCTGGKVPVNGECKAKGDAPLCTAGANAQEGTCTACTGAQRLYMGGCYDKCPYGNGADANTCADAPAGPASCNPQSPDATSCAPDSCNVVIEGQTFCSKCTGGKVPVNGECKAKGDAPLCTAGANAQEGTCTACTGAQRLYMGGCYDKCPYGNGADANTCADAPAGPASCNPQSPDATSCAPDSCNVVIEGQTFCSKCTGGKVPVNGECKAKGDAPLCTAGANAQEGTCTACTGAQRLYMGGCYDKCPYGNGADANTCADAPAGPASCNPQSPDATSCAPDSCNVVIEGQTFCSKCTGGKVPVNGECKAKGDAPLCTAGANAQEGTCTACTGAQRLYMGGCYDKCPYGNGADANTCADAPAGPASCNPQSPDATSCAPDSCNVVIEGQTFCSKCTGGKVPVNGECKAKGDAPLCTAGANAQEGTCTACTGAQRLYMGGCYDKCPYGNGADANTCADAPAGPASCNPQSPDATSCAPDSCNVVIEGQTFCSKCTGGKVPVNGECKAKGDAPLCTAGANAQEGTCTACTGAQRLYMGGCYDKCPYGNGADANTCADAPAGPASCNPQSPDATSCAPDSCNVVIEGQTFCSKCTGGKVPVNGECKAKGDAPLCTAGANAQEGTCTACTGAQRLYMGGCYDKCPYGNGADTNTCADAPAGPASCNPQSPDATSCAPDSCNVVIEGQTFCSKCTGGKVPVNGECKAKGDAPLCTAGANAQEGTCAACTGAQRLYMGGCYDKCPYGNGADANTCADAPAGCNTPNCKACDNPKTDNEVCTECNDGNYLTPTSQCVSDCTTLKGYYGDDSGKKTCKKCNDACAECKGADANQCTACPAGKMLQYTDENSPSSGTCVDGCKPQSGASGCEICGATIGGTKYCSKCSTSTEVPVNGVCKADNARAPVCSKKDNQGGCATCASGYFRQDNGCYKTDRQPGIQICTLASSAGKCETCANSLQPNDGACPSCHSTCKTCSAADSSDKCTSCAAGYYMVGSAAGPCTSCDSNSGSVKGVAGCLNCAPPSSSTGSVLCYLMNGDSAGGSTNKSGLSTGAIAGISVAVIVVVGGLVGFLCWWFLCRGKA

SEQ ID NO: 18 - protein, 632 aa, Giardia
MFCRLIVAGFVLQLAWAAPEAETCTEAGEGQAGKCLTSKCDVWINGKKYCSQCAKTDEYLVDGGCKAEAGASGCQLKARAADGTCTQCAQGYFLHKNGCYAIGGDVGRFICADAAAASRVSSTTPGVCEGCVVGYFKNPSAANNKDSCIACNDATGVGGKKGLEGCATCDPPSSDVAICKTCLEGFFGTNLGNAGSTCTACTDRDNCAKCDGGAGKCTKCKATANKPYLKKGETEDSNTCIDKSGCNDNSHFTDDADDPTNGKMCKKCSEGIADCKTCALKDNPEGTILITCSACIAGTNQPNADGTKCVLCDIQDCIKCNEENMCEECTGGKSLNPLKNMCMEGCPAGTRDVSGICTNCHNSCAECDGDSEASCTACYPGLVLSKSNTGATGTCIPECTGRYAENCEAGQCTAVVGGSKYCSKCKAGYVPVDGVCVSTTTRAVTGCTPNDNNDGTCKACTTTYFLQSGGCYQSAAYPGSNLCSNAQNGKCTNCANGQQPEASTGSCPACASGCKTCEVANKEACKTCLPGYYLAGAKCVKCDTNDPNDGSHIVGVPNCISCAPPTGNSGPVTCYVKTDGTNDGGNDNNAGGSTNKSGLSTGAIAGISVAVIVVVGGLVGFLCWWFICRGKA

SEQ ID NO: 19 - protein, 616 aa, Giardia
MFEKILFANCILQLAWAACLEDDGNPGTHDTTKCKKGHCDVSIGEQPYCSKCSVDNEHLVDGTCVVSATDQANTKCIDPVEGKCGSCKDGYFMYKSGCYNSGGSPGNEMCTSAPEGKCSTPAAGYFIIPTTDADASHQSVVSCSDSEGANGKSDKIYKGVEGCAECTLDNLATTATCTKCTTDFLHAPIEGGTACLTECPEGYFGHTATSGKQLKTCQSCSSPEASLIPAATGVPNCVKCTYDTKVVCEKCDQDKYLKTESGTTSCVSAEECKDGFFPTADAQGKKVCAKCSDTVNGGIEDCAKCSLKATPASAGPLITCSECTTHNLSPLKDACLTACPAGMYANSKVCTPCHESCASCSNDAEASCTACYPGSVLNRSSGDTGACIKECTGRYAENCEADQCKAVVGGSKYCSRCKAGYVPVDGVCVSTTTRAPTGCTPGDGVCTACTGSYFLQSGGCYSAGAFPGNTLCTTASDGKCQTCANGQAADTTSGSCPACPDGCSKCATSGSPKACSECLPGYYKSGSSCVKCDASANGIVGVPNCISCAPPAGGSGSVTCYVKTDGTSGGDDNTGGSTNKSGLSTGAIAGISVAVIVVVGGLIGFLCWWFICRGKA

SEQ ID NO: 20 - protein, 1937 aa, Giardia
MLVGFLLVCATVLAKDSGKDGCEKASNTDCGEELKRAGCATCTAVGPNGQTCLTCNGGQKVQLNGISCGDSCPSNSAANPDICECNEGFNLNSGKDGCEKASNTDCGEELKRAGCATCTAVGPNGQTCLTCNGGQKVQLNGISCGDSCPSNSAANPDICECNEGFNLNSGKDGCEKASNTDCGEELKRAGCATCTAVGPNGQTCLTCNGGQKVQLNGISCGDSCPSNSAANPDICECNEGFNLNSGKDGCEKASNTDCGEELKRAGCATCTAVGPNGQTCLTCNGGQKVQLNGISCGDSCPSNSAANPDICECNEGFNLNSGKDGCEKASNTDCGEELKRAGCATCTAVGPNGQTCLTCNGGQKVQLNGISCGDSCPSNSAANPDICECNEGFNLNSGKDGCEKASNTDCGEELKRAGCATCTAVGPNGQTCLTCNGGQKVQLNGISCGDSCPSNSAANPDICECNEGFNLNSGKDGCEKASNTDCGEELKRAGCATCTAVGPNGQTCLTCNGGQKVQLNGISCGDSCPSNSAANPDICECNEGFNLNSGKDGCEKASNTDCGEELKRAGCATCTAVGPNGQTCLTCNGGQKVQLNGISCGDSCPSNSAANPDICECNEGFNLNSGKDGCEKASNTDCGEELKRAGCATCTAVGPNGQTCLTCNGGQKVQLNGISCGDSCPSNSAANPDICECNEGFNLNSGKDGCEKASNTDCGEELKRAGCATCTAVGPNGQTCLTCNGGQKVQLNGISCGDSCPSNSAANPDICECNEGFNLNSGKDGCEKASNTDCGEELKRAGCATCTAVGPNGQTCLTCNGGQKVQLNGISCGDSCPSNSAANPDICECNEGFNLNSGKDGCEKASNTDCGEELKRAGCATCTAVGPNGQTCLTCNGGQKVQLNGISCGDSCPSNSAANPDICECNEGFNLNSGKDGCEKASNTDCGEELKRAGCATCTAVGPNGQTCLTCNGGQKVQLNGISCGDSCPSNSAANPDICECNEGFNLNSGKDGCEKASNTDCGEELKRAGCATCTAVGPNGQTCLTCNGGQKVQLNGISCGDSCPSNSAANPDICECNEGFNLNSGKDGCEKASNTDCGEELKRAGCATCTAVGPNGQTCLTCNGGQKVQLNGISCGDSCPSNSAANPDICECNEGFNLNSGKDGCEKASNTDCGEELKRAGCATCTAVGPNGQTCLTCNGGQKVQLNGISCGDSCPSNSAANPDICECNEGFNLNSGKDGCEKASNTDCGEELKRAGCATCTAVGPNGQTCLTCNGGQKVQLNGISCGDSCPSNSAANPDICECNEGFNLNSGKDGCEKASNTDCGEELKRAGCATCTAVGPNGQTCLTCNGGQKVQLNGISCGDSCPSNSAANPDICECNEGFNLNSGKDGCEKASNTDCGEELKRAGCATCTAVGPNGQTCLTCNGGQKVQLNGISCGDSCPSNSAANPDICECNEGFNLNSGKDGCEKASNTDCGEELKRAGCATCTAVGPNGQTCLTCNGGQKVQLNGISCGDSCPSNSAANPDICECNEGFNLNSGKDGCEKASNTDCGEELKRAGCATCTAVGPNGQTCLTCNGGQKVQLNGISCGDSCPSNSAANPDICECNEGFNLNSGKDGCEKASNTQCNTPNCKICDNPKTDNEVCTECNDGDYLTPTNQCVPDCTTISGYYGDNDKKCKACSPECAECVGPANNQCSSCPAGKKLTYTDDSNPNNGGTCGDACKVSADGTGCETCGAQIGGTAYCSKCKTSTQAPLNGDCAASSRATFCTKMGNGVCTQCEDNYFLKDGGCYQTDRQPGKQVCSNAQGGNGKCQTCANGLAATDGNCAECHPTCATCSAPSTASSCKTCATGYYKENGDDTTDGPCMKCSEKISGCKQCVSSSGSSVICLESEVGTGGSTNKSGLSTGAIAGISVAVIVVVGGLVGFLCWWFLCRGKA

SEQ ID NO: 21 - protein, 419 aa, Giardia
MFAKLIFTSLVLQLAEATRPAVKEQSGACTSPENAGCAACNPNNGDELCLSCTNAQEFIQLNKKGCTAACAGDGVIGDAAVDPKVCKCDGDNGYTLQGDACVKRQANECQTENCQECTGKGTANEVCTKCTSTHYLTPTNQCVPDCTVIKGYYGDTNEGKCKPCSPECAECVGPANNQCSACPAGKKLTYTDDSYPNNGGACGDACKVSADGAGCETCGAQIGGTAYCSKCKTSTQAPLNGDCAANTRTQFCTTVSNGVCTQCAANYFLKDGGCYQTDRQPGKQVCSSAQGGTCTKCANGLQVQSGACGNCHSTCATCSAPSIASSCKTCATGYYKENGDDTTDGLCKKCSEKISGCKQCVSSSGSSVICLESEVGTGGSVNKSGLSTGAIAGIAVAAVIVIGGLVGFLCWWFLCRGKA

SEQ ID NO: 22 - protein, 628 aa, Giardia
MLLVVFYFVLSALAGACTVEANTRDCTENKCEMVGETEICTQCKTGGNVPIDGVCKAVAEAANKCTKSDDNPVGAGDTTCGKCVNAYFMYKGGCYLAGAAGPGTGTKMCKQAAGGKCTQAADAKNYFIPPANTDDTHDSVVWCGDEIGVTLSSTQYKGVAKCLVCDAPGGAGAATCTTCEDGYFGATCKKCHESCRTCEAAEENKCKSCTDGYFLGATNGAAGKCLKCNSKTEEGWHGVDNCAKCTSSNTQNTPATCTECVANFYLKPAAGATPSSCVTETGCGDGYFPTIVDEIKKCIACGTAANGGIDDCKKCSLKTTSAKAGIEIVCTECNTKWLSPLGDACLDSCPPGTHADSGNICPLCHSTCAECDGNAEATSCRACYPGFVLSYGSDKVRGTCIQECTGKYAENCEENMCTAVLGGSKYCSKCKAGFVPIDGVCVSTASRAVTGCTPGNGVCIACTDSYFLQSGGCYQSTVFPGNKLCTLASNGKCTACSNGQTADGQGSCPACNAICATCAAGNIDQCQTCFPGYYKSGTKCVKCSITDNGITGVENCISCAPPAGNSGPVTCYMKTDDTNDGGNDNNGGSTNKSGLSTGAIAGISVAVIVVVGGLIGFLCWWFICRGKA

SEQ ID NO: 23 - protein, 255 aa, Giardia
MLLIAFYLVLSTLAVRHTTNHHSEYLRSGSRSNRDTGNRDNAYAAGNCKDGMEEQVGADTVCKQCNAGFVPINGVCTAQGTPSIATAGCKLANNDPPGQDSTVCEQCGTDATYFLYKGGCYDASTGVGQSLCKRASNGACTEAGEGYFAAPNAKATEQSVIPCSDTTGVTLTGDKQYVGVENCATCDAPAGDETVAKCKTCSDRFSLRDNQCVPSSVNKSGLSTGAIAGIAVAAVIVVGGLVGFLCWWFLCRGKA

SEQ ID NO: 24 - protein, 127 aa, Giardia
MLVGFLLVFVVTQANCAPELTRAGCKTCSPDGQTCTACTNDSHNVQVDGKSCDANCPEHSAANGQKVCECEGGYGPVTGENRCEPSNTNKSSGLSTGAIAGIAVAAVIVVGGLVGFLCWWFLCRGKA

SEQ ID NO: 25 - protein, 704 aa, Giardia
MFGRFLLAIVILQLARAACQADGSGSDGSCKTCGVTIGQEQYCSECNGANYAPVNGQCADVNAEGQSKTLCPAKGQGKCTQCGGASFMYKDGCYSKDTAPGQSMCTQASEGKCTEAAPGYFLNPLRANTKDSVVSCSDTTGFTDSGKTYRGVQHCERCDGAALTDAAGGDAKCTRCGQDKYLATTGTCGEGCTPDTEFSKEDSDNGKRCFACGDVTTGVASCEKCTPPSPDQAKPACTKCGGNNYLKTAADGTTTCVEQSACSPDSFPVENSQSGNRCVLCGDAANGGVDKCAACTPTDQGRIAPTITCIACTNGYKPSADKTTCEAVSNCKTPGCKACSNEGKENEVCTDCDSSTYLTPTSQCIDSCAKIGNYYGATEGAKKICKECTAANCKTCDGQGQCQACSDGFYKNGDACSPCHESCKTCSAGTASDCTECPTGKALRYGDDGTKGTCGEGCTTGQGSGACKTCGLTIDGASYCSECATTTEYPQNGVCAPKASRATPTCNDSPIQNGVCGTCADNYFKMNGGCYETVKYPGKTVCISAPNGGTCQKAADGYKLDSGTLTVCSEGCKECTSSTDCTTCLDGYVKSASACTKCDSSCETCNGAATTCKACATGYYKTASGEGACTSCESDSNGVTGIKGCLNCAPPSSSTGSVLCYLIQNTNKSGLSAGAIAGISVAVIVVVAGLVGFLCWWFICRGKA

SEQ ID NO: 26 - protein, 709 aa, Giardia
MFGRFLLAIVILQLARTACTQEADDGKCKTCGVTIGQEQYCSECNGANYAPVNGACEDVETQADKKALCKAHASGACTTCGGNSFMYKDGCYSSGEGLPGHSLCLSSDGDGVCTEAAPGYFLNPLRANTKDSVVSCSDTTGFTDSGKTYRGVQYCERCDGAALTDAAGGDAKCTRCGQDKYLKDNTCVDKAQCDSGSTNKFVAVDDSENGNKCVSCSDNLNGGVANCDTCSYDEQSKKIKCTKCTDNNYLKTTSEGTSCVQKDQCKDGFFPKDDSSAGNKCLPCNDSTDGIANCATCALVSGRSGAALVTCSACTDGYKPSADKTTCEAVSNCKTPGCKACSNEGKENEVCTDCDSSTYLTPTSQCIDSCAKIGNYYGATEGAKKICKECTAANCKTCDGQGQCQACSDGFYKNGDACSPCHESCKTCSAGTASDCTECPTGKALRYGDDGTKGTCGAGCATGTGAGACKTCGLTIDGASYCSECATATEYPQNGVCSSTTVRAAATCKAGSVAKGMCNSCTNGFLRMNGGCYETTKFPGKNVCEEAAPAGDTCQTPADGYKLNNGALITCSAGCKTCTSQDQCDTCKAGYAKTGGNTKKCVPCATGCSECNADDATKCTVCAAGYYLSKEKCIACDKSDGGSITGVANCANCAPPTNNKGPVLCYLIQNTNRSGLSTGAIAGISVAVVAVVGGLVGFLCWWFLCRGKA

SEQ ID NO: 27 - protein, 1347 aa, Giardia
MLVGFLLVCATVLAKDSGKTAQCDGDNGYTLQGDACTKAAPDNACQTLGTAGCATCDSGSGGETCLTCKKDAQYVAANKKSCKDACDTSGGEVIDQAASPAKVCKCDGDNGYTLQGDACTKAAPDNACQTLGTAGCATCDSGSGGETCLTCKKDAQYVAANKKSCKDACDTSGGEVIDQAASPAKVCKCDGDNGYTLQGDACTKAAPDNACQTLGTAGCATCDSGSGGETCLTCKKDAQYVAANKKSCKDACDTSGGEVIDQAASPAKVCKCDGDNGYTLQGDACTKAAPDNACQTLGTAGCATCDSGSGGETCLTCKKDAQYVAANKKSCKDACDTSGGEVIDQAASPAKVCKCDGDNGYTLQGDACTKAAPDNACQTLGTAGCATCDSGSGGETCLTCKKDAQYVAANKKSCKDACDTSGGEVIDQAASPAKVCKCDGDNGYTLQGDACTKAAPDNACQTLGTAGCATCDSGSGGETCLTCKKDAQYVAANKKSCKDACDTSGGEVIDQAASPAKVCKCDGDNGYTLQGDACTKAAPDNACQTLGTAGCATCDSGSGGETCLTCKKDAQYVAANKKSCKDACDTSGGEVIDQAASPAKVCKCDGDNGYTLQGDACTKAAPDNACQTLGTAGCATCDSGSGGETCLTCKKDAQYVAANKKSCKDACDTSGGEVIDQAASPAKVCKCDGDNGYTLQGDACTKAAPDNACQTLGTAGCATCDSGSGGETCLTCKKDAQYVAANKKSCKDACDTSGGEVIDQAASPAKVCKCDGDNGYTLQGDACTKAAPDNACQTLGTAGCATCDSGSGGETCLTCKKDAQYVAANKKSCKDACDTSGGEVIDQAASPAKVCKCDGDNGYTLQGDACTKAAPDNACQTLGTAGCATCDSGSGGETCLTCKKDAQYVAANKKSCKDACDTSGGEVIDQAASPAKVCKCDGDNGYTLQGDACTKAAPDNACQTLGTAGCATCDSGSGGETCLTCKKDAQYVAANKKSCKDACDTSGGEVIDQAASPAKVCKCDGDNGYTLQGDACTKAAPDNACQTENCQECTSKGTANEVCTKCTSTHYLTPTNQCVPDCAAISGYYGDTDKKCKPCSLECAECVGPANNQCSACPAGKKLTYTDDSHPNNGGACGDACKVSADGTGCETCGAQIGGTAYCSKCKTSTQAPLNGNCAANSRAAFCATITNGACTQCNEGYFLKDGGCYQTDRQPGKQVCSSAQGGTCQTCANGLQAQGGACGECHSTCATCSTAGAADKCKTCATGYYKTSDSDGPCMKCSEKISGCKQCVSSSGSSVICLESEVGTGGSVNKSGLSTGAIAGIAVAVIVVVGGLVGFLCWWFLCRGKA

SEQ ID NO: 28 - protein, 419 aa, Giardia
MLVGFLLVCATVLAKHNGKNGCEKASNTACEERLTQAGCETCTGVGQDQTCLTCGGGKKVQLNGVSCDATCPQNSAANDQNVCVCNPGFSLNNGKTACEKASNTQCNTPNCKACDNPKTDNEICTECNDGNYLTPTKQCTQSCGAIGSYYNGDKECEPCDPSCAGCTTKGPAKCTACPPGKMLKYTNDDPNQGGSCVDECKAEVDGCAECGAVIGGTKYCSKCKEDKWAPQNGVCANSVTRNSFCTNAAGGVCTQCAADHFLQDGGCYKLGRQPGEQICTLADSNGGCQTCANSLQPNNGACPSCHSTCKTCRDANSANACTTCATGYYMVGLDPGTCTSCESDSGSVKGVAGCMSCAPPSNNQGSVLCYLKNGDSTGGSTNRSGLSTGAIAGISVAVIVVVGGLVGFLCWWFLCRGKA

SEQ ID NO: 29 - protein, 587 aa, Giardia
MLVGFLLVCATVLAKDSGKDTCFPGYTLNPTTKKCDRNSAPCEVEGCDVCEESNPQQCKTCGSGYTLNPTTKKCDRNSAPCEVEGCDVCEESNPQQCKTCGSGYTLNPTTKKCDRNSAPCEVEGCDVCEESNPQQCKTCGSGYTLNPTTKKCDRNSAPCEVEGCDVCEESNPQQCKTCGSGYTLNPTTKKCDRNSAPCEVEGCDVCEESNPQQCKTCGSGYTLNPTTKKCDRNSAPCEVEGCDVCEESNPQQCKTCGSGYTLNPTTKKCDRNSAPCDTPNCKACDNPKTDNEICTECNDNNYLTPTSQCVSDCTTLKGYYGDDSGKKTCKRCNDACAECKGEGADKCTACPAGKMLQYTDADTPANGGTCMNQCSVSPANDGCAECGAQIGGTAYCSKCKNTQQAPLDGNCAANTRTRFCTTVSNGACTQCENNYFLKDGGCYQTNRQPGKQVCTQANGGKCQTCANGLAATDGNCAECHPTCATCSTAGTADKCKTCATGYYKENGSDTTTGLCKKCSEKISGCKQCVSSSGSSVICLESEVGTGGSVNKSGLSTGAIAGISVAVIVVVGGLVGFLCWWFLCRGKA

SEQ ID NO: 30 - protein, 900 aa, Giardia
MLVGFLLVFTVTQAHRTSVSTDCPIENCQTCSSDKATCEACKPGFVASGDNRACNPAPADCPIENCQTCSSDKATCEACKPGFVASGDNRACNPAPADCPIENCQTCSSDKATCEACKPGFVASGDNRACNPAPADCPIENCQTCSSDKATCEACKPGFVASGDNRACNPAPADCPIENCQTCSSDKATCEACKPGFVASGDNRACNPAPADCPIENCQTCSSDKATCEACKPGFVASGDNRACNPAPADCPIENCQTCSSDKATCEACKPGFVASGDNRACNPAPADCPIENCQTCSSDKATCEACKPGFVASGDNRACNPAPADCPIENCQTCSSDKATCEACKPGFVASGDNRACNPAPADCPIENCQTCSSDKATCEACKPGFVASGDNRACNPAPADCPIENCQTCSSDKATCEACKPGFVASGDNRACNPAPADCPIENCQTCSSDKATCEACKPGFVASGDNRACNPAPADCPIENCQTCSSDKATCEACKPGFVASGDNRACNPAPADCPIENCQTCSSDKATCEACKPGFVASGDNRACNPAPADCPIENCQTCSSDKATCEACKPGFVASGDNRACNPAPADCPIENCQTCSSDKQTCEACEPGKHLTPTKKACLDACPVGTYLSGQTCAPCDPSCAECSGAGASKCTACPAGKMLRYADESKLNEGGTCVEQCVEGPECETCGLTIGGTKYCSKCKGSNVPLNGVCTSNAARTLFCTTAANGACTVCAAGYFIQEGGCYKTDRLPGKSICTTPTGDGKCQTCANGLTAVSNMCPLCDSTCATCTVANQPDKCSACPPGRYLDASKACKLCTETSGSIQGVANCASCDPPTGNSGSVICYVKTDGTDNGGSVNKSGLSTGAIAGISVAVIVVVGGLVGFLCWWFLCRGKA

SEQ ID NO: 31 - protein, 200 aa, Giardia
MLSKLLFVSFILQLAQAVQVVEEAKAAVSAPTPCDAADPGATNCAAGKCDVTINGKTYCSKCKSGYVPVNGACTQQAQANMCTPGSGSTDGTCTACTQTQKLYKGGCYDNCPYGDGSAPNTCADAPAGCDLPNCKSCPDGTCTECNDGFVLGDDKKCVPSSANKSGLSTGAIAGIAVAAVIVVGGLVGFLCWWFLCRGKA

SEQ ID NO: 32 - protein, 200 aa, Giardia; identical to SEQ ID NO: 31

SEQ ID NO: 33 - protein, 403 aa, Giardia
MLVGFLLVCATVLAKHNEKTAPCEVEGCDVCEESNPQQCKTCGSGYTLNPTTKKCTKNPASDCGVQNCAQCVSGDNTRCETCSPGFDPNDDGTQCTPQADCPIVNCQTCSPDKQTCEECEPGKHLTPTKKACLDACPVGTYLSGQTCAPCDPSCAECSGAGASKCTACPAGKMLRYADESNPTDGTCVEQCVEGPECETCGLTIGGTKYCSKCKGNNVPLNGVCTSNAARTRFCTTAANGACTVCAAGYFIQEGGCYQTTRLPGKSICTTPTGDGKCQTCANGLTAVSNMCPLCDSTCATCTEANQPNKCSACPPGRYLDASKACKLCTETSNNIQGVANCASCAPPSNNQGPVLCYLMKDGGSTNKSGLSTGAIAGISVAVIVVVGGLVGFLCWWFICRGKA

SEQ ID NO: 34 - protein, 228 aa, Giardia
MFAGLIFASLVLQLAAATRPAERSRSDTPCTESGNDTCQTCSGSGSNEICLTCKNNDHFLTTNKKGCKAACDATGEIETPGANPKACKCDDASGYQLQGDGTCAKGQDTPCTESGNDTCQTCSGSGSNEICLTCKNNDHFLTTNKKGCKAACDATGEIETPGANPKACKCDDASGYQLQGDGTCAVSNTNKSSGLSTGAIAGIAVAAVIVVGGLVGFLCWWFLCRGKA

SEQ ID NO: 35 - protein, 636 aa, Giardia
MFYAFLLIGLTLQLATEECTPVSGGGPETCKTCGATIGGVSYCSQCNDSGSESAPTDGKCTTDNAVCNAKAEGKCTTCTGSSFMYKGGCYSKDTKPGNAACTQAAAGVCTQAAQGYFLPPDADRDNAHQSAIPCGSEEEVPAKNNHKYKGVPHCTQCDTPDVAADANAKAATCTACESGYFVDNSKGKTCTACADNCLTCTDGTVSKCKSCTAETYFLATEGSEGPCISCGDATQGSGAWKGVAGCAKCTKPQSAGPATCTECQADKYLKTESGTASCVSAEECKDGFFPTADAQGKKVCAKCSDTANGGIEDCAKCSLKATSARAGPMVTCSGCETKRLSPLNDACLEECPAGTYPDNRDSTGICASCHNTCASCSTNAETSCTACYPGYVLSRSSGDAGTCIKECTGDFMAHCKADGCSLNVGGSKYCDQCEDGYAPVDGVCTKVASTARDASGCKASGGKCTECGANYALLSGGCYNTNKVPGNSVCTLSVGGKCTMCVASGADPKGQACPTCPDGCLKCTGNVGSQTCSSCLSGYYLSTNKCFRCTAGDGASANAITGVENCISCAPPTGGNGGSVTCYVKNDDSSGSGTGGSTNKSGLSTGAIAGISVAVIVVVGGLVGFLCWWFICRGKA

SEQ ID NO: 36 - protein, 636 aa, Giardia; identical to SEQ ID NO: 35

SEQ ID NO: 37 - protein, 1099 aa, Giardia
MLLGLLLFCAVARANCKAGNTPSQDGTTCEPNANGCAKALTDAGCATCTPAGDDQTCLTCNPGSNKVRPDRKGCIASCPANSNEAGGICTCTAGNTPSQDGTTCEPNANGCAKALTDAGCATCTPAGDDQTCLTCNPGSNKVRPDRKGCIASCPANSNEAGGICTCTAGNTPSQDGTTCEPNANGCAKALTDAGCATCTPAGDDQTCLTCNPGSNKVRPDRKGCIASCPANSNEAGGICTCTAGNTPSQDGTTCEPNANGCAKALTDAGCATCTPAGDDQTCLTCNPGSNKVRPDRKGCIASCPANSNEAGGICTCTAGNTPSQDGTTCEPNANGCAKALTDAGCATCTPAGDDQTCLTCNPGSNKVRPDRKGCIASCPANSNEAGGICTCTAGNTPSQDGTTCEPNANGCAKALTDAGCATCTPAGDDQTCLTCNPGSNKVRPDRKGCIASCPANSNEAGGICTCTAGNTPSQDGTTCEPNANGCAKALTDAGCATCTPAGDDQTCLTCNPGSNKVRPDRKGCIASCPANSNEAGGICTCTAGNTPSQDGTTCEPNANGCAKALTDAGCATCTPAGDDQTCLTCNPGSNKVRPDRKGCIASCPANSNEAGGICTCTAGNTPSQDGTTCEPNANGCAKALTDAGCATCTPAGDDQTCLTCNPGSNKVRPDRKGCIASCPANSNEAGGICTCTAGNTPSQDGTTCEPNANGCAKALTDAGCATCTPAGDDQTCLTCNPGSNKVRPDRKGCIASCPANSNEAGGICTCTAGNTPSQDGTTCVSETACNTPNCKACDNPKTDREVCTECNDKSYLTPTNQCVSDCTAISGYYGDTDRKCKACSPECAECVGPANNQCSACPAGKALIYKSSDPMQGGTCGDACTADKNGCKVCGARIGGTDYCSQCSVDNQAPLNGVCTTSNARVAFCTEMNNGACTKCAANYFLKEGGCYETTKQPGKQICTLADSKGECETCANGLQPNNGACPSCHSTCKTCSTADSSDKCTSCAAGYYMVGSAAGPCTSCDSNSGSVKGVAGCMSCAPPSNNQGSVLCYLMNGDSAGGSTNKSGLSTGAIAGIAVAAVIIVGGLVGFLCWWFLCRGKA

SEQ ID NO: 38 - protein, 870 aa, Giardia
MLVGFLLVCATVLAKYNEKDTCFPGYTINNDTKQCTKDPEAPCNTPNCKACDNPKTDNEACTDCDPAYVLNGGQCVERKCNTPNCKACDNPKTDNEACTDCDPAYVLNGGQCVERKCNTPNCKACDNPKTDNEACTACDPAYVLNGGQCVEKACNTPNCKACDNPKTDNEACTDCDPAYVLNGGQCVERKCNTPNCKACDNPKTDNEACTACDPAYVLNGGQCVEKACNTPNCKACDNPKTDNEACTDCDPAYVLNGGQCVERKCNTPNCKACDNPKTDNEACTDCDPAYVLNGGQCVERKCNTPNCKACDNPKTDNEACTDCDPAYVLNGGQCVERKCNTPNCKACDNPKTDNEACTACDPAYVLNGGQCVEKACNTPNCKACDNPKTDNEACTDCDPAYVLNGGQCVERKCNTPNCKACDNPKTDNEACTACDPAYVLNGGQCVEKACNTPNCKACDNPKTDNEACTDCDPAYVLNGGQCVERKCNTPNCKACDNPKTDNEACTDCDPAYVLNGGQCVERKCNTPNCKACDNPKTDNEACTACDPAYVLNGGQCVEKACNTPNCKACDNPKTDNEACTECNDNNYLTPTNQCVPDCTAISGYYGDNDKKCKACSPECAECVGPANNQCSACPAGKKLTYTDDSHPNNGGACGDACKVSADGTGCETCGAQIGGTAYCSKCKTSTQAPLNGNCAANSRAAFCATITNGACTQCNEGYFLKDGGCYQTDRQPGKQVCSSAQGGTCQTCANGLQAQGGACGECHSTCATCSTADAADKCKTCATGYYKENGDDTTDGLCKKCSEKISGCKQCVSSSGSSVICLESEAGTGGSVNKSGLSTGAIAGISVAVIVVVGGLVGFLCWWFLCRGKA

SEQ ID NO: 39 - protein, 673 aa, Giardia
MLLVAFCFALSTLAATCSADTQVGKCKENMCEMAGSTEICTECKDQGNVPIDGICKPQNDNAVTTAGCKKKAGDNVDASSVRCEQCDAANHFLYKGGCYSKDATPGNQMCKTVTTNGICAEAATTKNYFVVPGATKTDQSVVWCGDVEGVTLGDGKKYTGVDGCTTCEKPEQATDAPKAATCNACGGGKIVKTVDGVTSCVEEADCNNGYFVDSRNGKKCSKCASSCKTCENTETQCTSCTEATPYLKKEDDSETGTCVNQGDCPATHYIDEAAKTCTTCTSGGAKDCKTCEKNGDGAVCKECPDSDKTIFGLNKKSCVASCPANSTPKATGQDSQVCECNEGLQPNTESTECRPISNCNTEHCLECTGEGADKEVCTKCLSEYYLTPTSQCVSDCTTLKGYYGDDSGKKTCKKCNDACVECKGEGADKCTACPAGKMLQYTDADTPANGGTCMNQCSVSSTNDGCAECGAQIGGTAYCSKCKNAQQAPLDGNCAANTRTRFCTTVSNGACTQCENNYFLKDGGCYQTNRQPGKQVCTTVQGGKCTKCASGLTADNGDCSNKRCHLSCETCTAANDANACATCSTGYYKPQSAGTKCNPCSEGLAGCRQCTVSSTDAFMCLEMGDGTSDNTGGSTNKSGLSTGAIAGISVAVIVVVGGLVGFLCWWFICRGKA

SEQ ID NO: 40 - protein, 673 aa, Giardia; identical to SEQ ID NO: 39

SEQ ID NO: 41 - protein, 635 aa, Giardia
MFYAFLLIGLALQLATEECTTVSGDQPDTCKACSAVINGKKYCSQCNGGGSQSAPTDGVCSADNNECSQKQDGVCTQCANKSFMYKGGCYKDSQAPGNTMCETATDGVCTQAKAGYFVPPGADASHQSVIPCGDEEEITVKNDKKYKGVLHCTQCEEPTEASDTTTPKAATCTACESGYFVDNSKGKTCTACADNCLTCTDGTVSKCKSCTAETYFLATEGSEGPCISCGDATQGSGAWKGVAGCAKCTKPQSAGPATCTECQADKYLKTESGTASCASAEECKDGFFPMTDAQNSNRKVCALCSEADKGGIANCKKCSLKATSARAGPIVTCSECTNNNLSPLKDECMLDCPAGTYANSKVCTRCHESCANCSDNAEASCTACYPGSVLEHDGDPTTGKCIQECTGRYAENCEAGQCTAVVGGSKYCSRCKTGFVPINDMCVSTTARAAAECVAGEGVCTSCTGAYFLESGGCYKTGAFPGNTLCIAAGANGKCANCANGQNADPQTGACPPCPANCSKCSGDSGVKTCTECYSGYYLDTGKECKKCSETSGNIQGVPNCVSCKAPSSPNAPTPVTCYVKTDGTNNGDNDNNGGSTNKSGLSTGAIAGISVAVVVVVAGLVGFLCWWFICRGKA

SEQ ID NO: 42 - protein, 128 aa, Giardia
MLLLVLCFLMSALAAQCKGRQHSNCATDQCRAGHVPIDVCADSSAVYGAGSECTDPNCKRCDQNPAECEECNSGFDLDGSTKQCISSNTNKSSGLSTGAIAGIAVAAVIIVGGLVGFLCWWFLCRGKA

SEQ ID NO: 43 - protein, 938 aa, Giardia
MLVGFLLVFVVTQANCAQELTQAGCKTCVGADAAQTCTECTTSGHKVQLDKRSCGPTCPAHSTASSNVCECDQGYTPNAGKTACEPNPSAGCAQELTQAGCKTCVGADAAQTCTECTTSGHKVQLDKRSCGPTCPAHSTASSNVCECDQGYTPNAGKTACEPNPSAGCAQELTQAGCKTCVGADAAQTCTECTTSGHKVQLDKRSCGPTCPAHSTASSNVCECDQGYTPNAGKTACEPNPSAGCAQELTQAGCKTCVGADAAQTCTECTTSGHKVQLDKRSCGPTCPAHSTASSNVCECDQGYTPNAGKTACEPNPSAGCAQELTQAGCKTCVGADAAQTCTECTTSGHKVQLDKRSCGPTCPAHSTASSNVCECDQGYTPNAGKTACEPNPSAGCAQELTQAGCKTCVGADAAQTCTECTTSGHKVQLDKRSCGPTCPAHSTASSNVCECDQGYTPNAGKTACEPNPSAGCAQELTQAGCKTCVGADAAQTCTECTTSGHKVQLDKRSCGPTCPAHSTASSNVCECDQGYTPNAGKTACEPNPSAGCAQELTQAGCKTCVGADAAQTCTECTTSGHKVQLDKRSCGPTCPAHSTASSNVCECDQGYTPNAGKTACEVASNTQCNTPNCKICDNPKTDNEICTECNDGDYLTPTKQCTQSCGAIGSYYNGDKVCEPCNPSCAACTTKGPAKCTLCPPGKRLQYTDENSPSSGTCVDECKPQSGASGCETCGATIGGTKYCSKCSTSTEVPVNGVCTADNARAPVCSKKDNQGGCTTCASGYFRQDNGCYKTDRQPGKQICTLADSNGGCQACANGLPPSSSDVCPSCHFTCKTCSTADTANTCTTCATGYYMVGSAAGPCTSCDSNSGSVKGVAGCMSCAPPSNNQGSVLCYLIKDTGSTNRSGLSTGAIVGIFVAVIVVVGGLVGFLCWWFLCRGKA

SEQ ID NO: 44 - protein, 2153 aa, Giardia
MLLVLLASCIAVQAAVCAPALIGAGCATCTGENDGQTCLTCNPQENKVQPGGKKCGVGCPANSTPKESVCECNGGYRPNAQGQCEQDPAAVCAPALIGAGCATCTGENDGQTCLTCNPQENKVQPGGKKCGVGCPANSTPKESVCECNGGYRPNAQGQCEQDPAAVCAPALIGAGCATCTGENDGQTCLTCNPQENKVQPGGKKCGVGCPANSTPKESVCECNGGYRPNAQGQCEQDPAAVCAPALIGAGCATCTGENDGQTCLTCNPQENKVQPGGKKCGVGCPANSTPKESVCECNGGYRPNAQGQCEQDPAAVCAPALIGAGCATCTGENDGQTCLTCNPQENKVQPGGKKCGVGCPANSTPKESVCECNGGYRPNAQGQCEQDPAAVCAPALIGAGCATCTGENDGQTCLTCNPQENKVQPGGKKCGVGCPANSTPKESVCECNGGYRPNAQGQCEQDPAAVCAPALIGAGCATCTGENDGQTCLTCNPQENKVQPGGKKCGVGCPANSTPKESVCECNGGYRPNAQGQCEQDPAAVCAPALIGAGCATCTGENDGQTCLTCNPQENKVQPGGKKCGVGCPANSTPKESVCECNGGYRPNAQGQCEQDPAAVCAPALIGAGCATCTGENDGQTCLTCNPQENKVQPGGKKCGVGCPANSTPKESVCECNGGYRPNAQGQCEQDPAAVCAPALIGAGCATCTGENDGQTCLTCNPQENKVQPGGKKCGVGCPANSTPKESVCECNGGYRPNAQGQCEQDPAAVCAPALIGAGCATCTGENDGQTCLTCNPQENKVQPGGKKCGVGCPANSTPKESVCECNGGYRPNAQGQCEQDPAAVCAPALIGAGCATCTGENDGQTCLTCNPQENKVQPGGKKCGVGCPANSTPKESVCECNGGYRPNAQGQCEQDPAAVCAPALIGAGCATCTGENDGQTCLTCNPQENKVQPGGKKCGVGCPANSTPKESVCECNGGYRPNAQGQCEQDPAAVCAPALIGAGCATCTGENDGQTCLTCNPQENKVQPGGKKCGVGCPANSTPKESVCECNGGYRPNAQGQCEQDPAAVCAPALIGAGCATCTGENDGQTCLTCNPQENKVQPGGKKCGVGCPANSTPKESVCECNGGYRPNAQGQCEQDPAAVCAPALIGAGCATCTGENDGQTCLTCNPQENKVQPGGKKCGVGCPANSTPKESVCECNGGYRPNAQGQCEQDPAAVCAPALIGAGCATCTGENDGQTCLTCNPQENKVQPGGKKCGVGCPANSTPKESVCECNGGYRPNAQGQCEQDPAAVCAPALIGAGCATCTGENDGQTCLTCNPQENKVQPGGKKCGVGCPANSTPKESVCECNGGYRPNAQGQCEQDPAAVCAPALIGAGCATCTGENDGQTCLTCNPQENKVQPGGKKCGVGCPANSTPKESVCECNGGYRPNAQGQCEQDPAAVCAPALIGAGCATCTGENDGQTCLTCNPQENKVQPGGKKCGVGCPANSTPKESVCECNGGYRPNAQGQCEQDPAAVCAPALIGAGCATCTGENDGQTCLTCNPQENKVQPGGKKCGVGCPANSTPKESVCECNGGYRPNAQGQCEQDPAAVCAPALIGAGCATCTGENDGQTCLTCNPQENKVQPGGKKCGVGCPANSTPKESVCECNGGYRPNAQGQCEQDPAAVCAPALIGAGCATCTGENDGQTCLTCNPQENKVQPGGKKCGVGCPANSTPKESVCECNGGYRPNAQGQCEQDPAAVCAPALIGAGCATCTGENDGQTCLTCNPQENKVQPGGKKCGVGCPANSTPKESVCECNGGYRPNAQGQCEQDPAAVCAPALIGAGCATCTGENDGQTCLTCNPQENKVQPGGKKCGVGCPANSTPKESVCECNGGYRPNAQGQCEQDPAAVCAPALIGAGCATCTGENDGQTCLTCNPQENKVQPGGKKCGVGCPANSTPKESVCECNGGYRPNAQGQCEQDPAAVCAPALIGAGCATCTGENDGQTCLTCNPQENKVQPGGKKCGVGCPANSTPKESVCECNGGYRPNAQGQCEQDPAAVCAPALIGAGCATCTGENDGQTCLTCNPQENKVQPGGKKCGVGCPANSTPKESVCECNGGYRPNAQGQCEPSNTNKSSGLSTGAIAGIAVAAVIVVGGLVGFLCWWFICRGKA

SEQ ID NO: 45 - protein, 128 aa, Giardia
MLLVLLASCIAVQAAVCAPALIGAGCATCTGENDGQTCLTCNPQENKVQPGGKKCGVGCPANSTPKESVCECNGGYRPNAQGQCEPSNTNKSSGLSTGAIAGIAVAAVIVVGGLVGFLCWWFICRGKA

SEQ ID NO: 46 - protein, 633 aa, Giardia
MLLIVFYLVLSALAANCETEGNKSNCDSGRCEMVGIVEVCTQCKTNGHVPIDGVCTPKNEADANCKKDGGSPLDQDAKICGQCAQGYFLHKGGCYAIGGNVGRIICNDPTPTLKGRNSVEGVCSACNSTSGFFKNPANVANKDSCIACDDTTGDSGNVGLEGCATCQHSGSGAATCLTCKDGYYDNNPSQDTVTCASCTDDCKTCIDTGNAKCTSCQTKYLKITDPNGVFGECVDENTCKQPGTHFPITTTDNIKVCALCSDAENKGVVGCAKCTSTPASDSGNAIIVKCIECTTPDTTKPNFAGTGCFACSATDCSNCSADNVCEKCGKGKKLSPLKDSCLDSCPAGTHNKDNVCVPCHTSCAECASDSVGESSCTACYPGFALRKGEDEATGACIPECTGKYAENCEAGQCTAIVGGSKYCSKCKAGYVPVDGVCVSTTARTPTGCTPNDNNDGTCKECTTTYFLQSGGCYNAQTFPGKLLCTAATGNGQCQTCAASGQSPAGGKCPECSEGCAKCTDSNTCNECFSGYYKGAGNKCFKCTDGDKANSDAITGVENCVSCAPPISGNGGSVICYVKTDGTGGGDNDNNTGGSTNKSGLSTGAIAGIAVAAVIVVGGLVGFLCWWFICRGKA

SEQ ID NO: 47 - protein, 633 aa, Giardia; identical to SEQ ID NO: 46

SEQ ID NO: 48 - protein, 598 aa, Giardia
MLVGFLLVCATVLAKDSGKTACEQKTGVCDGSLTTAGCATCTPAGSSQTCLTCTTSSHKIRPDEKGCISECPADVSTDVDGFCKCKSGYTPSTNGQTCEQKTGVCDGSLTTAGCATCTPAGSSQTCLTCTTSSHKIRPDEKGCISECPADVSTDVDGFCKCKSGYTPSTNGQTCEQKTGVCDGSLTTAGCATCTPAGSSQTCLTCTTSSHKIRPDEKGCISECPADVSTDVDGFCKCKSGYTPSTNGQTCEQKTGVCDGSLTTAGCATCTPAGSSQTCLTCTTSSHKIRPDEKGCISECPADVSTDVDGFCKCKSGYTPSTNGQTCEQKTGVCDGSLTTAGCATCTPAGSSQTCLTCTTSSHKIRPDEKGCISECPADVSTDVDGFCKCKSGYTPSTNGQTCEQKTGVCDGSLTTAGCATCTPAGSSQTCLTCTTSSHKIRPDEKGCISECPADVSTDVDGFCKCKSGYTPSTNGQTCEQKTGVCDGSLTTAGCATCTPAGSSQTCLTCTTSSHKIRPDEKGCISECPADVSTDVDGFCKCKSGYTPSTNGQTCEPSNTNKSGGLSTGAIAGIAVAAIIVVGGLVGFLCWWFLCRGKA

SEQ ID NO: 49 - protein, 1487 aa, Giardia
MFEKIIFGIAILQLALAAQTTGKNPAVTCAEDKTRNRTYKTQCTQASPSNCQVDHCTRCAAGNPAVCDECEPGYTANPEKTQCTQASPSNCQVDHCTRCAAGNPAVCDECEPGYTANPEKTQCTQASPSNCQVDHCTRCAAGNPAVCDECEPGYTANPEKTQCTQASPSNCQVDHCTRCAAGNPAVCDECEPGYTANPEKTQCTQASPSNCQVDHCTRCAAGNPAVCDECEPGYTANPEKTQCTQASPSNCQVDHCTRCAAGNPAVCDECEPGYTANPEKTQCTQASPSNCQVDHCTRCAAGNPAVCDECEPGYTANPEKTQCTQASPSNCQVDHCTRCAAGNPAVCDECEPGYTANPEKTQCTQASPSNCQVDHCTRCAAGNPAVCDECEPGYTANPEKTQCTQASPSNCQVDHCTRCAAGNPAVCDECEPGYTANPEKTQCTQASPSNCQVDHCTRCAAGNPAVCDECEPGYTANPEKTQCTQASPSNCQVDHCTRCAAGNPAVCDECEPGYTANPEKTQCTQASPSNCQVDHCTRCAAGNPAVCDECEPGYTANPEKTQCTQASPSNCQVDHCTRCAAGNPAVCDECEPGYTANPEKTQCTQASPSNCQVDHCTRCAAGNPAVCDECEPGYTANPEKTQCTQASPSNCQVDHCTRCAAGNPAVCDECEPGYTANPEKTQCTQASPSNCQVDHCTRCAAGNPAVCDECEPGYTANPEKTQCTQASPSNCQVDHCTRCAAGNPAVCDECEPGYTANPEKTQCTQASPSNCQVDHCTRCAAGNPAVCDECEPGYTANPEKTQCTQASPSNCQVDHCTRCAAGNPAVCDECEPGYTANPEKTQCTQASPSNCQVDHCTRCAAGNPAVCDECEPGYTANPEKTQCTQASPSNCQVDHCTRCAAGNPAVCDECEPGYTANPEKTQCTQASPSNCQVDHCTRCAAGNPAVCDECEPGYTANPEKTQCTQASPSNCQVDHCTRCAAGNPAVCDECEPGYTANPEKTQCTQASPSNCQVDHCTRCAAGNPAVCDECEPGYTANPEKTQCTQASPSNCQVDHCTRCAAGNPAVCDECEPGYTANPEKTQCTQASPSNCQVDHCTRCAAGNPAVCDECEPGYTANPEKTQCTQASPSNCQVDHCTRCAAGNPAVCDECEPGYTANPEKTQCTQASPSNCQVDHCTRCAAGNPAVCDECEPGYTANPEKTQCTQASPSNCQVDHCTRCAAGNPAVCDECEPGYTANPEKTQCTQASPSNCQVDHCTRCAAGNPAVCDECEPGYTANPEKTQCTQASPSNCQVDHCTRCAAGNPAVCDECEPGYTANPEKTQCTQASPSNCQVDHCTRCAAGNPAVCDECEPGYTANPEKTQCTQASPSNCQVDHCTRCAAGNPAVCDECEPGYTANPEKTQCTQASPSNCQVDHCTRCAAGNPAVCDECEPGYTANPEKTQCISSNTNKSSGLSTGAIAGIAVAAVIVVGGLVGFLCWWFLCRGKA

SEQ ID NO: 50 - protein, 1419 aa, Giardia
MLLGIVLLCAAVLAKECVPQISGCAECDESTGTKCTRCDPAGNTPFLMETTPDGGEGTCVGDCTQTPGYYGDASDDQNKKCKKCNAACAACSGAEATKCTRCDPAGNTPFLMETTPDGGEGTCVGDCTQTPGYYGDASDDQNKKCKKCNAACAACSGAEATKCTRCDPAGNTPFLMETTPDGGEGTCVGDCTQTPGYYGDASDDQNKKCKKCNAACAACSGAEATKCTRCDPAGNTPFLMETTPDGGEGTCVGDCTQTPGYYGDASDDQNKKCKKCNAACAACSGAEATKCTRCDPAGNTPFLMETTPDGGEGTCVGDCTQTPGYYGDASDDQNKKCKKCNAACAACSGAEATKCTRCDPAGNTPFLMETTPDGGEGTCVGDCTQTPGYYGDASDDQNKKCKKCNAACAACSGAEATKCTRCDPAGNTPFLMETTPDGGEGTCVGDCTQTPGYYGDASDDQNKKCKKCNAACAACSGAEATKCTRCDPAGNTPFLMETTPDGGEGTCVGDCTQTPGYYGDASDDQNKKCKKCNAACAACSGAEATKCTRCDPAGNTPFLMETTPDGGEGTCVGDCTQTPGYYGDASDDQNKKCKKCNAACAACSGAEATKCTRCDPAGNTPFLMETTPDGGEGTCVGDCTQTPGYYGDASDDQNKKCKKCNAACAACSGAEATKCTRCDPAGNTPFLMETTPDGGEGTCVGDCTQTPGYYGDASDDQNKKCKKCNAACAACSGAEATKCTRCDPAGNTPFLMETTPDGGEGTCVGDCTQTPGYYGDASDDQNKKCKKCNAACAACSGAEATKCTRCDPAGNTPFLMETTPDGGEGTCVGDCTQTPGYYGDASDDQNKKCKKCNAACAACSGAEATKCTRCDPAGNTPFLMETTPDGGEGTCVGDCTQTPGYYGDASDDQNKKCKKCNAACAACSGAEATKCTRCDPAGNTPFLMETTPDGGEGTCVGDCTQTPGYYGDASDDQNKKCKKCAEGQKPNTAGNKCFVCPDANCERCDQSDVCARCSTGAPLENGKCPAATPGCHSSCDGCTSDAMTNQADKCTGCKEGRYLKPNPAAGQSGTCLTAEECTSDKTHFTKEKVGDSKGMCLPCSDATHGIADCKKCALKTLSGETESTVVCSECTDKWLTPSGNACLEQCPAGTYPNDNNLCTPCHDTCAECNGNADAASCTACYPGYSLLYGSGTAGTCVKECTGAFGANCADGQCTADVGGAKYCAQCKDGYAPIDGICTAVKTGRDASVCTAAGGKCTKCAGEYTLMSGGCYGVAKLPGKSVCTLANNGKCTMCAANSQAPVQDKCPECSEGCAKCNDSNACTECLPGYYKNKSSACIPCSKDSTPITGVPNCVSCAPPAGGNGGPVLCYLMKGADNTGGSTNKSGLSTGAIAGISVAVIVVVGGLVGFLCWWFLCRGKA

SEQ ID NO: 51 - protein, 551 aa, Giardia
MLLVAFYFVLSALAAECSAEGTAKDNCEANHCEMVGGTEICTQCQTGKVPIDGQCAGATDSNTKCKNADGVADADQTCGKCLLETFMYKGGCYVTTKAPGNVMCGDAAAGKCTQVKAGYFLPPGADNAHDSVVSCGDTTGVTLTDNKKYTGVAGCGKCEQPGEAQNGTPKAATCTECQADKYLKTESGTTSCVDEGNCNNGFFPTTDAQSNNKKVCALCSEADKGGIADCKKCSLKATSARAGPMVTCSECTNNNLSPLKDECMLGCPAGTYANNKVCTLCHESCAGCQTDDKETSCTACYPGSVLEHDGDLTTGKCIQECTGRYAENCEAGQCTAVVGGSKYCSRCKTGFVPINGMCVSTTARAATECVAGEGVCTSCTGAYFLESGGCYKTGAFPGNTLCIAAGANGKCANCANGQNADPQTGACPPCPANCSKCSGDSDVKTCTECYSGYYLDTGKECKKCSETSGNIQGVPNCVSCKAPSSPNAPTPVTCYVKTDATNNGDNDNNGGSTNKSGLSTGAIAGISVAVVVVVGGLVGFLCWWFICRGKA

SEQ ID NO: 52 - protein, 551 aa, Giardia; identical to SEQ ID NO: 51

SEQ ID NO: 53 - protein, 699 aa, Giardia
MLLLAPCLLISALAASCSGPTASKCKDGECDMIGKTEVCTQCKTETDHLIDGECVPAGTDQAAAKCASPAQGKCGSCGDGYFMYKGGCYEFAGELGGLICADPAGGATVGKVTGVCKDCVEGFFKSPVAAANKQSCISCNDTTGADQYQGVDQCKTCNPPSNTGPATCTACDEGYFGAGTTTCIACGDENCATCTEATTTKKCSKCKATGKMYLKKESGSLTGICVEGNQCSTDSTLYPDDTEPKSCKPCTAGTFENCKTCTKSDTSVTCTACKANMVFGLGKKSCISSCPDNSEAKTENTCTCNDGFKLNEEETQCVPNDSPSNPCSTQDCKACSGAQTNKEICTECLSNKYLTPTNQCIDHCEYILGYYSSTEGNKRVCKKCEVANCLACSENGGCGLCKDGFYGEACSPCDSSCKTCSGNTANDCTSCKSGSTLTYGSTGNTGTCGAECAAGTGTGKCRECGLTVEGTKYCSVCSQNNEYPQNGVCAVKASRTDKCKDGSITGGVCNVCADGFFKMNGGCYSTSQLPGSTVCLSAQSTGGICKTPEEGFSLTGESLVTCYTGCAECTTTKDCSRCMDGYVKVGSACTKCHESCYTCEAGATTCKVCAPGYYKESSSNGPCRKCSEGLAGCRQCATPVNGKFICFETDDNTGDNTGGSTNKSGLSTGAIAGISVAVIVVVGGLVGFLCWWFICRGKA

SEQ ID NO: 54 - protein, 699 aa, Giardia
MLLLAPCLLISALAASCSGPTASKCKDGECDMIGKTEVCTQCKTETDHLIDGECVPAGTDQAAAKCASPAQGKCGSCGDGYFMYKGGCYEFAGELGGLICADPVGGAASDKVIGVCKDCVEGFFKSPVAAANKQSCISCNDTTGADQYQGVDQCKTCTPPSNTGPATCTACDEGYFGAGTTTCTACGDENCATCTEATTTKKCSKCKATGKMYLKKESGSLTGICVEGNQCSTDSTLYPDDTEPKSCKPCTAGTFENCKTCTKSDTSVTCTACKANMVFGLGKKSCISSCPDNSEAKTENTCTCNDGFKLNEEETQCVPNDSPSNPCNTQDCKACSGAQTNKEICTECLSNKYLAPTSQCIDHCEYILGYYSSTEGNKRVCKKCEVANCLACSENGGCGLCKDGFYGEACSPCDSSCKTCSGNTANDCTSCKSGSALTYGSTGNTGTCGAECAAGTGTGKCRECGLTVEGTKYCSVCSQNNEYPQNGVCAVKVSRTDKCKDGSITGGVCNVCADGFFKMNGGCYSTSQLPGSTVCLSAQSTGGTCKTPKEGFSLTGESLVACYTGCAECTTTKDCSRCMDGYVKVGSACTKCHESCYTCEAGATTCKVCAPGYYKESSSNGLCKRCSEGLAGCRQCATPVNGKFICFETDDNTGDNTGGSTNKSGLSMGAIAGISVAVIVVVGGLVGFLCWWFLCRGKA

SEQ ID NO: 55 - protein, 720 aa, Giardia
MFQLIPLFVASALMAACQQDGNHLTTCAHEKCETVGSTEICTQCKAGGVPVDGFCRPFGSPQAAAAGCTKADGAALDKTATTCEKCGDGYFLFMGGCYKTTDGPGSEICTAASNGVCTTCKADNGLFKNPVTPQKPGSECILCSDTIDRNGVMGVAGCSECSHTGTSGPATCTECQAGFVTKDSACVKCGDGCSACSADTPTQCTACVEGKFLKDGNTCVEATECGADKYADKKTWTCKACDPDIAGCTACEYNDATGKPRCTNCGTNKTPRTTLDGTSTCVTKDYAGCKGADGALFMKEDKTCVLCSTVSAGADPNDQGIAGCKKCTKDSATPPTCSECLDGYYNSATGGSGTATCEACGDNCATCAKDTKDQCMTCKPGFFMKGSGPGTCVPCDDQTDGVPGCATCTFSSSLTCNSCKPNYKQSGTGPFTCTKTCEDPTACGGTSGACDAMIIDDQGTTKHYCSYCGETNKIPIDGKCVDSGSINGNTCAKGVCTQCAQGYFLYMGGCYKVASPPGNLMCTEATTAGVCDTPNANNKYFVVPEAKPTQQSVLACGNPLGTLVGTDSTAKAYVGVDGCSQCTAPTAPSEGGMTAATCTACTNNNKPNLAGSGCFPCTVSGCSHCNRDDMCEACSSGKKVSPGRKSCVDSCPSNSTDDNSVCVCNDGYSPDSSGTSCVSSGANRSGLSTGAIAGIAVAVVVVVGGLVGFLCWWFICRGKA

SEQ ID NO: 56 - protein, 394 aa, Giardia
MLVGFLLVCATVLAKDSGKDTCFPGYTLNTDTKQCTKDPEAPCNVEGCETCVEGNAQQCKTCRPGYTINTDTKQCTKDPEAPCNTPNCKTCDNPKTDSEICTECNDGNYLTPTNQCVPDCTTISGYYGDTDKKCKACNPECAECVGPANNQCSSCPAGKKLTYTDDSNPNNGGTCGDACKVSADGTGCETCGAQIGGTAYCSKCKTSTQAPLNGDCAASSRATFCTKMGNGVCTQCEDNYFLKDGGCYQTDRQPGKQVCSSAQGGNGKCQACANGLAATDGNCAECHPTCATCSTAGAADKCKTCATGYYKENGDDTTDGPCKKCSEKISGCKQCVSSSGSSVICLESEVGTGGSVNKSGLSTGAIAGIAVAVIVVVGGLVGFLCWWFLCRGKA

SEQ ID NO: 57 - protein, 616 aa, Giardia
MFGKIIFGIAILQVVWAAAETCTEATSDSQSGKCKQNMCNVWIGGSNFCSQCSTAAEHLVNGKCITTGEDAEGACTTKNDGTCTSCKAGFFLHRGGCYEMGSDIGLLVCNDRTATADKDGICIACHDGYFKNPASDADKTKESCIACNNTAGVDHNKGVQNCATCDAPKTPGQSSAEQTATCKSCVDGYYGTTSCQQCHADCRTCTGNGEDKCTSCKDTGKQYFKEGANSDGTGTCVDENGCGNTHFPIAEDKKCHLCGSVSEGGVADCKTCSKTGDSVKCLTCEGTKKPNEAGTGCFVCPMEHCEKCSKDNVCEACGSEKKLSPLGDACLDACPAGTRTDANVCNLCHESCASCSTNAEASCTACYPGYVLNRSSDDTGTCIKECTGDFMAHCKADGCSLNVGGSKYCDQCEEGYAPVDGVCTSIPATARDASGCKASGGKCTECGANYALLSGGCYNTQKLPGSSVCTAAQNKGQCQTCANGQTYADKNCPTCTEGCVKCAGSKETCTDCLAGYYKTIDNKCVKCTASSGDNNQITGVENCISCAPPAGGSGPVTCYVTQQKADDGTGGDTGGDSTNRSGLSTGAIAGISVAVVAVVGGLVGFLCWWFVCRGKA

SEQ ID NO: 58 - protein, 692 aa, Giardia
MFDKLIFASLALQLTWATQVKRMVRSATCDSTTSGSTKCAAEKCNVWIGGKDYCSQCSTDAELLIDGGCAPTTSDLAKKCISDNKGKCSSCGDGYFLHKGGCYKFGTAPGNAVCTEPSAPGDSLPAGVCTTCGSGYFKNPAESAASTPPCIACNDTAGNSGNTGLVGCGTCDPPVSGQATCTSCLDGFFGIGEGTVTCTECTGECKTCKGGADQCTSCKTSSKYLKITDSVAETGECIDQGQCTETHFAMVDGGINMCYLCNTTDKGGKVGCRTCTKSGTVTCKTCLDGFFGTTDCVACHEDCLTCKIEAAKCTSCKADTKPYFKEGADNDQTGTCVDEVECKGDHFSTIDTSNSDKKICVPCSKTDKGGITNCKTCAFKVSSTEERPAITCTECTTNNLSPLKDECMAACPAGTYANNKVCASCHSSCAGCQTDDRETSCTACYPGYSLLYEPNGATGRCVKECTGAFITNCADGQCTADVGGAKYCAQCKDGYAPIDGICTTMAAAGRDASVCTAAGGKCTACTGDYALVSGGCYGIQKLPGKAICIAANNGECTTCANGQQPSGKVCPTCPAGCSKCTGSAPSQQCSECFPGYYKSGDKCVKCDKDSENIKGVPNCVSCKEPANSSGAVTCYLTQQKTDDGTGGDTGGDSMNKSGLSTGAIAGISVAVIVVVGGLVGFLCWWFICRGKA

SEQ ID NO: 59 - protein, 737 aa, Giardia
MFGSFVLAGVLAQIAWAGKATERAAHCADNTNCAADACNVLIGGKLYCSRCNTGFVPINGQCADKEGATDKCKDGSGGDTADQTCGQCAEQTFMYKGGCYEAAQQPGQTMCQAADAGVCTQAAQGYFVPPGADASHQSVIPCGDEEEITVKNDKKYKGVLHCTRCNAPTEAADANAKAATCTACGDSKIVKTAKDSATSCVTEEECTGTEGFFVKNGGTKTCEACDPGCKTCKTEAAKCTSCKDDKPYLKKDNGSDTGTCVTEAECKTGNTHYPDDTEPKTCKTCAEGTSDGCATCEKGADGAVACKTCGSNKKVQPNKKGCIAKCPETVSAEKDGVCECVEGYVPDNAGTGCTKKPDPQCNTPGCKTCSEPKTSKEVCTECEDPKALTPTGQCIYGCEHLEGYYEGTSEGGKKACKKCEVENCLLCNGQGQCETCKDGYYKSGAACAKCNTSCKTCANGNSNGCTSCEPKQVLSYEGEGTGTCKPGCKPVSGGKDGTCKSCDLNIDGTSYCSACNVGTEYPENGVCVKKSARTASCQAEPSNGVCGTCARGFFRMNGGCYETTKLPGKSVCEEVASAGDTCQTPADGYKLNNGALITCSAGCKTCTSQDQCDTCKAGYAKDSGNTKKCVPCATGCSECNADDATKCTVCAAGYYLSKEKCIACDKSDGGSITGVANCASCTPPTNNKGSVLCYLIQNTNKSGLSAGAIAGISVAVIVVVAGLVGFLCWWFICRGKA

SEQ ID NO: 60 - protein, 239 aa, Giardia
MLLVPLYFILGVLTATCTGRAQNNCANNKCEMLGATEICTQCNAGYVPIGGVCTAHNDQAVVAGTGAGCQKTGDTAVDGGSTVCEKCTEANYFLFMGGCYKTGEAPGNLICTAAASGKCSACVENGNVFKNKNSSPTLGTECILCSDDTGSNNNKGVANCATCTAPSADSGTATCKTCLPEFALDGSANACISNSGTGGNVNKSGLSTGAIAGIAVAVVIVVGGLVGFLCWWFLCRGKA

SEQ ID NO: 61 - protein, 658 aa, Giardia
MFEKIIFGIAILQVVWAAAETCTVATSDPESKKCKQDKCDVWIGGSNFCSQCSTAAEHLVNGKCITTGEDAEGACTTKNDGTCTSCKAGFFLHRGGCYKIGTEPGNLICEDTQASQTQGVCEACSPGYFKNPTESLDKTKESCIACNQTTAIDENKGVQNCATCTIENPAGALRLGKTATCKTCFEGFFVASGGTACTACNDDNCATCVGAGNSKCTRCKLKSAGGNDKEYLKVTDASSNSGECVDTAGCPATHYVDEEAKECNTCVSGGTVDCTTCEKGANGVVCKTCTTGKKTIFGLNRKSCVASCPANSTPKATGQGSQMCECNEGLQPNTESTECQPISNCNTEHCLECTGEGADKEVCTKCLSEYYLTPTSQCVSDCTTLKGYYGNDTDRKCKKCNDACIECKGEGADKCTACPAGRMLQYTDADTPANGGTCMNQCSVSPANDGCAECGAQIGGTAYCSKCKNTQQAPLDGNCAANTRTRFCTTVSNGACTQCENNYFLKDGGCYQTDRQPGKQVCTTVQGGKCTKCASGLTADNGDCSNKRCHLSCETCTAANDANACATCSTGYYKPQSAGTKCNPCSEGLAGCRQCTVSSTGAFMCLEMGDGTGDNTGGSVNRGGLSTGAIAGISVAVVAVVGGLVGFLCWWFLCRGKA

SEQ ID NO: 62 - protein, 1983 aa, Giardia
MLAVILLACTTVLAGIVPKTACNPEIPGCATCTTTGSEQTCTSCATGGEKVRPDKKGCIPQCPPDVSTESGEFCECKSTHQPSPDGQTCVPKTGACNPEIPGCATCTTTGSEQTCTSCATGGEKVRPDKKGCIPQCPPDVSTESGEFCECKSTHQPSPDGQTCVPKTGACNPEIPGCATCTTTGSEQTCTSCATGGEKVRPDKKGCIPQCPPDVSTESGEFCECKSTHQPSPDGQTCVPKTGACNPEIPGCATCTTTGSEQTCTSCATGGEKVRPDKKGCIPQCPPDVSTESGEFCECKSTHQPSPDGQTCVPKTGACNPEIPGCATCTTTGSEQTCTSCATGGEKVRPDKKGCIPQCPPDVSTESGEFCECKSTHQPSPDGQTCVPKTGACNPEIPGCATCTTTGSEQTCTSCATGGEKVRPDKKGCIPQCPPDVSTESGEFCECKSTHQPSPDGQTCVPKTGACNPEIPGCATCTTTGSEQTCTSCATGGEKVRPDKKGCIPQCPPDVSTESGEFCECKSTHQPSPDGQTCVPKTGACNPEIPGCATCTTTGSEQTCTSCATGGEKVRPDKKGCIPQCPPDVSTESGEFCECKSTHQPSPDGQTCVPKTGACNPEIPGCATCTTTGSEQTCTSCATGGEKVRPDKKGCIPQCPPDVSTESGEFCECKSTHQPSPDGQTCVPKTGACNPEIPGCATCTTTGSEQTCTSCATGGEKVRPDKKGCIPQCPPDVSTESGEFCECKSTHQPSPDGQTCVPKTGACNPEIPGCATCTTTGSEQTCTSCATGGEKVRPDKKGCIPQCPPDVSTESGEFCECKSTHQPSPDGQTCVPKTGACNPEIPGCATCTTTGSEQTCTSCATGGEKVRPDKKGCIPQCPPDVSTESGEFCECKSTHQPSPDGQTCVPKTGACNPEIPGCATCTTTGSEQTCTSCATGGEKVRPDKKGCIPQCPPDVSTESGEFCECKSTHQPSPDGQTCVPKTGACNPEIPGCATCTTTGSEQTCTSCATGGEKVRPDKKGCIPQCPPDVSTESGEFCECKSTHQPSPDGQTCVPKTGACNPEIPGCATCTTTGSEQTCTSCATGGEKVRPDKKGCIPQCPPDVSTESGEFCECKSTHQPSPDGQTCVPKTGACNPEIPGCATCTTTGSEQTCTSCATGGEKVRPDKKGCIPQCPPDVSTESGEFCECKSTHQPSPDGQTCVPKTGACNPEIPGCATCTTTGSEQTCTSCATGGEKVRPDKKGCIPQCPPDVSTESGEFCECKSTHQPSPDGQTCVPKTGACNPEIPGCATCTTTGSEQTCTSCATGGEKVRPDKKGCIPQCPPDVSTESGEFCECKSTHQPSPDGQTCVPKTGACNPEIPGCATCTTTGSEQTCTSCATGGEKVRPDKKGCIPQCPPDVSTESGEFCECKSTHQPSPDGQTCVPKTGACNPEIPGCATCTTTGSEQTCTSCATGGEKVRPDKKGCIPQCPPDVSTESGEFCECKSTHQPSPDGQTCVPKTGACNPEIPGCATCTTTGSEQTCTSCATGGEKVRPDKKGCIPQCPPDVSTESGEFCECKSTHQPSPDGQTCVPKTGACNPEIPGCATCTTTGSEQTCTSCATGGEKVRPDKKGCIPQCPPDVSTESGEFCECKSTHQPSPDGQTCVPKTGACNPEIPGCATCTTTGSEQTCTSCATGGEKVRPDKKGCIPQCPPDVSTESGEFCECKSTHQPSPDGQTCVPKTGACNPEIPGCATCTTTGSEQTCTSCATGGEKVRPDKKGCIPQCPPDVSTESGEFCECKSTHQPSPDGQTCVPKTGACNPEIPGCATCTTTGSEQTCTSCATGGEKVRPDKKGCIPQCPPDVSTESGEFCECKSTHQPSPDGQTCVPKTGACNPEIPGCATCTTTGSEQTCTSCATGGEKVRPDKKGCIPQCPPDVSTESGEFCECKSTHQPSPDGQTCVPSNTNKSSGLSTGAIAGIAVAAVIVVGGLVGFLCWWFLCRGKA

SEQ ID NO: 63 - protein, 1029 aa, Giardia
MLVGFLLVCATVLAKYSGKTSSEAVANTNCAQELQNAGCKTCGPNDQTCLDCKTPGENVQLDKRSCGPTCPQNSSPNQNVCECNPGFNLNDRKDACEAVANTNCAQELQNAGCKTCGPNDQTCLDCKTPGENVQLDKRSCGPTCPQNSSPNQNVCECNPGFNLNDRKDACEAVANTNCAQELQNAGCKTCGPNDQTCLDCKTPGENVQLDKRSCGPTCPQNSSPNQNVCECNPGFNLNDRKDACEAVANTNCAQELQNAGCKTCGPNDQTCLDCKTPGENVQLDKRSCGPTCPQNSSPNQNVCECNPGFNLNDRKDACEAVANTNCAQELQNAGCKTCGPNDQTCLDCKTPGENVQLDKRSCGPTCPQNSSPNQNVCECNPGFNLNDRKDACEAVANTNCAQELQNAGCKTCGPNDQTCLDCKTPGENVQLDKRSCGPTCPQNSSPNQNVCECNPGFNLNDRKDACEAVANTNCAQELQNAGCKTCGPNDQTCLDCKTPGENVQLDKRSCGPTCPQNSSPNQNVCECNPGFNLNDRKDACEAVANTNCAQELQNAGCKTCGPNDQTCLDCKTPGENVQLDKRSCGPTCPQNSSPNQNVCECNPGFNLNDRKDACEAVANTNCAQELQNAGCKTCGPNDQTCLDCKTPGENVQLDKRSCGPTCPQNSSPNQNVCECNPGFNLNDRKDACEAVANTNCAQELQNAGCKTCGPNDQTCLDCKTPGENVQLDKRSCGPTCPQNSSPNQNVCECNPGFNLNDRKDACEAVANTNCAQELQNAGCKTCGPNDQTCLDCKTPGENVQLDKRSCGPTCPQNSSPNQNVCECNPGFNLNDRKDACEAVANTNCAQELQNAGCKTCGPNDQTCLDCKTPGENVQLDKRSCGPTCPQNSSPNQNVCECNPGFNLNDRKDACEAVANTNCAQELQNAGCKTCGPNDQTCLDCKTPGENVQLDKRSCGPTCPQNSSPNQNVCECNPGFNLNDRKDACEAVANTNKSSGLSTGAIAGIAVAAVIVVGGLVGFLCWWFLCRGKA

SEQ ID NO: 64 - protein, 842 aa, Giardia
MFDKLIFVSLALQMALASQTASKAKTNPTPCAAANPGATNCAADSCNVEIGGQTFCSKCTGDKVPVNGECKAKTDAGMCTVGTNDKAGTCTACTNAHYLYKGGCYAECPDGTQKNEGRNTCDEVAPAGPTPCAAANPGATNCAADSCNVEIGGQTFCSKCTGDKVPVNGECKAKTDAGMCTVGTNDKAGTCTACTNAHYLYKGGCYAECPDGTQKNEGRNTCDEVAPAGPTPCAAANPGATNCAADSCNVEIGGQTFCSKCTGDKVPVNGECKAKTDAGMCTVGTNDKAGTCTACTNAHYLYKGGCYAECPDGTQKNEGRNTCDEVAPAGPTPCAAANPGATNCAADSCNVEIGGQTFCSKCTGDKVPVNGECKAKTDAGMCTVGTNDKAGTCTACTNAHYLYKGGCYAECPDGTQKNEGRNTCDEVAPAGPTPCAAANPGATNCAADSCNVEIGGQTFCSKCTGDKVPVNGECKAKTDAGMCTVGTNDKAGTCTACTNAHYLYKGGCYAECPDGTQKNEGRNTCDEVAPAGCNLPNCEVCSEDKQKCTKCQSNYFLTPEKNACLGSCPAGTYLSGQTCAPCDPSCAECSGAGASKCTACPAGKMLRYADETKLNEGGQCVEQCVEGPECETCGLTIGGTKYCSKCKGSNVPLNGVCTSNAARTRFCTTAANGACTVCAAGYFIQEGGCYETTRQPGKQVCALTDNKGKCQTCTNSLGPDGAGTCPSCDPTCKTCSAANTANTCTTCATGYYKTALEGACTSCENSNGDITGVKDCLNCAPPPNNKGSVLCYLMKDGDSTGGSVNKSGLSTGAIAGISVAVIVVVGGLVGFLCWWFLCRGKA

SEQ ID NO: 65 - protein, 168 aa, Giardia
MLYLVGLAFAYLALADPKSCTNSQNCASGDNCLDVNMNGSPTEVCTKCEPNNVPINGACQLCGEGHYLYSGGCYAACPQGTPNPETNTCDGVPTPDCNLPNCKSCPDGTCTECNDGFVPSNGSECVSSSVNKSELSTGAIAGIAVAVIVVVGGLVGFLCWWFLCRGKA

SEQ ID NO: 66 - protein, 1602 aa, Giardia
MLIGFLLVCATVLAKNSGKTACVAASNTACAAALDTAGCKTCGPDAQTCLDCKTPGENVQLDKRSCKANCPQNSSPNQNVCECDPGFSLNNGKDACEAVANVNCAAALDTAGCKTCGPDAQTCLDCKTPGENVQLDKRSCKANCPQNSSPNQNVCECDPGFSLNNGKDACEAVANVNCAAALDTAGCKTCGPDAQTCLDCKTPGENVQLDKRSCKANCPQNSSPNQNVCECDPGFSLNNGKDACEAVANVNCAAALDTAGCKTCGPDAQTCLDCKTPGENVQLDKRSCKANCPQNSSPNQNVCECDPGFSLNNGKDACEAVANVNCAAALDTAGCKTCGPDAQTCLDCKTPGENVQLDKRSCKANCPQNSSPNQNVCECDPGFSLNNGKDACEAVANVNCAAALDTAGCKTCGPDAQTCLDCKTPGENVQLDKRSCKANCPQNSSPNQNVCECDPGFSLNNGKDACEAVANVNCAAALDTAGCKTCGPDAQTCLDCKTPGENVQLDKRSCKANCPQNSSPNQNVCECDPGFSLNNGKDACEAVANVNCAAALDTAGCKTCGPDAQTCLDCKTPGENVQLDKRSCKANCPQNSSPNQNVCECDPGFSLNNGKDACEAVANVNCAAALDTAGCKTCGPDAQTCLDCKTPGENVQLDKRSCKANCPQNSSPNQNVCECDPGFSLNNGKDACEAVANVNCAAALDTAGCKTCGPDAQTCLDCKTPGENVQLDKRSCKANCPQNSSPNQNVCECDPGFSLNNGKDACEAVANVNCAAALDTAGCKTCGPDAQTCLDCKTPGENVQLDKRSCKANCPQNSSPNQNVCECDPGFSLNNGKDACEAVANVNCAAALDTAGCKTCGPDAQTCLDCKTPGENVQLDKRSCKANCPQNSSPNQNVCECDPGFSLNNGKDACEAVANVNCAAALDTAGCKTCGPDAQTCLDCKTPGENVQLDKRSCKANCPQNSSPNQNVCECDPGFSLNNGKDACEAVANVNCAAALDTAGCKTCGPDAQTCLDCKTPGENVQLDKRSCKANCPQNSSPNQNVCECDPGFSLNNGKDACEAVANVNCAAALDTAGCKTCGPDAQTCLDCKTPGENVQLDKRSCKANCPQNSSPNQNVCECDPGFSLNNGKDACEAVANVNCAAALDTAGCKTCGPDAQTCLDCKTPGENVQLDKRSCKANCPQNSSPNQNVCECDPGFSLNNGKDACEAVANVNCAAALDTAGCKTCGPDAQTCTACTEASNNVQIDKKSCKADCPSNSAANGQHVCECAVGYQPTPGQNQCEKAPNTQCNTPNCKTCDNPKTDNEICTECNDGNYLTPTKQCTQSCGAIGSYYNGDKVCEPCDPSCAGCTTKGPAKCTACPPGKMLKYTNDDPNQGGSCVDECKAEMDGCAECGAVIGGTKYCSKCKEDKWAPQNGVCANSVTRNSFCTNAAGGVCTQCAADHFLQDGGCYKLGRQPGVQICAAAGPNSLCTTCVNGQRPDTNTGACPVCPTGCDTCTGTSSRAPECQSCLLGYYFDSDKKLCVKCTENSSAIQGVSSCVSCSPPSNNQGSVVCYLINDSGSTNKSSRLSTGAIAGISVAVVVVVGGLVGFLCWWFLCRGKA

SEQ ID NO: 67 - protein, 627 aa, Giardia
MLLVAFYFVLSALAAACKQAQNCANERCEMVGETEICTECKDQGNVPVNGVCMPKDNDAVTTAGCKKNGGADLGAEDKVCGQCDGVHFLYKGGCYSTADATGQKLCTDAAEGVCSAAAVGYFIPPGAQKTDQSVILCGDVTEITLTNGKKYKGVQHCTVCTAPEAAESTAKPAVCTACDEGFFAASEGTCTACADNNNCAKCDAGADKCTKCKATAANKYFKDSGDGTGTCVNEQTCKEQSTHFPKDDPNNGNKCLSCSDDKSGGIADCKTCTPKENSEGPILITCSACATDTNKPNVAGTKCIACTVKDCKKCNDDGTCAECDNTRKLTPTKECVDKCEKLEGYFDGDDGTCRACNSVCKTCNGEDPYQCTGCPAKKVLKYTVESTPDSGSTCVDECTTNTNGCAECGATIGEAKYCSKCSDAKQAPLNGNCTASVRAAASCTQIENGICKKCATNYFLFEGGCYETTRQPGMQICKDAAGNDGKCKTCANNLPSNIDTGACPSCPAGCATCTAAGQTYTCQTCLAGYYLDSTKNLCIKCTESSGNIQGVTNCVSCNPPAGNSGPVTCYVKKDGTSDGGNDNSTGGSTNKSGLSTGAIAGISVAVIVVVGGLIGFLCWWFICRGKA

SEQ ID NO: 68 - protein, 736 aa, Giardia
MFGSFVLAGVLVQIAWAEKVTERAAQCADNTNCAAEACNVLIGGKLYCSQCNTGFVPINGQCAGKEDAKTKCKDTDGGDTADQTCGQCAEQTFMYKGGCYEAAQQPGQTICQAAENGKCTQAKAGYFVPPGADASHQSVIPCGDEEEITVKNDKKYKGVVHCTQCNAPAEAADANAKAATCTACGDSKIVKTAKDQATSCVTEKECTDAPGFFVDTTSGKKCSKCAETCKTCKTEAAKCTSCKDDKPYLKKDDESTTGTCVDANGCPATHYVDKEAKECNTCVSGGTVDCTTCEKGANGVVCKTCTTGTKTKFGLGKKSCVENCPSNSSDEKTPGTCECVEGYVPDDAGTGCTKKSDPQCNTPGCKTCSDPKKDKEVCTECEDPKALTPTGQCIDNCGDLGGYYEGTNEGGKKACKKCEVENCLLCNGQGQCETCKDGYYKSGAACAKCDTSCKTCANGKPNGCTSCEPKQVLSYEGEGTGTYKPECKPVSGGKDGTCKSCDLSIDGTSYCSACNVGTEYPENGVCVKKSARTASCQVEPSNGVCGTCAKGFFRMNGGCYETTKLPGKNVCEEAAPTGDTCQTPADGYKLNNGALITCSAGCKTCTSQDQCDTCKAGYAKTGGNTKKCVPCATGCSECNADDATKCTVCAAGYYLSKEKCIACDKSDGGSITGVANCANCAPPTNNKGPVLCYLIQNTNRSGLSTGAIAGISVAVIAVVGGLVGFLCWWFICRGKA

SEQ ID NO: 69 - protein, 793 aa, Giardia
MLVGFLLVCATVLAKDTGKTACELSNTECAQNLKDAGCKTCVGTEPDQTCTECTDPSHNVQIDKKSCDANCPEHAAANSKVCGCVAGYQPTPGQNQCELSNTECAQNLKDAGCKTCVGTEPDQTCTECTDPSHNVQIDKKSCDANCPEHAAANSKVCGCVAGYQPTPGQNQCELSNTECAQNLKDAGCKTCVGTEPDQTCTECTDPSHNVQIDKKSCDANCPEHAAANSKVCGCVAGYQPTPGQNQCELSNTECAQNLKDAGCKTCVGTEPDQTCTECTDPSHNVQIDKKSCDANCPEHAAANSKVCGCVAGYQPTPGQNQCELSNTECAQNLKDAGCKTCVGTEPDQTCTECTDPSHNVQIDKKSCDANCPEHAAANSKVCGCVAGYQPTPGQNQCELSNTECAQNLKDAGCKTCVGTEPDQTCTECTDPSHNVQIDKKSCDANCPEHAAANSKVCGCVAGYQPTPGQNQCEKAPNTQCNTPNCKTCDNPKTDNEICTECNDGNYLTPTKQCTQSCGTIGSYYDGDKACEPCDPSCAGCTTKGPAKCTLCPPGKRLQYTNDDPNQGGSCVDECKAEMDGCAECGAIIGGTKYCSKCKEDKWAPQNGVCANSVTRNSFCTNAAGGVCTQCAADHFLQDGGCYKLGRQPGVQICAAAGPNSLCTTCVNGQRPDTNTGACPVCPTGCDTCTGTSSRAPECQSCLLGYYFDSDKKLCVKCTENSSAIQGVSSCVSCAPPSNNQGSVVCYLINDSGSTNKSSGLSTGAIAGISVAVVVVVGGLVGFLCWWFLCRGKA

SEQ ID NO: 70 - protein, 531 aa, Giardia
MLVGIGLIFAVALTEVCSPSIDGCAECDSTGQGCTKCDANGNTPYLKKTNPSDPTGTCVSAVDCQGSAGYYTDDSVSDAKECKKCAEGQKPNTAGTQCFSCSDANCERCDQNDVCARCSTGAPPENGKCPAATPGCHSSCDGCTENAMTNQADKCTGCKEGRYLKPESAAGQSGTCLTAEECTSDTTHFTKEKAGDSKGMCLPCSDATHGIAGCKKCALKTLSGEAESTVVCSECTDKWLTPSGNACLDNCPAGTYPNDNNLCTSCHDTCEECNGNADAASCTACYPGYSLLYGSGTAGTCVKECTGAFGANCADGQCTADVGGAKYCAQCKDGYAPIDGICTAVAAAGRTNVCTAADGKCTKCAGEYTLMSGGCYGVAKLPGKSVCTLASNGKCIMCAANGQAPVQEKCPECSEGCAKCNDSNACTECLPGYYKGAGDKCFKCTASSGNNNQITGVANCVSCAPPAGGSGSVTCYVKTDGTSGGDDNTGGSVNKSGLSTGAIAGIAVAVVVVVGGLVGFLCWWFICRGKA

SEQ ID NO: 71 - protein, 409 aa, Giardia
MFEKILLGIAILQMARASTCQAQSGGDPGTCEKCDALIGQTKYCSKCNGANYAPVNGACEDVETQEDKKALCKAHASGACTTCGGASFMYKDGCYSKDTEPGQSMCTQASEGKCTEAAPGYFAPVGAANTEQSVVACGDTTGVTIAAGGNTYKGIADCAECGAPDATAGAEAGKVATCTKCGVSKYLKDNTCVDKAQCDSGNTNKLVAVDDPENGNKCVSCSDNLNGGVANCDTCSYDEQSKKIKCTKCTDNNYLKTTSEGTSCVQKDQCKDGFFPKDDSSAGNKCLPCNDSTDGIANCATCALVSGRSGAALVTCSACIDGKRPNKEGAACFECNMEGCVYCSGANKCEECSDGFKLEGDKCVSSGSAGVNKSGLSTGAIAGISVAVIAVVAGLVGFLCWWFVCRGKA

SEQ ID NO: 72 - protein, 1480 aa, Giardia
MLVVELLFVLNVLAANCAGGTRNSRATGNQCGTIEGISSPMECAEGHALDEAANACRAPPSFQCEVDKLVTIGSAQACTQCKQGFAPIDGVCTAFGDDLVTKTAKCTQSGGAAIEGTDTSCGKCGGDGYFLFMGGCYKTGASPGELICTNAVGGVCAACKADGSVFQNKASVKTPGSECILCSDSVGADSNKGVANCAACDAPTGDTGTAKCKACAEGHALDEAANACRAPPSFQCEVDKLVTIGSAQACTQCKQGFAPIDGVCTAFGDDLVTKTAKCTQSGGAAIEGTDTSCGKCGGDGYFLFMGGCYKTGASPGELICTNAVGGVCAACKADGSVFQNKASVKTPGSECILCSDSVGADSNKGVANCAACDAPTGDTGTAKCKACAEGHALDEAANACRAPPSFQCEVDKLVTIGSAQACTQCKQGFAPIDGVCTAFGDDLVTKTAKCTQSGGAAIEGTDTSCGKCGGDGYFLFMGGCYKTGASPGELICTNAVGGVCAACKADGSVFQNKASVKTPGSECILCSDSVGADSNKGVANCAACDAPTGDTGTAKCKACAEGHALDEAANACRAPPSFQCEVDKLVTIGSAQACTQCKQGFAPIDGVCTAFGDDLVTKTAKCTQSGGAAIEGTDTSCGKCGGDGYFLFMGGCYKTGASPGELICTNAVGGVCAACKADGSVFQNKASVKTPGSECILCSDSVGADSNKGVANCAACDAPTGDTGTAKCKACAEGHALDEAANACRAPPSFQCEVDKLVTIGSAQACTQCKQGFAPIDGVCTAFGDDLVTKTAKCTQSGGAAIEGTDTSCGKCGGDGYFLFMGGCYKTGASPGELICTNAVGGVCAACKADGSVFQNKASVKTPGSECILCSDSVGADSNKGVANCAACDAPTGDTGTAKCKACAEGHALDEAANACRAPPSFQCEVDKLVTIGSAQACTQCKQGFAPIDGVCTAFGDDLVTKTAKCTQSGGAAIEGTDTSCGKCGGDGYFLFMGGCYKTGASPGELICTNAVGGVCAACKADGSVFQNKASVKTPGSECILCSDSVGADSNKGVANCAACDAPTGDTGTAKCKACAEGHALDEAANACRAPPSFQCEVDKLVTIGSAQACTQCKQGFAPIDGVCTAFGDDLVTKTAKCTQSGGAAIEGTDTSCGKCGGDGYFLFMGGCYKTGASPGELICTNAVGGVCAACKADGSVFQNKASVKTPGSECILCSDSVGADSNKGVANCAACDAPTGDTGTAKCKACAEGHALDEAANACRAPPSFQCEVDKLVTIGSAQACTQCKQGFAPIDGVCTAFGDDLVTKTAKCTQSGGAAIEGTDTSCGKCGGDGYFLFMGGCYKTGASPGELICTNAVGGVCAACKADGSVFQNKASVKTPGSECILCSDSVGADSNKGVANCAACDAPTGDTGTAKCKACAEGHALDEAANACVSSGGAGGSVNKGGLSTGAIAGITVAVVVVVGGLAGFLCWWFICRGKA

SEQ ID NO: 73 - protein, 680 aa, Giardia
MFQLIPLFVASALMAACQPDGNHTATCAQNKCETVGSAEICTECRAGGVPVDGFCRPPGSPQAAAAGCTQADGTALDKTATTCEKCGDGYFLFMGGCYKTTDGPGSEICTAASNGVCTTCKADNGLFKNPATAPEKGRECILCHDATGADGYMGVEGCATCTAPTNNKGAATCTECQDGYYNDGGACKKCVDGCIDCTGANQCTTCEDGKYLKNNQCVDAGQCDQGTYADPTTGQCKPCGITDCATCEYNATISQPQCKTCSTSSNKMVKTAADGTTTCVDDGGCTNGNTHFVEGTNQKLCVPCGDTTNGGVLGCSTCSSKTTCTKCLDGYYDNDDSQDTATCVACGGQNCETCAKATSDKCTTCKPGFFLKDSSSGECISCSDTANGGREGCSVCSNDSGFKCTDCKPNYKKQLNGGADDDYTCVKTCEDDTACGGTSGACDAIVINENGKELHYCSYCGDNSKYPIDGKCTNVNAGNTGCTNNVCKSCTAGYFLYMGGCYKIGAEPGNLMCKTAEGGKCTAVNANNRYFVVPEAQATDQSVLACGNPLGTLVGTDSTSKAYVGVDGCSQCTAPVALTEAGMAAATCTSCDSDKVPNKDGTGCVLCSVGDCKHCVVDDVCGECSDGYSLDSSGASCVSSSSNRSGLSTGAIAGISVAVIAVVGGLVGFLCWWFLCRGKA

SEQ ID NO: 74 - protein, 1181 aa, Giardia
MLVGIGLIFAVALADACSPSIDGCAECDSTGKKCTKCDANGNTPYLKKTNPSDPTGTCVSAVDCQGSAGYYTDDSVSDAKECKKCNAPCTACAGTADKCTKCDANGAAPYLKKTNPSDPTGTCVSAVDCQGSAGYYTDDSVSDAKECKKCNAPCTACAGTADKCTKCDANGAAPYLKKTNPSDPTGTCVSAVDCQGSAGYYTDDSVSDAKECKKCNAPCTACAGTADKCTKCDANGAAPYLKKTNPSDPTGTCVSAVDCQGSAGYYTDDSVSDAKECKKCNAPCTACAGTADKCTKCDANGAAPYLKKTNPSDPTGTCVSAVDCQGSAGYYTDDSVSDAKECKKCNAPCTACAGTADKCTKCDANGAAPYLKKTNPSDPTGTCVSAVDCQGSAGYYTDDSVSDAKECKKCNAPCTACAGTADKCTKCDANGAAPYLKKTNPSDPTGTCVSAVDCQGSAGYYTDDSVSDAKECKKCNAPCTACAGTADKCTKCDANGAAPYLKKTNPSDPTGTCVSAVDCQGSAGYYTDDSVSDAKECKKCNAPCTACAGTADKCTKCDANGAAPYLKKTNPSDPTGTCVSAVDCQGSAGYYTDDSVSDAKECKKCNAPCTACAGTADKCTKCDANGAAPYLKKTNPSDPTGTCVSAVDCQGSAGYYTDDSVSDAKECKKCNAPCTACAGTADKCTKCDANGAAPYLKKTNPSDPTGTCVSAVDCQGSAGYYTDDSVSDAKECKKCAEGQKPNTAGTQCFSCSDANCERCDQNDVCARCSTGAPPENGKCPAATPGCHSSCDGCTENAMTNQADKCTGCKEGRYLKPESAAGQSGACLTAEECTSDKTHFTREKAGDSKGMCLSCSDATHGITGCKKCALKTLSGEAESTVVCSECTDKRLTPSGNACLDNCPAGTYADNINGVSVCASCHATCAECNGDANAASCTACYPGYSLLYGSGTAGTCVKECTGAFITNCADGQCTANVGGAKYCAQCKDGYAPIDGICTTVAAAGRDASVCTAADGKCTKCAGEYTLMSGGCYGVAKLPGKSVCTLASNGKCTMCAANNQAPVQEKCPECSEGCAKCNDSNACTECLPGYYKGAGDKCFKCTASSGNNNQITGVANCVSCAPPAGGNGGPVTCYIKTDGDNTGGSVNKSGLSTGAIAGISVAVVVVVGGLVGFLCWWFICRGKA

SEQ ID NO: 75 - protein, 864 aa, Giardia
MLVGFLLVFTVTQAHRTSVSTDCPIVNCQTCSQDKQTCVACKQGFVPNEGNTECNSAPAECPIVNCQTCSQDKQTCVACKQGFVPNEGNTECNSAPAECPIVNCQTCSQDKQTCVACKQGFVPNEGNTECNSAPAECPIVNCQTCSQDKQTCVACKQGFVPNEGNTECNSAPAECPIVNCQTCSQDKQTCVACKQGFVPNEGNTECNSAPAECPIVNCQTCSQDKQTCVACKQGFVPNEGNTECNSAPAECPIVNCQTCSQDKQTCVACKQGFVPNEGNTECNSAPAECPIVNCQTCSQDKQTCVACKQGFVPNEGNTECNSAPAECLIVNCQTCSQDKQTCVACKQGFVPNEGNTECNSAPAECPIVNCQTCSQDKQTCVACKQGFVPNEGNTECNSAPAECLIVNCQTCSQDKQTCVACKQGFVPNEGNTECNSAPAECPIVNCQTCSQDKQTCVACKQGFVPNEGNTECNSAPAECPIVNCQTCSQDKQTCVACKQGFVPNEGNTECNSAPAECLIVNCQTCSQDKQTCVACKQGFVPNEGNTECNSAPAECPIVNCQTCSQDKQTCDACEPGKHLTPTKKACLTDCPAGTYLSGQTCAPCDPSCAECSGAGASRCTACPAGKMLRYADESKLNEGGQCVEQCVEGPECETCGLTIGGTKYCSKCKGNNVPLNGVCTSNAARTQFCTTAADGACTVCAAGYFVQGGGCYEITRQPGKQVCALTDNKGKCQTCTNSLGPDGAGTCPSCDPTCKTCSAANAANTCTTCATGYYKIALEGACTSCENDSNGITGVKGCLNCAPPPSNTGPVLCYLMKDGDSTGGNVNKSGLSTGAIAGISVAVIVIVGGLVGFLCWWFICRGKA

SEQ ID NO: 76 - protein, 385 aa, Giardia
MLLPALCFLMSGLAAQRTKQPAPSCQVDNCEQCNADNVHCDRCVPSDDTKCERCNEGFTVSDDKTVCNQSPAQCNTPNCKTCDNPKTDNEICTKCNDGDYLTPTNQCVPDCTAISGYYGDTDKKCKACNPECAECVGPANNQCTACPVGKMLQYTDTNTPVNGGTCMDQCSVSSTNDGCAECGAQIGGTAYCSKCKNTQQAPLNGNCAASSRVAFCATITSGACTKCNEGYFLKDGGCYQTDRQPGKQVCSNAQGGNGKCQTCANGLAASDGNCAECHSTCATCSTADAADKCKTCATGYYKENGDDTTAGLCKKCSEKISGCKQCVSSSGSSVICLESEVGTGGSVNKSGLSTGAIAGISVAVIVIVGGLVGFLCWWFLCRGKA

SEQ ID NO: 77 - protein, 1154 aa, Giardia
MLVGFLLVCATVLAKDSGKDTCFPGYTLNTDTKQCTKDPEAPCNVEGCETCVEGNAQQCKTCRPGYTINTDTKQCTKDPEAPCNVEGCETCVEGNAQQCKTCRPGYTINTDTKQCTKDPEAPCNVEGCETCVEGNAQQCKTCRPGYTINTDTKQCTKDPEAPCNVEGCETCVEGNAQQCKTCRPGYTINTDTKQCTKDPEAPCNVEGCETCVEGNAQQCKTCRPGYTINTDTKQCTKDPEAPCNVEGCETCVEGNAQQCKTCRPGYTINTDTKQCTKDPEAPCNVEGCETCVEGNAQQCKTCRPGYTINTDTKQCTKDPEAPCNVEGCETCVEGNAQQCKTCRPGYTINTDTKQCTKDPEAPCNVEGCETCVEGNAQQCKTCRPGYTINTDTKQCTKDPEAPCNVEGCETCVEGNAQQCKTCRPGYTINTDTKQCTKDPEAPCNVEGCETCVEGNAQQCKTCRPGYTINTDTKQCTKDPEAPCNVEGCETCVEGNAQQCKTCRPGYTINTDTKQCTKDPEAPCNVEGCETCVEGNAQQCKTCRPGYTINTDTKQCTKDPEAPCNVEGCETCVEGNAQQCKTCRPGYTINTDTKQCTKDPEAPCNVEGCETCVEGNAQQCKTCRPGYTINTDTKQCTKDPEAPCNVEGCETCVEGNAQQCKTCRPGYTINTDTKQCTKDPEAPCNVEGCETCVEGNAQQCKTCRPGYTINTDTKQCTKDPEAPCNVEGCETCVEGNAQQCKTCRPGYTINTDTKQCTKDPEAPCNVEGCETCVEGNAQQCKTCRPGYTINTDTKQCTKDPEAPCNVEGCETCVEGNAQQCKTCRPGYTINTDTKQCTKDPEAPCNTPNCKTCDNPKTDNEICTKCNDGDYLTPTNQCVPDCTAISGYYGDTDKKCKACNPECAECVGPANNQCTACPVGKMLQYTDTNTPVNGGTCMDQCSVSSTNDGCAECGAQIGGTAYCSKCKNTQQAPLNGNCAASSRVAFCATITSGACTKCNEGYFLKDGGCYQTDRQPGKQVCSNAQGGNGKCQTCANGLAASDGNCAECHSTCATCSTADAADKCKTCATGYYKENGDDTTAGLCKKCSEKISGCKQCVSSSGSSVICLESEVGTGGSVNKSGLSTGAIAGISVAVIVIVGGLVGFLCWWFLCRGKA

SEQ ID NO: 78 - protein, 740 aa, Giardia
MFGSFIFAGLAIQIAWAEKVAERAREAHCANNANCAANACNVLIGGKLYCSQCNTGFVPINGKCVGKDDVTDKCTAADGNTASDETCAKCAGQTFMYKGGCYEQAIEPGNVMCGGAAGGKCTQATEGYFLPPGADNAHDSVVSCGDSIGVTLTGNKKYTGVDGCTACDGLQLTVEASGVAKCTACGPDAQQTARIVKTDGDVTSCVTEHECTSTAGFFVDATGSKKCTKCAETCKTCETEATKCTSCNEDKPYLKKAQSQDQAGECVTEEACTSGNTHYADDEEPKTCKPCTAGTFENCKTCTKSDTSVTCTACKENMVFGLGKKSCISSCPDNSEAKTENTCTCNDGFKLDEEETQCVPNDSPSNPCSTQDCKACSGAQTNKEICTECLSNKYLTPTNQCIDHCEYILGYYSSTEGNKRVCKKCEVANCLACSENGGCGLCKDGFYGEACSPCDSSCKTCSGNTANDCTSCKSGSALTYGSTGNTGTCGAECAAGTGTGKCRECGLTVEGTKYCSVCSQNNEYPQNGVCAVKTSRTDKCKDGSITGGVCNVCADGFFKMNGGCYSTSQLPGSTVCLSAQSTGGTCKTPEEGFSLTGESLVACYTGCAECTTTRDCSRCMDGYVKVGSACTKCHESCYTCEADATTCKVCTPGYYKESSSNGPCRKCSEGLAGCRQCATPVNGKFICFETDDNTGDNTGGSTNKSGLSTGAIAGISVAVIVVVGGLVGFLCWWFICRGKA

SEQ ID NO: 79 - protein, 689 aa, Giardia
MFQLIPLFVASALMAACQPDGDHAATCQTGKCETVGSAEICTECKTGGVPVDGFCRPFGSPQAAAAGCTKAGGAALDKMTATCEKCGDGYFLFMGGCYKTTDGPGSEICTKAEGGLCTECKTANGLFKNPAATPEKGSECILCSDINGADGYTGVANCAQCTKSDSNKGAATCTACQAGYYKDFQACSKCDGTCLTCETSAAQCTSCPEGKYLKGDKSCVNNNGCTGNTYADPESGKCLPCNTIDQACTQCEVDSTTKKPKCTNCGGQKMVKTAIDGTTTCVDANGCATSNVDGSHFLNDGSTKCILCSDDSESLEANKGTPGCKTCKKNGAKPTCSECLDGYYNSGNGGTVTCEACGANCATCTQAGNDKCTKCKPGFFMKGNGPTGECVACDNAQGGIDGCAECTKESTGPLKCTKCKPNRKPAGTSDNYTCTEKTCEDPTACGGTAGSCDAIVIDDQGTTKHYCSYCGDSSQAPIDGLCASEAQKAGNTCANGVCTQCTNNYFLYMGGCYSTQKAPGSFMCKTAGNTGICTEAANNRYFVVPGASNTDQSVLACSNPLGTLTGTGDTAKAYVGVEGCSQCTAPAALSDGGMAPAVCTSCDSSKKPNRDGSGCVLCSVGGCKSCVMDNICGECNSGFSLDNGKCVSSGANRSGLSAGAIAGISVAVVAVVGGLVGFLCWWFVCRGKA

SEQ ID NO: 80 - protein, 747 aa, Giardia
MFCRFVLAGVILQFVWTAQIAEKAGTATCADQTTNCADEACNVLIDGKLYCSQCKADPADRAPVNGVCTDVSSDTAVCKTHAGGKCTGCNGNSFMYKGGCYERAKPPGNAMCQAADAGKCTEAVAGNKYFVPPADTDDAHDSVVSCGDATGVTLTGDKIYTGVAGCATCEKPEQLSASGTKAATCTACQEGKYLKTATDSATSCVTEEECTGTEGFFVKNGGTKTCEACDPGCKTCKTEAAKCTSCKDDKPYLKKDNGSDTGTCVTETECKNQSTHYADDTEPKTCKACAEGTSNGCATCEKGADGAVACKTCENQKKVQPNKKGCVESCPLNSNEEKTSGVCECVEGYVPEEAGTGCMKKSDPPAAPCNTPGCKTCSEPKTSKEVCTECEGTKALTPTGQCIDACGDLGGYYAGTNEGGKKACKKCEVENCLLCNGQGQCETCKDGYYKKETACAKCDTSCKTCANGNSNGCTSCEPKKALSYEGEGNTGTCKPGCEPNANNCEKCELTVDGTAYCSKCKEAGQFPQNGVCSAAAGKAITCTTKGTGVCDKCANGLLRMNGGCYETTKFPGKSVCLAAAEASDACQTPADGYKLNNGALITCSAGCKTCTSQDQCDTCKAGYAKTGGNTKKCVPCATECSECNANDATKCTVCAAGYYPSKEKCIACDKSDGGSITGVANCASCAPPSAGSGSVLCYLMNGESTGGSTNKSGLSTGAIAGISVAAVVIVAGLVGFLCWWFICRGKA

SEQ ID NO: 81 - protein, 741 aa, Giardia
MFGSFIFAGLAIQIAWAEKVAEHVREVQCADNTNCAADACNVLIGDKLYCSQCDAGSVPINGKCVGKDGATDKCKDSSGGNTADQTCGQCAGQTFMYKGGCYEAAQQPGQTMCTQASEGKCTQAAQGYFVPPGADVSHQSVIPCGDATGITLGDKTYTGVAGCTTCDGSALTSQANGVAKCTACGPDAQQTARIVKTDGGATSCVTEQECTGTEGFFVDTTGGKKCSKCAETCKTCKTGAAKCTSCKDDKPYLKKDDESTTGTCVDANGCPATHYVDKEAKECNTCASGGTVDCATCEKGPTGVVCKTCGPNKKIQPNKKGCVESCPLNSNEEKTSGVCECVEGYVPDNAGTGCTKKSDPQCNTPGCKTCSEPKTSKEVCTECEGTKALTPTGQCIDNCGDLGGYYAGTNEGGKKACKKCEVENCLLCNENGQCDTCKDGYYKSGAACAKCDTSCKTCANGNSNGCTSCEPKKALSYEGEGNTGTCKPGCEPNANNCEKCELTVNGTAYCSKCKDAGQFPQNGVCSAAAGKAITCTTQGSGVCNKCANGLLRMNGGCYETTKFPGKSVCLAAAEASDACQTPADGYKLDNGALTTCSAGCKTCTSQDQCDTCKAGYAKTGGNTQKCVPCATGCSECNANDATKCTVCAAGYYLSKEKCIACDKSDGGSITGVANCASCAPPSAGSGSVLCYLIKDGDSTDGSTNKSGLSTGAIAGISVAVIVVVGGLVGFLCWWFICRGKA

SEQ ID NO: 82 - protein, 741 aa, Giardia; identical to SEQ ID NO: 81

SEQ ID NO: 83 - protein, 1474 aa, Giardia
MLVGFLLVCATVLAKDSGKDTCFPGYTLNTDTKQCTKDPEAPCNVEGCETCVEGNAQQCKTCRPGYTINTDTKQCTKDPEAPCNVEGCETCVEGNAQQCKTCRPGYTINTDTKQCTKDPEAPCNVEGCETCVEGNAQQCKTCRPGYTINTDTKQCTKDPEAPCNVEGCETCVEGNAQQCKTCRPGYTINTDTKQCTKDPEAPCNVEGCETCVEGNAQQCKTCRPGYTINTDTKQCTKDPEAPCNVEGCETCVEGNAQQCKTCRPGYTINTDTKQCTKDPEAPCNVEGCETCVEGNAQQCKTCRPGYTINTDTKQCTKDPEAPCNVEGCETCVEGNAQQCKTCRPGYTINTDTKQCTKDPEAPCNVEGCETCVEGNAQQCKTCRPGYTINTDTKQCTKDPEAPCNVEGCETCVEGNAQQCKTCRPGYTINTDTKQCTKDPEAPCNVEGCETCVEGNAQQCKTCRPGYTINTDTKQCTKDPEAPCNVEGCETCVEGNAQQCKTCRPGYTINTDTKQCTKDPEAPCNVEGCETCVEGNAQQCKTCRPGYTINTDTKQCTKDPEAPCNVEGCETCVEGNAQQCKTCRPGYTINTDTKQCTKDPEAPCNVEGCETCVEGNAQQCKTCRPGYTINTDTKQCTKDPEAPCNVEGCETCVEGNAQQCKTCRPGYTINTDTKQCTKDPEAPCNVEGCETCVEGNAQQCKTCRPGYTINTDTKQCTKDPEAPCNVEGCETCVEGNAQQCKTCRPGYTINTDTKQCTKDPEAPCNVEGCETCVEGNAQQCKTCRPGYTINTDTKQCTKDPEAPCNVEGCETCVEGNAQQCKTCRPGYTINTDTKQCTKDPEAPCNVEGCETCVEGNAQQCKTCRPGYTINTDTKQCTKDPEAPCNVEGCETCVEGNAQQCKTCRPGYTINTDTKQCTKDPEAPCNVEGCETCVEGNAQQCKTCRPGYTINTDTKQCTKDPEAPCNVEGCETCVEGNAQQCKTCRPGYTINTDTKQCTKDPEAPCNVEGCETCVEGNAQQCKTCRPGYTINTDTKQCTKDPEAPCNVEGCETCVEGNAQQCKTCRPGYTLNTDTKQCTKDPEAPCNVEGCETCVEGNAQQCKTCRPGYTINTDTKQCTKDPEAPCNVEGCETCVEGNAQQCKTCRPGYTINTDTKQCTKDPEAPCNTPNCKTCDNPKTDSEICTECNDGNYLTPTNQCVPDCTTISGYYGDTDKKCKACNPECAECVGPANNQCSSCPAGKKLTYTDDSNPNNGGTCGDACKVSADGTGCETCGAQIGGTAYCSKCKTSTQAPLNGDCAASSRATFCTKMGNGVCTQCEDNYFLKDGGCYQTDRQPGKQVCSSAQGGNGKCQTCANGLAATDGNCAECHPTCATCSTAGAADKCKTCATGYYKENGDDTTDGPCKKCSEKISGCKQCVSSSGSSVICLESEVGTGGSVNKSGLSTGAIAGIAVAVIVVVGGLVGFLCWWFLCRGKA

SEQ ID NO: 84 - protein, 636 aa, Giardia
MLLVAFYFVLSALTAACQSDAQIAKCTQCVKISTSDTEICTECKAEGDVPINGVCTPKGDATVTTAGCKTDAGAEITTEKTCGQCDGAYFLHKNGCYAIGGDVGRLICADAAAAGRVSSKTPGVCEGCVVGYFKNPSAANNKDSCIACNDATGVVDGGNTYKGILNCATCQPPASAGAARQDKVAVCESCLEGFFVDSNGAACTACQDNNCAKCDAGAGKCTKCKATANKPYLKKGETEDSNTCVDKSGCNDNSHFTDDADDPTNGKMCKKCSEGIADCKTCALKDNPEGTILITCSACIAGTNQPNADGTKCVLCDIQDCIKCNEENMCEECTGGKSLSPLKNMCMEGCPAGTRDVSGICTNCHNSCAECDGDSEASCTACYPGLVLSKSNTGATGTCIPECTGRYAENCEAGQCTAVVGGSKYCSRCKAGFAPVDGVCVSTTTRAVTGCMPNDNNDGTCKACTTTYFLQSGGCYQSAAYPGSNLCSNAQNGKCTNCANGQQPEASTGSCPACASGCKTCEVANKEACKTCLPGYYLAGAKCVKCDTNDPNDGSHIVGVPNCVSCAPPTGGNGGPVTCYVKTDVTNDGGNDNNGGNTNKSGLSTGAIAGISVAVIVVVGGLVGFLCWWFICRGKA

SEQ ID NO: 85 - protein, 142 aa, Giardia
MLVGFLLVCATVLAKDSGKTACVASNTNCASGLDTAGCKTCAGAEPDQTCLDCKVSGQNVQLDKRSCAVGCPLNSAANDQKVCVCDQGFSLNDGKTACVSSGTNKSNGLSTGAIAGIVVAAVIVIGGLVGFLCWWFLCRGKA

SEQ ID NO: 86 - protein, 748 aa, Giardia
MFQLIPLFVASALMAACQPDGNHTATCAQNKCETVGATEICTQCRAGGVPVDGFCWPPGSPQAAAAGCTEEDGATLDKTATTCGKCGDGYFLFMGGCYKVGQDPGSEICTKASDGVCTTCKTDNGLFKNPATAPKPGSECILCSDIKGADGYTGVENCAQCTKSDSNKGAATCTECQDGYYKDAKGACVQCQGNCATCETSATQCTSCKAGFYLKDGNSCVAEGECTNTVYPDPESGKCKACSTITDCTECSFDKATGKPQCTACGSQKTPRTTLDGTSTCVDKTLDGCKGADGALFMKDDTTCALCGDASPGAGANDKGIAGCKTCTKQQSQKPECTSCLDGYFFEQSSKTCSACASNCATCTSADVSTCTECLPGYFLKTEGETKCAACDSTPDGGREGCSLCSSNGGFKCTECKPNYKKQSNGGAGDDYTCTKTCEDETACGGTAGACDAIVVGNDGSMLSYCSKCVGAGYGPINGKCTNALAGNTCADGVCTRCTNNYFLYMGGCYDVSKAPGNLMCSAAPSGFCTTPVGRYFKIPGDSAAQQSVLACGNPVGATAGDKAYVGVLDCTACAAPQAPAANAMAAAVCSACDKTKKPNKDGSGCTLCAVGGCKSCAIDGMCEVCAEDNKKPNMAGSTCYVCPAQGCSHCSADNKCEACTNKDQRPSLDGTQCIVCDIERCMRCSAEGVCGECEEGYVPRDGMCVSSGTNRSGLSTGAIAGISVAVVVVVGGLVGFLCWWFICRGKA

SEQ ID NO: 87 - protein, 532 aa, Giardia
MLLLVLCFLMSAFTAQRTKQPTSDCGVANCAQCVSGDNTKCETCSPGFDLSNDKTQCNQRPASNCGVANCAQCVSGDNTKCETCSPGFDLSNDKTQCNQRPASNCGVANCAQCVSGDNTKCETCSPGFDLSNDKTQCNQRPASNCGVANCAQCVSGDNTKCETCSPGFDLDENTKQCNQSPASNCGVANCAQCVSGDNTKCETCSPGFDLDENTKQCNQSPASNCGVANCAQCVSGDNTKCTKCQSNYFLTPEKNACLTSCPAGSYAVGQTCAPCDSSCAECSGAGASKCTACPAGKMLRYADESKLNEGGQCVEQCVEGPECETCGLTIGGTKYCSKCKGSNVPLNGVCTSNAARTLFCTTAANGACTACAAGYFIQEGGCYKTDRLPGKSICTTDNGGKCQTCANGQTPDGGTGVCPLCDSTCKTCAAGQTQQCQTCFSGYYKSGTKCVKCDASDGQITGVTDCVSCAPPSTNQGPVTCYVKMDGSSGGSSTNKSGLSTGAIAGISVAVIVVVGGLVGFLCWWFICRGKA

SEQ ID NO: 88 - protein, 445 aa, Giardia
MLIGFLLVCATVLAKHNEKGSSANCNTPNCRDCTNPKAENEACTDCDPAYVLNGGQCVEKACNTPNCKACDNPKTDNEVCTACDPAYVLNGGQCVEKACNTPNCKACDNPKTDNEVCTACDPAYVLNGGQCVEKACNTPNCKACDNPKTDNEVCTKCNDGDYLTPTNQCVPDCTAISGYYGDSDKKCKACNPECAECVGPANNQCTACPVGKMLQYTDTNTPVNGGTCMDQCSVSSTNDGCAECGAQIGGTAYCSKCKNTQQAPLNGNCAASSRVAFCATITSGACTKCNEGYFLKDGGCYQTDRQPGKQVCSSAQGGTCQTCANGLQAQGGACGECHSTCATCSTAGDPNKCKTCATGYYKENGDDTTAGLCKKCSEKISGCKQCVSSSGSSVICLESEVGTGGSVNKSGLSTGAIAGISVAVVVVVGGLVGFLCWWFVCRGKA

SEQ ID NO: 89 - protein, 719 aa, Giardia
MFGRFLLAGAILQLARAACEEDKTSTDGKCKTCGVTIGQDTWCSVCIGENYAPINGTCADITTDSVGSVFCTQKAGGVCTQCAGNSFMFAGGCYSSSEGLPGYNLCLRSAGNGVCAEAAPGYFIPGETAATKPSVISCSDKTGLLITAHTYKGVEFCEECSGSELTSGQDGTAKCTKCGASKYLKDNACVDNAEACGKGYFGKPDAAAGNKCIACTDQSDGGTAGCAECMYDSNTRKAICTKCTTDYLRKKADGTTECVAANECDDTQKGFYKVVDSTNGNKCVSCADGAGLAVGTDGAWKGVDGCAKCIKPADINTPTKCDECKPGYEISTDKTKCTSTAPPDCPIENCKVCSEDKRACEECNSNNYLTPTRMCIDDCKKIGNYYYTSNANNKLICKECAVANCKECENTGTCKTCDDGFYKSSEECKACDSNCKTCNGGTSADCTKCLSGAVLKYGNDGTKGTCGAGCATGTGAGACKTCGLIIDGTSYCSECAVETEYPQGGVCSSTTVRAAATCKAGSVAKGMCNSCTNGFLRMNGGCYETTKFPGKSVCEEAASAGDTCQKEAPGYHLNNNDLVTCSPGCKTCTSNTVCTACMEGYVKTSDSCAKCAAGCATCTGSTTACDTCSTGYYKSGTTCVSCTESNSDKTITGVANCASCAPPLNNKGSVLCYLIKDSGSTNKSGLSAGAIAGISVAVIIVVGGLVGFLCWWFMCRGKA

SEQ ID NO: 90 - protein, 485 aa, Giardia
MLLPALCFLMSGLAAQRTKQPAPSCQVDNCEQCNADNVHCDQCAAGFDPNTDKTQCVRACQVDNCEQCNADNVHCDQCAAGFDPNTDKTQCVRACQVDNCEQCNADNVHCDQCAAGFDPNTDKTQCVRACQVDNCEQCNADNVHCDQCAAGFDPNTDKTQCVRACQVDNCEQCNADNVHCDQCAAGFDPNTDKTQCVRACQVDNCEQCNADNVHCDQCAAGFDPNTDKTQCVRACQVDNCEQCNADNVHCDQCAAGFDPNTDKTQCVRACQVDNCEQCNADNVHCDQCAAGFDPNTDKTQCVRACQVDNCEQCNADNVHCDQCAAGFDPNTDKTQCVRACQVDNCEQCNADNVHCDQCAAGFDPNTDKTQCVRACQVDNCEQCNADNVHCDQCAAGFDPNTDKTQCVRACQVDNCEQCNADNVHCDQCAAGFDPNTDKTQCISSSINKSSGLSTGAIAGISVAVVVVVGGLVGFLCWWFLCRGKA

SEQ ID NO: 91 - protein, 1229 aa, Giardia
MLIGFLLVCVVTRAECAQNLKDAGCETCTEAGPSQTCLTCSGGQKVLLDGKSCGANCPPNSVASPNVCECDQGFSLNSGKDGCVAASNTECAQNLKDAGCETCTEAGPSQTCLTCSGGQKVLLDGKSCGANCPPNSAASPNVCECDQGFSLNSGKDGCVAASNTECAQNLKDAGCETCTEAGPSQTCLTCSGGQKVLLDGKSCGANCPPNSAASPNVCECDQGFSLNSGKDGCVAASNTECAQNLKDAGCETCTEAGPSQTCLTCSGGQKVLLDGKSCGANCPPNSAASPNVCECDQGFSLNSGKDGCVAASNTECAQNLKDAGCETCTEAGPSQTCLTCSGGQKVLLDGKSCGANCPPNSAASPNVCECDQGFSLNSGKDGCVAASNTECAQNLKDAGCETCTEAGPSQTCLTCSGGQKVLLDGKSCGANCPPNSAASPNVCECDQGFSLNSGKDGCVAASNTECAQNLKDAGCETCTEAGPSQTCLTCSGGQKVLLDGKSCGANCPPNSAASPNVCECDQGFSLNSGKDGCVAASNTECAQNLKDAGCETCTEAGPSQTCLTCSGGQKVLLDGKSCGANCPPNSAASPNVCECDQGFSLNSGKDGCVAASNTECAQNLKDAGCETCTEAGPSQTCLTCSGGQKVLLDGKSCGANCPPNSAASPNVCECDQGFSLNSGKDGCVAASNTECAQNLKDAGCETCTEAGPSQTCLTCSGGQKVLLDGKSCGANCPPNSAASPNVCECDQGFSLNSGKDGCVAASNTECAQNLKDAGCETCTEAGPSQTCLTCSGGQKVLLDGKSCGANCPPNSAASPNVCECDQGFSLNSGKDGCVAASNTECAQNLKDAGCETCTEAGPSQTCLTCSGGQKVLLDGKSCGANCPPNSAASPNVCECDQGYTLNAGKTACEKASNTQCNTPNCKICDNPKTDNEICTECNDNNYLTPTKQCTQSCGAIGSYYNGDKVCEPCDSSCAACTTTGPAKCTLCPPGKRLQYTNDDPSQGGSCVDECKPQSGASGCETCGATIGGTKYCSKCSTSTEVPVNGVCTADNARAPVCSKKDNQGGCTTCASGYFLQDGGCYKTDRQPGEQICTLADSNGGCQTCANSLQPNNGACPSCHSTCKTCRDANSANTCTTCATGYYMVGLNAGPCTSCDSNSGSVKGVAGCMSCAPPSSNTGSVLCYLIKDTGSTNKSGLSTGAIAGISVAVIVVVGGLVGFLCWWFLCRGKA

SEQ ID NO: 92 - protein, 205 aa, Giardia
MLSVIPLICTIVLAKNMAKATDCNPPIDGCSTCTGTGDGQTCTGCTAGDQKVQPNGKGCIAGCPPNSDDVGGICTCKSTHKPSDNGQTCVPKTDCNPPIDGCSTCTGTGDGQTCTGCTAGDQKVQPNGKGCIAGCPPNSDDVGGICTCKSTHKPSDNGQTCVPSNTNKSSGLSTGAIAGIAVAAVIVVGGLVGFLCWWFLCRGKA

SEQ ID NO: 93 - protein, 2293 aa, Giardia
MLSVIPLICTIVLAKNMAKATDCNPPIDGCSTCTGTGDGQTCTGCTAGDQKVQPNGKGCIAGCPPNSDDVGGICTCKSTHKPSDNGQTCVPKTDCNPPIDGCSTCTGTGDGQTCTGCTAGDQKVQPNGKGCIAGCPPNSDDVGGICTCKSTHKPSDNGQTCVPKTDCNPPIDGCSTCTGTGDGQTCTGCTAGDQKVQPNGKGCIAGCPPNSDDVGGICTCKSTHKPSDNGQTCVPKTDCNPPIDGCSTCTGTGDGQTCTGCTAGDQKVQPNGKGCIAGCPPNSDDVGGICTCKSTHKPSDNGQTCVPKTDCNPPIDGCSTCTGTGDGQTCTGCTAGDQKVQPNGKGCIAGCPPNSDDVGGICTCKSTHKPSDNGQTCVPKTDCNPPIDGCSTCTGTGDGQTCTGCTAGDQKVQPNGKGCIAGCPPNSDDVGGICTCKSTHKPSDNGQTCVPKTDCNPPIDGCSTCTGTGDGQTCTGCTAGDQKVQPNGKGCIAGCPPNSDDVGGICTCKSTHKPSDNGQTCVPKTDCNPPIDGCSTCTGTGDGQTCTGCTAGDQKVQPNGKGCIAGCPPNSDDVGGICTCKSTHKPSDNGQTCVPKTDCNPPIDGCSTCTGTGDGQTCTGCTAGDQKVQPNGKGCIAGCPPNSDDVGGICTCKSTHKPSDNGQTCVPKTDCNPPIDGCSTCTGTGDGQTCTGCTAGDQKVQPNGKGCIAGCPPNSDDVGGICTCKSTHKPSDNGQTCVPKTDCNPPIDGCSTCTGTGDGQTCTGCTAGDQKVQPNGKGCIAGCPPNSDDVGGICTCKSTHKPSDNGQTCVPKTDCNPPIDGCSTCTGTGDGQTCTGCTAGDQKVQPNGKGCIAGCPPNSDDVGGICTCKSTHKPSDNGQTCVPKTDCNPPIDGCSTCTGTGDGQTCTGCTAGDQKVQPNGKGCIAGCPPNSDDVGGICTCKSTHKPSDNGQTCVPKTDCNPPIDGCSTCTGTGDGQTCTGCTAGDQKVQPNGKGCIAGCPPNSDDVGGICTCKSTHKPSDNGQTCVPKTDCNPPIDGCSTCTGTGDGQTCTGCTAGDQKVQPNGKGCIAGCPPNSDDVGGICTCKSTHKPSDNGQTCVPKTDCNPPIDGCSTCTGTGDGQTCTGCTAGDQKVQPNGKGCIAGCPPNSDDVGGICTCKSTHKPSDNGQTCVPKTDCNPPIDGCSTCTGTGDGQTCTGCTAGDQKVQPNGKGCIAGCPPNSDDVGGICTCKSTHKPSDNGQTCVPKTDCNPPIDGCSTCTGTGDGQTCTGCTAGDQKVQPNGKGCIAGCPPNSDDVGGICTCKSTHKPSDNGQTCVPKTDCNPPIDGCSTCTGTGDGQTCTGCTAGDQKVQPNGKGCIAGCPPNSDDVGGICTCKSTHKPSDNGQTCVPKTDCNPPIDGCSTCTGTGDGQTCTGCTAGDQKVQPNGKGCIAGCPPNSDDVGGICTCKSTHKPSDNGQTCVPKTDCNPPIDGCSTCTGTGDGQTCTGCTAGDQKVQPNGKGCIAGCPPNSDDVGGICTCKSTHKPSDNGQTCVPKTDCNPPIDGCSTCTGTGDGQTCTGCTAGDQKVQPNGKGCIAGCPPNSDDVGGICTCKSTHKPSDNGQTCVPKTDCNPPIDGCSTCTGTGDGQTCTGCTAGDQKVQPNGKGCIAGCPPNSDDVGGICTCKSTHKPSDNGQTCVPKTDCNPPIDGCSTCTGTGDGQTCTGCTAGDQKVQPNGKGCIAGCPPNSDDVGGICTCKSTHKPSDNGQTCVPKTDCNPPIDGCSTCTGTGDGQTCTGCTAGDQKVQPNGKGCIAGCPPNSDDVGGICTCKSTHKPSDNGQTCVPKTDCNPPIDGCSTCTGTGDGQTCTGCTAGDQKVQPNGKGCIAGCPPNSDDVGGICTCKSTHKPSDNGQTCVPKTDCNPPIDGCSTCTGTGDGQTCTGCTAGDQKVQPNGKGCIAGCPPNSDDVGGICTCKSTHKPSDNGQTCVPKTDCNPPIDGCSTCTGTGDGQTCTGCTAGDQKVQPNGKGCIAGCPPNSDDVGGICTCKSTHKPSDNGQTCVPKTDCNPPIDGCSTCTGTGDGQTCTGCTAGDQKVQPNGKGCIAGCPPNSDDVGGICTCKSTHKPSDNGQTCVPKTDCNPPIDGCSTCTGTGDGQTCTGCTAGDQKVQPNGKGCIAGCPPNSDDVGGICTCKSTHKPSDNGQTCVPKTDCNPPIDGCSTCTGTGDGQTCTGCTAGDQKVQPNGKGCIAGCPPNSDDVGGICTCKSTHKPSDNGQTCVPSNTNKSSGLSTGAIAGIAVAAVIVVGGLVGFLCWWFLCRGKA

SEQ ID NO: 94 - protein, 721 aa, Giardia
MFEKILFTNCILQLAWIIQTVAGACTPGETGPTKCKTCDAIIGTDSYCSECDQAGEGPINGVCTSELSGNTCANKICTQCVKNYFLYKGGCYKFAESPGNIICEDAIDAAGGTDGVCTTCKAANGFFKHPAPAETKQSCIACNETAGVVDSDTTYKGTSNCLKCDPPAAAIGARADKMAVCTLCDQTKYLKESACVEKAGCGANMFGKPSVQDGNKCIACGDSNAGIEGCAECTAPDEPTIKPTCTKCTGNNYLKTTSEGTSCVQKEQCNGAYFPNDSVDGKKQCVSCGDATNKGITDCTACNLLSSPLETVLIKCSACRSGKKPNEDGSACVDAPGPSPEECSIEGCQICSDDKKTCDKCQSNNYLTPTKLCISDCKKLGNYYLATEQTTGSCRECAMVNCKECTENGKCGICNDGFYLLNEECKPCNDSCKTCEGGVESDKCTSCKSGSALIYAGNGNTGTCSLGCIPKSSADPGSCKTCDLAIDGTKYCSVCNVDKEYPQNGACAGIKARASSCQDGNVNNGVCSKCETGFFLMNGGCYEITKYPGKTVCSKTAADGTCETPATGFSLSSNTLKACFEGCAKCATGDDCSECISGYVSGSTPNSCEKCSTGCATCYPTATTCTSCLAGYYQSGPKCIACDKDDSTIKGISNCLNCAPPSSGSGSVLCYLMKGADNNGGSTNKSGLSTGAIAGISVAVIVVVGGLVGFLCWWFVCRGKA

SEQ ID NO: 95 - protein, 661 aa, Giardia
MLYGLLAMFEKILFGILILQVARAAKTCTEASSDPQTGQCKQGKCISIGGDRVCTDCAKPGEVPINGECKDKSDGLITTAGCEKVDGALDEHSTTCGKCTKAGYFLHKGGCYVQAAPPGQTVCKSASSSAGLCETCNDANGFFKNMGASDNTHQSCIACNEADTIDGFRGVPNCKVCTPPEGPGSATCTTCEGEYYLLAVTPSSCVEKTQCKTDHFPVTAKGIKKCVPCGDTDAGGIIDCKTCTLKEARGLAGESAIKCTTCNGGKTPNDEGSTCVDAPEPPPSDCPVENCQKCSADKKTCEECKDKNYLTPTGMCIKYCEYILGYYSSTEGGKGICKKCEVKNCVVCDPNGKCGFCEDGFYADDAGICQKCDGSCKNCKGNTANDCTECKPGTILDYANGQKGKCAPECVVNTDKATGNCKACDLIVKGTRYCSACSQDNEYPQNGVCAPKPSGRAATCTSQGTGVCNSCANGLLRMNGGCYEDEKYPAHSVCATVATTGGTCDRPMPGFNLNNENNLVICPEGCKTCNTANECTECMDGYIAFSNVKACTKCHESCYTCETAAATCKVCARGYYKESSDSGPCKKCSEGLAGCRQCTVSSTSAFMCLEMGDSTGDNNGGSTNKSGLSTGAIAGISVAVIVVVGGLVGFLCWWFVCRGKA

SEQ ID NO: 96 - protein, 661 aa, Giardia; identical to SEQ ID NO: 95

SEQ ID NO: 97 - protein, 734 aa, Giardia
MLVGIGLIFAVALADACSPSIDGCAECDSTGQGCTKCDANGNTPYLKKTNPGDQTGTCVSKEDCTRDGGYYADDTTDPNAKECKKCDATCAACSSGLATACTKCEAGGATPYLKKTNPGDQTGTCVSKEDCTRDGGYYADDTTDPNAKECKKCDATCAACSSGLATACTKCEAGGATPYLKKTNPGDQTGTCVSKEDCTRDGGYYADDTTDPNAKECKKCDATCAACSSGLATACTKCEAGGATPYLKKTNPGDQTGTCVSKEDCTRDGGYYADDTTDPNAKECKKCDAGQKPNTAGTQCFACPDSNCERCDQSDVCARCSTGAPPENGKCPAATPGCHSSCKDCVSGANTSEDDKCLSCSGDNYLKVTDTDAHSGVCVSASACTSDTTHFTKEVADSTGSKKMCLSCSDATHGITGCKKCALKTLSGETESTVVCSECTDKRLTPSGNACLEQCPAGTYADNINGVSVCASCHATCAECNGNADAASCTACYPGYSLLYGSGTAGTCVKECTGAFITNCADGQCTANVGGAKYCAQCKDGYAPIDGICTAVKTGRDASVCTAAGGKCTKCAGEYTLMSGGCYGVAKLPGKAVCTTANNGKCTMCAANNRAPVQEKCPECSEGCAKCNDSNACTECLPGYYKGAGDKCFKCTASSGNNNQITGVANCVSCAPPAGNAGGPVTCYIKTDGDNTGGSVNKSGLSTGAIAGISVAVIVVVGGLVGFLCWWFVCRGKA

SEQ ID NO: 98 - protein, 583 aa, Giardia
MLYLAGLAFAYLALADPKSCTNSQNCASGNNCLDVNINGQQKEVCTKCEATHVPVEGACQAKDGQDKCTPQDAPDGTCKACQGSTYLYSGGCYAACPDGTYADAGVCQPCEASCVKCEKKDAGTRCVKCQATHVPVEGACQAKDGQDKCTPQDAPDGTCKACQGSTYLYSGGCYAACPDGTYADAGVCQPCEASCVKCEKKDAGTRCVKCQATHVPVEGACQAKDGQDKCTPQDAPDGTCKACQGSTYLYSGGCYTACPQGTPNSETNTCDGVPAPDCNLPNCEVCSDDKQTCTKCQGNYFLTPEKNACLASCPAGSYAVGQTCGPCDPSCAECSGAGASKCTACPAGKMLRYADESNPTDGTCVEQCVEGPECETCGLTIGGTKYCSKCKGSNVPLNGVCTSNAARTRFCTTAADGACTACAAGYFIQEGGCYQTTRLPGKSICTTDSGGKCQTCANGQNPNSGTGVCPLCDSTCKTCAAGQTQQCQTCFSGYYKSGTKCVKCDASDSQITGVTNCVSCAPPSGDSGSVTCYVKMDGTDNGGSVNKSGLSTGAIAGISVAVIVVVGGLVGFLCWWFLCRGKA

SEQ ID NO: 99 - protein, 398 aa, Giardia
MLLGFLLVCAVTQASCAAGCKTCDPGDQTCTACTNDSHKIQVDGKSCDAACPAHSAASSNVCECEGGYRPVTGENRCEKASNTQCNTPNCKTCDNPKTDNEICTECNDNNYLTPTKQCTQSCGAIGSYYDGDKACEPCDPSCAGCTTKGPAKCTACPPGKMLKYTNDDPSQGGSCVDECKAEMDGCAECGAVIGGTKYCSKCKEDKWAPQNGVCANSVTRNSFCTNAAGGVCTQCAADHFLQDGGCYKLGRQPGVQICAAVGPNSLCTTCVNGQRPDTNTGACPVCPTGCDTCTGTSSRAPECQSCLLGYYFDSDKKLCVKCTENSSAIQGVSSCVSCAPPSNNQGSVVCYLINDSGSTNKSSGLSTGAIAGIAVAAVIVVGGLVGFLCWWFLCRGKA

SEQ ID NO: 100 - protein, 1921 aa, Giardia
MLLGLLLFCTVARANCKAGNTPSANGQTCVPNADQCEDPLTTAGCATCTGTGSAQTCLTCSSSKKVRPDKKGCIASCPPSVTTENSGVCECTPGNKPSSDGTTCVPNADQCEDPLTTAGCATCTGTGSAQTCLTCSSSKKVRPDKKGCIASCPPSVTTENSGVCECTPGNKPSSDGTTCVPNADQCEDPLTTAGCATCTGTGSAQTCLTCSSSKKVRPDKKGCIASCPPSVTTENSGVCECTPGNKPSSDGTTCVPNADQCEDPLTTAGCATCTGTGSAQTCLTCSSSKKVRPDKKGCIASCPPSVTTENSGVCECTPGNKPSSDGTTCVPNADQCEDPLTTAGCATCTGTGSAQTCLTCSSSKKVRPDKKGCIASCPPSVTTENSGVCECTPGNKPSSDGTTCVPNADQCEDPLTTAGCATCTGTGSAQTCLTCSSSKKVRPDKKGCIASCPPSVTTENSGVCECTPGNKPSSDGTTCVPNADQCEDPLTTAGCATCTGTGSAQTCLTCSSSKKVRPDKKGCIASCPPSVTTENSGVCECTPGNKPSSDGTTCVPNADQCEDPLTTAGCATCTGTGSAQTCLTCSSSKKVRPDKKGCIASCPPSVTTENSGVCECTPGNKPSSDGTTCVPNADQCEDPLTTAGCATCTGTGSAQTCLTCSSSKKVRPDKKGCIASCPPSVTTENSGVCECTPGNKPSSDGTTCVPNADQCEDPLTTAGCATCTGTGSAQTCLTCSSSKKVRPDKKGCIASCPPSVTTENSGVCECTPGNKPSSDGTTCVPNADQCEDPLTTAGCATCTGTGSAQTCLTCSSSKKVRPDKKGCIASCPPSVTTENSGVCECTPGNKPSSDGTTCVPNADQCEDPLTTAGCATCTGTGSAQTCLTCSSSKKVRPDKKGCIASCPPSVTTENSGVCECTPGNKPSSDGTTCVPNADQCEDPLTTAGCATCTGTGSAQTCLTCSSSKKVRPDKKGCIASCPPSVTTENSGVCECTPGNKPSSDGTTCVPNADQCEDPLTTAGCATCTGTGSAQTCLTCSSSKKVRPDKKGCIASCPPSVTTENSGVCECTPGNKPSSDGTTCVPNADQCEDPLTTAGCATCTGTGSAQTCLTCSSSKKVRPDKKGCIASCPPSVTTENSGVCECTPGNKPSSDGTTCVPNADQCEDPLTTAGCATCTGTGSAQTCLTCSSSKKVRPDKKGCIASCPPSVTTENSGVCECTPGNKPSSDGTTCVPNADQCEDPLTTAGCATCTGTGSAQTCLTCSSSKKVRPDKKGCIASCPPSVTTENSGVCECTPGNKPSSDGTTCVPNADQCEDPLTTAGCATCTGTGSAQTCLTCSSSKKVRPDKKGCIASCPPSVTTENSGVCECTPGNKPSSDGTTCVPNADQCEDPLTTAGCATCTGTGSAQTCLTCSSSKKVRPDKKGCIASCPPSVTTENSGVCECTPGNKPSSDGTTCVPNADQCEDPLTTAGCATCTGTGSAQTCLTCSSSKKVRPDKKGCIASCPPSVTTENSGVCECTPGNKPSSDGTTCVPNADQCEDPLTTAGCATCTGTGSAQTCLTCSSSKKVRPDKKGCIASCPPSVTTENSGVCECTPGNKPSSDGTTCVSETACNTPNCKTCDNPKTDNEICTECNDGDYLTPTKQCTQSCGAIGSYYDGDKACEPCDPSCAGCTTKGPAKCTLCPPGKRLQYTNDDPNQGGSCVDECKAEVDGCAECGAVIGGTKYCSKCKEDKWAPQNGVCANSVTRNSFCTNAAGGVCTQCAADHFLQDGGCYKLGRQPGIQICTLADSNGGCQTCANSLQPNDGACPSCHSTCKTCSTADSSDKCTSCAAGYYMVGSGPNTCISCDSNSGSVKGVAGCMSCAPPPNNQGSVVCYLINDSGSTNKSSGLSTGAIAGISVAVVVVVGGLVGFLCWWFLCRGKA

SEQ ID NO: 101 - protein, 627 aa, Giardia
MLLVVFYLVLSALAAACKQAQNCVEDKCEMIGDTEICTQCTAGKVPIDGVCTAVGSAAGKCTKAEGQAVDDTDKTCGKCVDAYFMYKGGCYLAGAAGPGTGTKMCKQAAGGKCTQAADAKNYFIPPANTDDTHDSVVWCGDEIGVTLSSTQYKGVAKCLVCDAPGGAGAATCTTCEDGYFGATCEKCHESCRTCEAAEENKCKSCTDGYFLGATNGAAGKCLKCNSKTEEGWHGVDNCAKCTSSNTQNTPATCTECVANFYLKPAADATPSSCVTETGCGDGYFPTIVDEVKKCIACSAATNGGIDDCKKCSLKTTSAKAGVEIVCTECNTKWLSPLRDACLDSCPPGTHADSGNICPLCHSTCAECDGNAGANFCTVCYPGFVLKRGETGNMGMCVPECTGEYAENCEADQCTAVIGSSKYCSRCKVGFAPVDGVCVSTASRAVTGCTAGNDGTCTACTGTYFLQSGGCYQSTTYPGNTLCSIAASGKCTTCANGQTADSNLGSCPACPAGCSKCATSGSPKACSECFPGYYKSGDSCARCDTNNSQITGVANCVSCAPPSNGQGSVICYITRQETDDGTGDNTGGSTNKSGLSTGAIAGISVAVIVVVGGLVGFLCWWFICRGKA

SEQ ID NO: 102 - protein, 627 aa, Giardia; identical to SEQ ID NO: 101

SEQ ID NO: 103 - protein, 425 aa, Giardia
MLYLAGLAFAYLALADPKSCTNSQNCASGDNCLDVNMNGSPTEVCTKCEPNNVPIDGACKPAADNTNSCVTSDSGAGGVCASCQGSTYLYKGGCYAACPQGTPNSETNTCDGVPAPDCNLANCEVCSEDKQKCTKCQSNYFLTPEKNACLASCPAGSYAVGQTCAPCDPSCAECSGAGASKCTACPAGKMLRYADESKLNEGGQCVEQCVEGPECETCGLTIGGTKYCSKCKGNNVPLNGVCTSNAARTRFCTTVANGACTVCAAGYFIQEGGCYKTDRLPGKSICTTPTGDGKCQTCANGLTAVSNMCPLCDSTCATCTVANQPDKCSTCPPGRYLDASKACKLCTETSGSIQGVANCASCAPPTGNSGSVICYVKTDGTDNGGSTNKSGLSTGAIAGISVTAVVVVAGLVSFLCWWFLCRGKA

SEQ ID NO: 104 - protein, 1431 aa, Giardia
MLVGFLLVCAVTQASCAAGCQTCNPADQTCTACTDSSHNIQVDGKSCAADCPPNSAPNQKVCECEGGYGPVAGQNRCEQNPSAGCAAGCQTCNPADQTCTACTDSSHNIQVDGKSCAADCPPNSAPNQKVCECEGGYGPVAGQNRCEQNPSAGCAAGCQTCNPADQTCTACTDSSHNIQVDGKSCAADCPPNSAPNQKVCECEGGYGPVAGQNRCEQNPSAGCAAGCQTCNPADQTCTACTDSSHNIQVDGKSCAADCPPNSAPNQKVCECEGGYGPVAGQNRCEQNPSAGCAAGCQTCNPADQTCTACTDSSHNIQVDGKSCAADCPPNSAPNQKVCECEGGYGPVAGQNRCEQNPSAGCAAGCQTCNPADQTCTACTDSSHNIQVDGKSCAADCPPNSAPNQKVCECEGGYGPVAGQNRCEQNPSAGCAAGCQTCNPADQTCTACTDSSHNIQVDGKSCAADCPPNSAPNQKVCECEGGYGPVAGQNRCEQNPSAGCAAGCQTCNPADQTCTACTDSSHNIQVDGKSCAADCPPNSAPNQKVCECEGGYGPVAGQNRCEQNPSAGCAAGCQTCNPADQTCTACTDSSHNIQVDGKSCAADCPPNSAPNQKVCECEGGYGPVAGQNRCEQNPSAGCAAGCQTCNPADQTCTACTDSSHNIQVDGKSCAADCPPNSAPNQKVCECEGGYGPVAGQNRCEQNPSAGCAAGCQTCNPADQTCTACTDSSHNIQVDGKSCAADCPPNSAPNQKVCECEGGYGPVAGQNRCEQNPSAGCAAGCQTCNPADQTCTACTDSSHNIQVDGKSCAADCPPNSAPNQKVCECEGGYGPVAGQNRCEQNPSAGCAAGCQTCNPADQTCTACTDSSHNIQVDGKSCAADCPPNSAPNQKVCECEGGYGPVAGQNRCEQNPSAGCAAGCQTCNPADQTCTACTDSSHNIQVDGKSCAADCPPNSAPNQKVCECEGGYGPVAGQNRCEQNPSAGCAAGCQTCNPADQTCTACTDSSHNIQVDGKSCAADCPPNSAPNQKVCECEGGYGPVAGQNRCEQNPSAGCAAGCQTCNPADQTCTACTDSSHNIQVDGKSCAADCPPNSAPNQKVCECEGGYGPVAGQNRCEQNPSAGCAAGCQTCNPADQTCTACTDSSHNIQVDGKSCAADCPPNSAPNQKVCECEGGYGPVAGQNRCEQNPSAGCAAGCQTCNPADQTCTACTDSSHNIQVDGKSCAADCPPNSAPNQKVCECEGGYGPVAGQNRCEQNPSAGCAAGCQTCNPADQTCTACTDSSHNIQVDGKSCAADCPPNSAPNQKVCECEGGYGPVAGQNRCEQNPSAGCAAGCQTCNPADQTCTACTDSSHNIQVDGKSCAADCPPNSAPNQKVCECEGGYGPVAGQNRCISSSVNKSGLSTGAIAGIAVAAVIVVGGLVGFLCWWFLCRGKA

SEQ ID NO: 105 - protein, 587 aa, Giardia
MFYAVLLIGLMLEMARAAQAGDECEEVTGSDPNTCKTCSAVINGKKYCSQCNDSGSQSAPTDGKCTADNNECSTKNNGVCTQCAHESFMYKGGCYKKATEPGNTMCETANAGVCTQAKAGYFVPPGADRDNAHQSVIPCGDVEEVLVGNSHKYKGVLHCKVCDAPKAAASDTNPVPATCTTCEDGFFGPTCEACQDENCATCAVTGNNKCSKCKGTGTKTYLKVDGGSTGTCVEASGCTAATFPKVDEQQGNKCAACNSAPDGGIANCATCSLLTQGSRATPLVTCLTCEQNKYLTPEKNACLDACPAGMYANSKVCTPCHESCASCSTNAKTSCTACYPGYVLSKGDDGATGTCIPECTGRYAENCADGQCTAVVGGSKYCSKCKAGYAPVDGICVSTATREVMGCTPGNDGTCTACTGSYFLQSGGCYQSTAYPGNTLCSSAQNGQCQTCAANGQSPAGGKCPECSEGCAKCGASNSDVCTECYSGYYRTGTGKCFKCAADSDNGIVGVPNCVSCAPPTNGQGSVICYITRQETDDGTGGDTGGDSMNKSGLSTGTIAGISVAVIVVVGGLVGFLCWWFVCRGKA

SEQ ID NO: 106 - protein, 593 aa, Giardia
MFYAVLLIGLMLEMAWAAQAGDECEEVTGSEPNTCKTCSAVINGKKYCSQCNDTGNSNSGGAPTDGVCSADNNECSQKQDGKCTQCANKSFMYKGGCYKDSQAPGNTMCETATDGVCTQAKAGYFLPPDADRDNAHQSVIPCGDVEEVLVGNSHKYKGVLHCKVCDAPKAAASDTNPVPATCTTCEDGFFGPTCEACQDENCATCAVTGNNKCSKCKGTGTKTYLKVDSGSTGTCVEASGCTAATFPKVDEQQGNKCAACNSVPDGGIANCATCSLLTQGSRAAPLVTCLTCEQNKYLTPEKNACLDTCPAGMYAVSGDSGNVCTPCHESCASCSTNAKTSCTACYPGYVLSKGDDGATGTCIPECTGRYAENCADGQCTAVVGGSKYCSKCKAGYAPVDGVCVSTTTRAALGCTPGDGVCTACTGSYFLQSGGCYQSTAYPGNTLCSSAQNGQCQTCAANGQSPAGGKCPECSEGCAKCGASNSDVCTECYSGYYRTGTGKCFKCAADSDNGIVGVPNCVSCAPPSNGQGSVICYITRQETDDGTGGDTGGDSMNKSGLSTGAIAGISVAVVVVVGGLVGFLCWWFICRGKA

SEQ ID NO: 107 - protein, 593 aa, Giardia; identical to SEQ ID NO: 106

SEQ ID NO: 108 - protein, 197 aa, Giardia
MFDKLIFVSLALQMALASQTASKAKTNPTPCAAANPGATNCAADSCNVEIGGQTFCSKCTGDKVPVNGECKAKTDAGMCTAGTSDKAGTCTACTGAHSLYKGGCYDECPYGPTANERVCADAPAGCDLPNCKSCPDGTCTECNDGFVLGDDKKCVPSSVNKSGLSTGAIAGIAVAAVIVVGGLVGFLCWWFLCRGKA

SEQ ID NO: 109 - protein, 591 aa, Giardia
MFYAVLLIGLALQLATEECTPVSSGGPNTCKACDAVINGKKYCSQCNDTGNSDSSGAPTDGVCSADNNECSQKQDGKCTQCANKSFMYKGGCYKDSQAPGNTMCETATDGVCTQAKAGYFLPPDADRDNAHQSVIPCGDDTVVTLGNSKQYKGVPHCTQCEKPTEASDTTTAKAATCTACEDGFFGATCEACQDENCATCAMTGNNKCSKCKGTGTKTYLKVDGGSTGTCVEASGCTAATFPKVDEQQGNKCAACNSVPDGGIANCATCSLLTQGSRAAPLVTCLTCEQNKYLTPEKNACLDTCPAGMYAVSGDSGNVCTPCHESCASCSNDAATSCTACYPGHVLSRSSGDAGTCIKECTGDFMAHCKADGCSLNVGGSKYCDQCEEGYAPVDGVCTSIPATARDASGCKASGGKCTECGANYALLSGGCYNTQKLPGSSVCTAAQNKGQCQTCANGQSPAGGKCPACTEGCVKCAGSKETCTDCLAGYYKGAGDKCFKCTDSDKASSNAITGVENCISCAPPAGGNGPVTCYVTQQKADDGTGGDTGGDSTNKSGLSTGAIAGISVAVVAVVGGLVGFLCWWFLCRGKA

SEQ ID NO: 110 - protein, 775 aa, Giardia
MLAVILLVCTTVLAGIGPKTACDPPIPGCSTCATPPGGEQTCTGCATVGQKVQPNGKGCIAKCPDNANEAGGICTCTETYQPSEDGLTCVLKTACDPPIPGCSTCATPPGGEQTCTGCATVGQKVQPNGKGCIAKCPDNANEAGGICTCTETYQPSEDGLTCVLKTACDPPIPGCSTCATPPGGEQTCTGCATVGQKVQPNGKGCIAKCPDNANEAGGICTCTETYQPSEDGLTCVLKTACDPPIPGCSTCATPPGGEQTCTGCATVGQKVQPNGKGCIAKCPDNANEAGGICTCTETYQPSEDGLTCVLKTACDPPIPGCSTCATPPGGEQTCTGCATVGQKVQPNGKGCIAKCPDNANEAGGICTCTETYQPSEDGLTCVLKTACDPPIPGCSTCATPPGGEQTCTGCATVGQKVQPNGKGCIAKCPDNANEAGGICTCTETYQPSEDGLTCVPKAGACNTPNCKACDNPKTDREVCTECNDNNYLTPTNQCIPDCTTISGYYGDTDRKCKACSPECAECVGPANNQCSACPAGKALIYKSSDPVQGGTCGDACTADKNGCKVCGARIGGTDYCSQCSVDNQAPLNGVCTTSNARVAFCTEMNNGACIKCAANYFLKEGGCYETTKQPGKQICTLADSRGKCETCANSLRPNDGACPSCHSTCNTCSAADSSDQCTSCAAGYYMVGSAAGPCTSCDSNSGSVKGVAGCMSCAPPSSSTGSVLCYLMNGDSAGGSTNKSGLSTGAIAGISVAVIVVVGGLVGFLCWWFLCRGKA

SEQ ID NO: 111 - protein, 593 aa, Giardia
MFYAVLLIGLMLEMARAAQAGDECEEVTGSEPNTCKACSAVINGKKYCSQCNSGGSQSAPTDGKCTTDNNECSQKQDGKCTQCANKSFMYKGGCYKDSQAPGNTMCETATDGVCTQAKAGYFLPPDADRDNAHQSVIPCGDDTVVTLGNSKQYKGVPHCTQCEKPTEASDTTTAKAATCTACEDGFFGATCEACQDENCATCAMTGNNKCSKCKGTGTKTYLKVDSGSTGTCVEASGCTAATFPKVDEQQGNKCAACNSVPDGGIANCATCSLLTQGSRAAPLVTCLTCEQNKYLTPEKNACLDTCPAGMYAVSGDSGNVCTPCHESCASCSNDAATSCTACYPGHVLSRSSGDAGTCIKECTGDFMAHCKADGCSLNVGGSKYCDQCEEGYAPVDGVCTSIPATARDASGCKASGGKCTECGANYALLSGGCYNTQKLPGSSVCTAAQNKGQCQTCANGQSPAGGKCPACTEGCVKCAGSKETCTDCLAGYYKGAGDKCFKCTDSDKASSNAITGVENCISCAPPAGGNGPVTCYVTQQKADDGTGGDTGGDSTNKSGLSTGAIAGISVAVVAVVGGLVGFLCWWFLCRGKA

SEQ ID NO: 112 - protein, 410 aa, Giardia
MLAVILLVCTTVLAGIGPKTACDPPIPGCSTCATPPGGEQTCTGCATVGQKVQPNGKGCIAKCPDNANEAGGICTCTETYQPSEDGLTCVPKAGACNTPNCKACDNPKTDREVCTECNDNNYLTPTNQCIPDCTTISGYYGDTDRKCKACSPECAECVGPANNQCSACPAGKALIYKSSDPVQGGTCGDACTADKNGCKVCGARIGGTDYCSQCSVDNQAPLNGVCTTSNARVAFCTEMNNGACTKCAANYFLKEGGCYETTKQPGKQICTLADSRGKCETCANSLRPNDGACPSCHSTCNTCSAADSSDQCTSCAAGYYMVGSAAGPCTSCDSNSGSVKGVAGCMSCAPPSSSTGSVLCYLMNGDSAGGSTNKSGLSTGAIAGISVAVIVVVGGLVGFLCWWFLCRGKA

SEQ ID NO: 113 - protein, 521 aa, Giardia
MLLLVLCFLMSALAAQRTKQPTSDCGVANCAQCNADGRTCDQCSEGYNLNQEKTQCTKACAVANCAQCNADGRTCDQCSEGYNLNQEKTQCTKACAVANCAQCNADGRTCDQCSEGYNLNQEKTQCTKACAVANCAQCNADGRTCDQCSEGYNLNQEKTQCTKACAVANCAQCNADGRTCDQCSEGYNLNQEKTQCTKNPEARCNTPNCKTCDSPKTDSEICTECNNGNYLTPTKQCTQSCGTIGSYYNGDKVCEPCDPSCAACITKGPAKCTLCPPGKRLQYTDEGATQNGGSCVDECKPEGGASGCETCGATIGGTKYCSKCSTSTEVPVNGVCTADNARAAACKVKDGKGGCTTCESGYFLQDGGCYKLGRQPGEQICTAASSAGKCETCANSLQPNNGACPSCHSTCKTCRDANSANACTTCAAGYYMVGSAAGPCTSCDSNSGSVKGVAGCMSCAPPSSSTGSVLCYLMNGDSAGGSTNKSGLSTGAIAGISVAVIVVVGGLVGFLCWWFLCRGKA

SEQ ID NO: 114 - protein, 419 aa, Giardia
MLLIAFYLGLSALAAQCKQVQNCAAGKCEMVGGTEICTECATNGNVPINGECTPKGNAADKCKKVNGNELVDDKTCGKCENTYFMYKGGCYQLGSDVALLICNDQAASPGGRNAVAGVCTECNATGGFFKSPEAADTTDSCISCSDTTGVQVNGGNTYKGIENCVVCAAPERGTGNENKIAACESCLEGFFVASNKAVCTRCTDNDNCAKCDAGENKCTKCKATASKPYLKKGETEDSNTCVNSNECTTDKTYFTDDTDDPTHGKMCKKCSEGIADCKKCAPSSPSALATVSAIVCTECTTQTNKPNVAGTGCFTCSVDGCSNCSENDVCEKCGPNKKVSPGRKSCVDSCPENSIDDNSVCTCSSGYSPDSSGASCVSTGSNRSGLSTGAIAGISVAVIVVVGGLIGFLCWWFVCRGKA

SEQ ID NO: 115 - protein, 734 aa, Giardia
MFGSFVLAGVLVQIALAEKVTERARQAECADKTNDCEICDVLIDGKLYCSRCNTGFVPINGKCADKEGAKANCKGADGGDTADRTCAQCAEQTFMYKGSCYQTSQAPGSSMCKTAADGKCTEALESKAYFVPPGADKTHDSVVSCGDATGVTLADKTYKGVDGCTACDAPAPADASGAKVATCTACQADKYLKTATDPATSCVTEKECTDAPGFFVDTTDGKKCSKCAETCKTCKTEAAKCTSCNGDKPYLKKDGESTTGTCVDAKGCPETHYVDEGAKECNTCVSAGTTDCTTCEKGPTGVVCKTCTSGTKTKFGLGKKSCVENCPSNSNDEKTAGTCECVDGYVLNGAGTGCTKKPDPQCNTPGCKTCSEPKTSKEVCTECEGPKALTPTGQCIDNCGDLGGYYAGTNEGGKKACKKCEVENCLLCNLQGQCDTCKDGYYKSGAACAKCDTSCKTCANGNSNGCTSCEPKKALSYEGEGNTGTCKSECKPGTNNCEKCELTVDGTAYCSKCKDANQFPQNGVCSAAAGKAITCTTQGGGVCNKCANGLLRMNGGCYETTKLPGKNVCEEVTQDGDTCKTEAPGYHLNNNDLVTCSPGCKTCTSNTVCTTCMYGYVKTDNKCTKCATGCATCAGSASNCDICSTGYYKSGTTCVSCTANTADSTITGVANCASCAPPLNDKGSVLCYLVQSGENTNKGGLSTGAIAGIAVAVIIVVGGLVGFLCWWFMCRGKA

SEQ ID NO: 116 - protein, 271 aa, Giardia
MLYLAGLAFAYLALADPKSCTNSQNCASGTNCLDVNINGQQKEICTKCEATHVPVEGACQAKDGQDKCTPQDAPDGTCKACQGSTYLYSGGCYAACPDGFYGKGDNTCASCDSSCDKCEAKTPTSSRCTKCAVTHVPIDGACETIAAAGAKCTAKSTPDGTCQSCKGENYLYRGGCYVSCPQGTPNSETNTCDGVPAPDCNLPNCKSCPGGTCTECNDGFVLGDDKNCVPSSVNKSGLSTGAIAGIAVAAIIVVGGLVGFLCWWFICRGKA

SEQ ID NO: 117 - protein, 708 aa, Giardia
MLLIALHLVTSILAAPCQPDGDHAASCQTDKCETVGYSEICTECRAGGVPVGGFCWPPGTPQAAAAGCTRADGTALAGSDTICGKCGDGYFLFMGGCYKTSQWSEICTAADKGVCTTCKAGAAYLFQNPASPVAPGNECVLCSDVAPRDGVTGVAGCYTCTAPGGGTGAATCTACQGGYAKKGDACVQCGPGCLTCESATPTQCTACPKGKFLKGTECVEASGCGSDSYADPKVDKCKACATDIADCATCEYNATISQPQCKTCSSSKIVKTAADGTTTCVAEGECTSTHFIDQTPPKACVLCGDDARGGVAGCSSCPGKDQCSACLAGYIKKGSGNSVTCDPCGENCATCTQAGNDKCDTCKPGYFLKQPGSAGKCFACDSKADNGIEGCSQCNSGLTPTCTDCKSNYRKEGTNPVKCTKVCEDPTACGGTSGACGAVVVDSAGAFSQYCSLCGDPATFPIDGVCTGTKGDNTCENGVCTRCAAGFFLYMGGCYDVSKAPGSHMCKTAEGGRCTAPSENGRYFLVPGASNTDQSVLACENPLGTVIGAGSTAKAYVGVYGCTACTAPAALEAPGMTPATCTACSGNNKPNLAGSGCFTCTVDGCSHCGAGGKCEACTSKDQRPNTDGSQCIACSIDGCVRCSEENKCGRCGDDYRLEGEACVSTKPSGGNRSGLSTGAIAGISVAVVVVVAGLVGFLCWWFICRGKA

SEQ ID NO: 118 - protein, 370 aa, Giardia
MLLPALCFLMSGLAAQRTKQPTSGCQVDNCERCVPSDETKCEACNSGFDLDENTKQCNPAPAECPIVNCQTCSQDKQTCVACEPGKHLTPTKKACLDACPVGTYLSGQTCAPCDPSCAECSGAGASKCTACPAGKMLRYTDETKLNEGGQCVEQCVEGPECETCGLTIGGTKYCSKCKGSNVPLNGVCTSNAARTQFCTTAADGACTACAAGYFIQEGGCYQTTRLPGKSICTTDNGGKCQTCANGQTPDGGTGVCPLCDSTCKTCTAGQTQQCQTCFSGYYKSGTKCVKCDASDGQITGVTDCVSCAPPSGDSGSVTCYVKMDGSSGGNSTNKSGLSTGAIAGIAVAAVIVVGGLVGFLCWWFICRGKA

SEQ ID NO: 119 - protein, 718 aa, Giardia
MLLIALHLATSILAAPCQPDGDHAASCQTDKCETVGYSEICTECRAGGVPVGGFCWPPGSPQAAAAGCTRADGTALAGSDTACGKCGDGYFLFMGGCYKTSQWSEICTAADKGVCTTCKADAVYLFQNPASPVAPGNECVLCSDVTPRDGVTGVAGCYTCTAPGGGTGAATCTACQGGYATKDGACVQCGPGCLTCESATPTQCTACLGGKFLKGTECVEAGGCGSDSYADPKADECKACATDIAGCAACEYSDATGKPRCTDCNGKLVRTAADGTTTCVEKTDDGCKATDSGLFMKDDATACILCSDTVTEQEKKNQGIVGCKKCSRTGATPPTCTECLEGYIKNTNSGFTCDACGENCATCSEKADKTKCQTCKTGFFLRGGTSPGTCVPCDNPTDGVDGCATCTFAGSLTCNSCKPNYRKEGTNPVKCTKACEDPTACGGTSGACGAVVVDSAGAFSQYCSLCGDPATFPIDGVCTGTKGDNTCANGVCTQCAAGYFLYMGGCYSTQKAPGSHMCKTAEGGRCTAPSENSRYFLVPGASNTDQSVLACENPLGTVIGAGSTAKAYVGVYGCTACTAPAALEAPGMAPATCTACSGNNKPNLAGSGCFTCTIDGCSHCGAGGKCEACTSKDQRPNTDGTKCIPCSIDGCVRCSEENKCGQCGDDYSLEGDKCVSSGANKSSGLSTGAIAGISVAVVVVVAGLVGFLCWWFICRGKA

SEQ ID NO: 120 - protein, 633 aa, Giardia
MFEKIIFGIAILQVVWAATTCTEASSDPQTGQCATGKCDVWIGGSNFCSQCSTAAEYLINGLCYPDNKDNGCEGQPSTGVCTQCAQGFFLHRGGCYKIGTEPGNLICEDTQASQTQGVCEACSSGYFKNPAADAAGTPPCIACNDTVGNSNNVGIANCKTCASPSAAGTENAPQTATCTACVDGFSPDSTGKTCVAVQCAENCLTCTSSGEDKCKSCKDGYFLGAASGGEGKCIKCNDTTGANSYKGIANCAKCTQPQSAGPAVCTECAADLYLKIDRGVMECVAAAGCGEGFFPTTVGGVKKCIGCSEAGNGGIDKCAKCTLKTPAPEAGVKVTCSECDSQKKLSPLKDECMDSCPAGTYDKQNVCTPCHSSCASCTDATSTTCTACYPGFVLNAASGASAGTCIPECTGQYAENCADGQCTAIVGGSKYCSKCKAGYVPVDGVCVSTTTRAVTGCTPGDGVCTACTGSYFLQSGGCYQSTTYPGNTLCSSATNGKCQTCANGQTADNQGSCPACPDGCSKCTGSASPQQCQTCLPGYYKSGDSCVKCDASANGIVGVPNCISCAPPAGGSGSVTCYVKTDGTSGGDDNTGGSANRSGLSTGAIAGISVAVIVVVAGLVGFLCWWFICRGKA

SEQ ID NO: 121 - protein, 493 aa, Giardia
MLLKITLTLAIALAECQEGSFLYMGKCHRREPGAGMQAPDPVLCPEAVSGPGNCKPGKCFGIGGEELSYCSQCADATEVPLNGACDNSEETQACTQMSDGVCTQCAKKTFMYKGGCYSTIGVPGVKMCKEATDGVCTSPAPGYFVLPADDRDASHQSVVSCGDGEGAPGRTKLYKGVKGCAECTLSVPATTATCNRCTTKNLSPLKDACLTDCPAGMYANNKVCTPCHESCASCSTNAEASCTACYPGSVLSRSSGGTGACMKECTGKYAENCEAGQCTAVVGGSKYCSRCKAGYVPVDGVCVSITTRAPTGCTPSDNNDGTCKACTTTYFLQSGGCYSAGAFPGNTLCSSAANGKCQTCANGQAADTTSGSCPACPDGCSKCTESASPQQCSECLPGYYKSGSSCVKCDASDNGIVGVPNCISCAPPAGGSGSVTCYVKTDGTSGGDNNTGGSTNRGGLSTGAIAGISIAVVVVVGGLVGFLCWWFVCRGKA

SEQ ID NO: 122 - protein, 615 aa, Giardia
MFEKIIFGIAILQVVWAATTCTEASSDPQTGQCATGKCDVWIGGSNFCSQCSTAAEHLINGKCVPEGEDTEGKCTAKNDGTCESCKAGFFLHRGGCYEMGSDIGLLVCNDRTATADKDGICIACHDGYFKNPASDADKTKESCIACNNTAGVDHNKGVQNCATCDAPKTPGQSSAEQTATCKSCVDGYYGTTSCQQCHADCRTCTGNGEDKCTSCKDTGKQYFKEGANSDGTGTCVDENGCGNTHFPIAEDKKCHLCGSVSEGGVADCKTCSKTGDSVKCLTCEGTKKPNEAGTGCFVCPMEHCEKCSKDNVCEACGSEKKLSPLGDACLDACPAGTRTDANVCNLCHESCASCSTNAEASCTACYPGYVLNRSSDDTGTCIKECTGDFMAHCKADGCSLNVGGSKYCDQCEEGYAPVDGVCTSIPAAARDASGCKASGGKCTECGANYALLSGGCYNTQKLPGSSVCTAAQNKGQCQTCANGQSPAGRKCPACTEGCVKCAGSKETCTDCLAGYYKDAGDKCFKCTDSDKASSNAITGVENCISCAPPAGGNGPVTCYVTQQKADDGTGGDTGGDSTNRSGLSTGAIAGISVAVIVVGGLVGFLCWWFICRGKA

SEQ ID NO: 123 - protein, 1088 aa, Giardia
MLVGFLLVCVTVLAKRSGQNGSEKCNTPNCRDCTNPKAENEACTGCDPAYVLSGSQCVERKCNTPNCRDCTNPKAENEACTGCDPAYVLSGSQCVERKCNTPNCRDCTNPKAENEACTGCDPAYVLSGSQCVERKCNTPNCRDCTNPKAENEACTGCDPAYVLSGSQCVERKCNTPNCRDCTNPKAENEACTGCDPAYVLSGSQCVERKCNTPNCRDCTNPKAENEACTGCDPAYVLSGSQCVERKCNTPNCRDCTNPKAENEACTGCDPAYVLSGSQCVERKCNTPNCRDCTNPKAENEACTGCDPAYVLSGSQCVERKCNTPNCRDCTNPKAENEACTGCDPAYVLSGSQCVERKCNTPNCRDCTNPKAENEACTGCDPAYVLSGSQCVERKCNTPNCRDCTNPKAENEACTGCDPAYVLSGSQCVERKCNTPNCRDCTNPKAENEACTGCDPAYVLSGSQCVERKCNTPNCRDCTNPKAENEACTGCDPAYVLSGSQCVERKCNTPNCRDCTNPKAENEACTGCDPAYVLSGSQCVERKCNTPNCRDCTNPKAENEACTGCDPAYVLSGSQCVERKCNTPNCRDCTNPKAENEACTGCDPAYVLSGSQCVERKCNTPNCRDCTNPKAENEACTGCDPAYVLSGSQCVERKCNTPNCRDCTNPKAENEACTGCDPAYVLSGSQCVERKCNTPNCRDCTNPKAENEACTGCDPAYVLSGSQCVERKCNTPNCRDCTNPKAENEACTGCDPAYVLSGSQCVERKCNTPNCRDCTNPKAENEACTECNDGDYLTPTSQCVSDCTTLKGYYGDDSGKKTCKRCNDACAECKGEGADKCTACPAGKMLKYTDENSPSSGTCVDGCKPQSGASGCETCGATIGGTKYCSKCSTSTEVPVNGVCTADNARAAACKVKDGKGGCTTCASGYFRQDNGCYKTDRQPGIQICTLASQGDKCETCANSLQPSAAGVCPLCDSACKTCTSANDANTCSSCVVGYYQVGTKCVRCDTNDPNGNKPITGVKDCVSCAPPAGGDGGSVICYVKTDGTDNGGSVNKSGLSTGAIAGIAVAVIVIVGGLVGFLCWWFLCRGKA

SEQ ID NO: 124 - protein, 185 aa, Giardia
MTGSGQRSVSAPVILLPVTGEHQEAFSLHGLPCTADAMFAKLIFTSLVLQLAEAIRPAEKSRSDNACGDLGTAGCATCDSNSGNKICLTCTDPAKFIAVNKKSCKAACDANGGEIEAPVVGSTKACKCDEDNGYTLQGDACVIPNTNKSSGLSTGAIAGIAVAAVIVVGGLVGFLCWWFLCRGKA

SEQ ID NO: 125 - protein, 634 aa, Artificial Sequence
  VSP fused to VSV-G
MLLIAFYLILSTFAVDCKNSGNSCEAGQCDTIGDTEICMQCNQGKVPINGICTAHSEEAVTNAGCKKNGGTNIEESDKVCGQCGNGYFLHKGGCYKIGEAPGNLICADEASNPGARTAGVCGACKDGYYKNSDAVATADSCIACEDANCATCGGAGENKCTKCIDGYFVGATGNEGGCIKCDATTGPNSYKGVAGCAKCEKPKNAGPAKCIECAADYLKTEADEQTSCVSEAVCREGKTHFPTTDSAGGNKKVCVSCGTTNNGGIENCGECTSKESAARAGTEITCTKCSSNNLSPLGDACLTDCPAGTYAVSGDSGSVCKPCHNTCAGCQTDDRETSCTACYPGYSLLYESNGATGRCVKECTGAFITNCADGQCTANVGGAKYCTQCKDGYAPIDGICTAVAAAGRDVSVCTATGGKCTACTGNYALLSGGCYNTQTLPGKSVCKAVANSNDGKCKTCANGQAPDPATNFCPLCDSTCAECSTKNDADACTKCFPGYYKTGNKCIKCTESSNNGKKIDGIPDCLSCEAPINTGPVICYVKTDGTSDDNSGNGGDSTNKSGLSTGGSEQKLISEEDLSGGGGSKSSIASFFFIIGLIIGLFLVLRVGIHLCIKLKHTKKRQIYTDIEMNRLGK

SEQ ID NO: 126 - protein, 1275 aa, SARS-CoV-2
MVVFLVLLPLVSSQCVNLTTRTQLPPAYTNSFTRGVYYPDKVFRSSVLHSTQDLFLPFFSNVTWFHAIHVSGTNGTKRFDNPVLPFNDGVYFASTEKSNIIRGWIFGTTLDSKTQSLLIVNNATNVVIKVCEFQFCNDPFLGVYYHKNNKSWMESEFRVYSSANNCTFEYVSQPFLMDLEGKQGNFKNLREFVFKNIDGYFKIYSKHTPINLVRDLPQGFSALEPLVDLPIGINITRFQTLLALHRSYLTPGDSSSGWTAGAAAYYVGYLQPRTFLLKYNENGTITDAVDCALDPLSETKCTLKSFTVEKGIYQTSNFRVQPTESIVRFPNITNLCPFGEVFNATRFASVYAWNRKRISNCVADYSVLYNSASFSTFKCYGVSPTKLNDLCFTNVYADSFVIRGDEVRQIAPGQTGKIADYNYKLPDDFTGCVIAWNSNNLDSKVGGNYNYLYRLFRKSNLKPFERDISTEIYQAGSTPCNGVEGFNCYFPLQSYGFQPTNGVGYQPYRVVVLSFELLHAPATVCGPKKSTNLVKNKCVNFNFNGLTGTGVLTESNKKFLPFQQFGRDIADTTDAVRDPQTLEILDITPCSFGGVSVITPGTNTSNQVAVLYQDVNCTEVPVAIHADQLTPTWRVYSTGSNVFQTRAGCLIGAEHVNNSYECDIPIGAGICASYQTQTNSPRRARSVASQSIIAYTMSLGAENSVAYSNNSIAIPTNFTISVTTEILPVSMTKTSVDCTMYICGDSTECSNLLLQYGSFCTQLNRALTGIAVEQDKNTQEVFAQVKQIYKTPPIKDFGGFNFSQILPDPSKPSKRSFIEDLLFNKVTLADAGFIKQYGDCLGDIAARDLICAQKFNGLTVLPPLLTDEMIAQYTSALLAGTITSGWTFGAGAALQIPFAMQMAYRFNGIGVTQNVLYENQKLIANQFNSAIGKIQDSLSSTASALGKLQDVVNQNAQALNTLVKQLSSNFGAISSVLNDILSRLDKVEAEVQIDRLITGRLQSLQTYVTQQLIRAAEIRASANLAATKMSECVLGQSKRVDFCGKGYHLMSFPQSAPHGVVFLHVTYVPAQEKNFTTAPAICHDGKAHFPREGVFVSNGTHWFVTQRNFYEPQIITTDNTFVSGNCDVVIGIVNNTVYDPLQPELDSFKEELDKYFKNHTSPDVDLGDISGINASVVNIQKEIDRLNEVAKNLNESLIDLQELGKYEQGSYIKWPWYIWLGFIAGLIAIVMVTIMLCCMTSCCSCLKGCCSCGSCCKFDEDDSEPVLKGVKLHYT

SEQ ID NO: 127 - protein, 1275 aa, SARS-CoV-2
MVVFLVLLPLVSSQCVNLTTRTQLPPAYTNSFTRGVYYPDKVFRSSVLHSTQDLFLPFFSNVTWFHAIHVSGTNGTKRFDNPVLPFNDGVYFASTEKSNIIRGWIFGTTLDSKTQSLLIVNNATNVVIKVCEFQFCNDPFLGVYYHKNNKSWMESEFRVYSSANNCTFEYVSQPFLMDLEGKQGNFKNLREFVFKNIDGYFKIYSKHTPINLVRDLPQGFSALEPLVDLPIGINITRFQTLLALHRSYLTPGDSSSGWTAGAAAYYVGYLQPRTFLLKYNENGTITDAVDCALDPLSETKCTLKSFTVEKGIYQTSNFRVQPTESIVRFPNITNLCPFGEVFNATRFASVYAWNRKRISNCVADYSVLYNSASFSTFKCYGVSPTKLNDLCFTNVYADSFVIRGDEVRQIAPGQTGKIADYNYKLPDDFTGCVIAWNSNNLDSKVGGNYNYLYRLFRKSNLKPFERDISTEIYQAGSTPCNGVEGFNCYFPLQSYGFQPTNGVGYQPYRVVVLSFELLHAPATVCGPKKSTNLVKNKCVNFNFNGLTGTGVLTESNKKFLPFQQFGRDIADTTDAVRDPQTLEILDITPCSFGGVSVITPGTNTSNQVAVLYQGVNCTEVPVAIHADQLTPTWRVYSTGSNVFQTRAGCLIGAEHVNNSYECDIPIGAGICASYQTQTNSPRRARSVASQSIIAYTMSLGAENSVAYSNNSIAIPTNFTISVTTEILPVSMTKTSVDCTMYICGDSTECSNLLLQYGSFCTQLNRALTGIAVEQDKNTQEVFAQVKQIYKTPPIKDFGGFNFSQILPDPSKPSKRSFIEDLLFNKVTLADAGFIKQYGDCLGDIAARDLICAQKFNGLTVLPPLLTDEMIAQYTSALLAGTITSGWTFGAGAALQIPFAMQMAYRFNGIGVTQNVLYENQKLIANQFNSAIGKIQDSLSSTASALGKLQDVVNQNAQALNTLVKQLSSNFGAISSVLNDILSRLDKVEAEVQIDRLITGRLQSLQTYVTQQLIRAAEIRASANLAATKMSECVLGQSKRVDFCGKGYHLMSFPQSAPHGVVFLHVTYVPAQEKNFTTAPAICHDGKAHFPREGVFVSNGTHWFVTQRNFYEPQIITTDNTFVSGNCDVVIGIVNNTVYDPLQPELDSFKEELDKYFKNHTSPDVDLGDISGINASVVNIQKEIDRLNEVAKNLNESLIDLQELGKYEQGSYIKWPWYIWLGFIAGLIAIVMVTIMLCCMTSCCSCLKGCCSCGSCCKFDEDDSEPVLKGVKLHYT

SEQ ID NO: 128 - protein, 1275 aa, Artificial Sequence
  Artificial variant from SARS-CoV-2
MVVFLVLLPLVSSQCVNLTTRTQLPPAYTNSFTRGVYYPDKVFRSSVLHSTQDLFLPFFSNVTWFHAIHVSGTNGTKRFDNPVLPFNDGVYFASTEKSNIIRGWIFGTTLDSKTQSLLIVNNATNVVIKVCEFQFCNDPFLGVYYHKNNKSWMESEFRVYSSANNCTFEYVSQPFLMDLEGKQGNFKNLREFVFKNIDGYFKIYSKHTPINLVRDLPQGFSALEPLVDLPIGINITRFQTLLALHRSYLTPGDSSSGWTAGAAAYYVGYLQPRTFLLKYNENGTITDAVDCALDPLSETKCTLKSFTVEKGIYQTSNFRVQPTESIVRFPNITNLCPFGEVFNATRFASVYAWNRKRISNCVADYSVLYNSASFSTFKCYGVSPTKLNDLCFTNVYADSFVIRGDEVRQIAPGQTGKIADYNYKLPDDFTGCVIAWNSNNLDSKVGGNYNYLYRLFRKSNLKPFERDISTEIYQAGSTPCNGVEGFNCYFPLQSYGFQPTNGVGYQPYRVVVLSFELLHAPATVCGPKKSTNLVKNKCVNFNFNGLTGTGVLTESNKKFLPFQQFGRDIADTTDAVRDPQTLEILDITPCSFGGVSVITPGTNTSNQVAVLYQDVNCTEVPVAIHADQLTPTWRVYSTGSNVFQTRAGCLIGAEHVNNSYECDIPIGAGICASYQTQTNSPRRARSVASQSIIAYTMSLGAENSVAYSNNSIAIPTNFTISVTTEILPVSMTKTSVDCTMYICGDSTECSNLLLQYGSFCTQLNRALTGIAVEQDKNTQEVFAQVKQIYKTPPIKDFGGFNFSQILPDPSKPSKRSFIEDLLFNKVTLADAGFIKQYGDCLGDIAARDLICAQKFNGLTVLPPLLTDEMIAQYTSALLAGTITSGWTFGAGAALQIPFAMQMAYRFNGIGVTQNVLYENQKLIANQFNSAIGKIQDSLSSTASALGKLQDVVNQNAQALNTLVKQLSSNFGAISSVLNDILSRLDKVEAEVQIDRLITGRLQSLQTYVTQQLIRAAEIRASANLAATKMSECVLGQSKRVDFCGKGYHLMSFPQSAPHGVVFLHVTYVPAQEKNFTTAPAICHDGKAHFPREGVFVSNGTHWFVTQRNFYEPQIITTDNTFVSGNCDVVIGIVNNTVYDPLQPELDSFKEELDKYFKNHTSPDVDLGDISGINASVVNIQKEIDRLNEVAKNLNESLIDLQELGKYEQGSYIKWPWYIWLGFIAGLIAIVMVTIMLCCMTSCCSCLKGCCSCGSCCKFDEDDSEPVLKGVALAYT

SEQ ID NO: 129 - protein, 1275 aa, Artificial Sequence
  Artificial variant from SARS-CoV-2
MVVFLVLLPLVSSQCVNLTTRTQLPPAYTNSFTRGVYYPDKVFRSSVLHSTQDLFLPFFSNVTWFHAIHVSGTNGTKRFDNPVLPFNDGVYFASTEKSNIIRGWIFGTTLDSKTQSLLIVNNATNVVIKVCEFQFCNDPFLGVYYHKNNKSWMESEFRVYSSANNCTFEYVSQPFLMDLEGKQGNFKNLREFVFKNIDGYFKIYSKHTPINLVRDLPQGFSALEPLVDLPIGINITRFQTLLALHRSYLTPGDSSSGWTAGAAAYYVGYLQPRTFLLKYNENGTITDAVDCALDPLSETKCTLKSFTVEKGIYQTSNFRVQPTESIVRFPNITNLCPFGEVFNATRFASVYAWNRKRISNCVADYSVLYNSASFSTFKCYGVSPTKLNDLCFTNVYADSFVIRGDEVRQIAPGQTGKIADYNYKLPDDFTGCVIAWNSNNLDSKVGGNYNYLYRLFRKSNLKPFERDISTEIYQAGSTPCNGVEGFNCYFPLQSYGFQPTNGVGYQPYRVVVLSFELLHAPATVCGPKKSTNLVKNKCVNFNFNGLTGTGVLTESNKKFLPFQQFGRDIADTTDAVRDPQTLEILDITPCSFGGVSVITPGTNTSNQVAVLYQGVNCTEVPVAIHADQLTPTWRVYSTGSNVFQTRAGCLIGAEHVNNSYECDIPIGAGICASYQTQTNSPRRARSVASQSIIAYTMSLGAENSVAYSNNSIAIPTNFTISVTTEILPVSMTKTSVDCTMYICGDSTECSNLLLQYGSFCTQLNRALTGIAVEQDKNTQEVFAQVKQIYKTPPIKDFGGFNFSQILPDPSKPSKRSFIEDLLFNKVTLADAGFIKQYGDCLGDIAARDLICAQKFNGLTVLPPLLTDEMIAQYTSALLAGTITSGWTFGAGAALQIPFAMQMAYRFNGIGVTQNVLYENQKLIANQFNSAIGKIQDSLSSTASALGKLQDVVNQNAQALNTLVKQLSSNFGAISSVLNDILSRLDKVEAEVQIDRLITGRLQSLQTYVTQQLIRAAEIRASANLAATKMSECVLGQSKRVDFCGKGYHLMSFPQSAPHGVVFLHVTYVPAQEKNFTTAPAICHDGKAHFPREGVFVSNGTHWFVTQRNFYEPQIITTDNTFVSGNCDVVIGIVNNTVYDPLQPELDSFKEELDKYFKNHTSPDVDLGDISGINASVVNIQKEIDRLNEVAKNLNESLIDLQELGKYEQGSYIKWPWYIWLGFIAGLIAIVMVTIMLCCMTSCCSCLKGCCSCGSCCKFDEDDSEPVLKGVALAYT

SEQ ID NO: 130 - protein, 1276 aa, Artificial Sequence
  Artificial variant from SARS-CoV-2
MVVFLVLLPLVSSQCVNLTTRTQLPPAYTNSFTRGVYYPDKVFRSSVLHSTQDLFLPFFSNVTWFHAIHVSGTNGTKRFDNPVLPFNDGVYFASTEKSNIIRGWIFGTTLDSKTQSLLIVNNATNVVIKVCEFQFCNDPFLGVYYHKNNKSWMESEFRVYSSANNCTFEYVSQPFLMDLEGKQGNFKNLREFVFKNIDGYFKIYSKHTPINLVRDLPQGFSALEPLVDLPIGINITRFQTLLALHRSYLTPGDSSSGWTAGAAAYYVGYLQPRTFLLKYNENGTITDAVDCALDPLSETKCTLKSFTVEKGIYQTSNFRVQPTESIVRFPNITNLCPFGEVFNATRFASVYAWNRKRISNCVADYSVLYNSASFSTFKCYGVSPTKLNDLCFTNVYADSFVIRGDEVRQIAPGQTGKIADYNYKLPDDFTGCVIAWNSNNLDSKVGGNYNYLYRLFRKSNLKPFERDISTEIYQAGSTPCNGVEGFNCYFPLQSYGFQPTNGVGYQPYRVVVLSFELLHAPATVCGPKKSTNLVKNKCVNFNFNGLTGTGVLTESNKKFLPFQQFGRDIADTTDAVRDPQTLEILDITPCSFGGVSVITPGTNTSNQVAVLYQDVNCTEVPVAIHADQLTPTWRVYSTGSNVFQTRAGCLIGAEHVNNSYECDIPIGAGICASYQTQTNSPGSASSVASQSIIAYTMSLGAENSVAYSNNSIAIPTNFTISVTTEILPVSMTKTSVDCTMYICGDSTECSNLLLQYGSFCTQLNRALTGIAVEQDKNTQEVFAQVKQIYKTPPIKDFGGFNFSQILPDPSKPSKRSFIEDLLFNKVTLADAGFIKQYGDCLGDIAARDLICAQKFNGLTVLPPLLTDEMIAQYTSALLAGTITSGWTFGAGAALQIPFAMQMAYRFNGIGVTQNVLYENQKLIANQFNSAIGKIQDSLSSTASALGKLQDVVNQNAQALNTLVKQLSSNFGAISSVLNDILSRLDPPEAEVQIDRLITGRLQSLQTYVTQQLIRAAEIRASANLAATKMSECVLGQSKRVDFCGKGYHLMSFPQSAPHGVVFLHVTYVPAQEKNFTTAPAICHDGKAHFPREGVFVSNGTHWFVTQRNFYEPQIITTDNTFVSGNCDVVIGIVNNTVYDPLQPELDSFKEELDKYFKNHTSPDVDLGDISGINASVVNIQKEIDRLNEVAKNLNESLIDLQELGKYEQEGSYIKWPWYIWLGFIAGLIAIVMVTIMLCCMTSCCSCLKGCCSCGSCCKFDEDDSEPVLKGVALAYT

SEQ ID NO: 131 - protein, 1276 aa, Artificial Sequence
  Artificial variant from SARS-CoV-2
MVVFLVLLPLVSSQCVNLTTRTQLPPAYTNSFTRGVYYPDKVFRSSVLHSTQDLFLPFFSNVTWFHAIHVSGTNGTKRFDNPVLPFNDGVYFASTEKSNIIRGWIFGTTLDSKTQSLLIVNNATNVVIKVCEFQFCNDPFLGVYYHKNNKSWMESEFRVYSSANNCTFEYVSQPFLMDLEGKQGNFKNLREFVFKNIDGYFKIYSKHTPINLVRDLPQGFSALEPLVDLPIGINITRFQTLLALHRSYLTPGDSSSGWTAGAAAYYVGYLQPRTFLLKYNENGTITDAVDCALDPLSETKCTLKSFTVEKGIYQTSNFRVQPTESIVRFPNITNLCPFGEVFNATRFASVYAWNRKRISNCVADYSVLYNSASFSTFKCYGVSPTKLNDLCFTNVYADSFVIRGDEVRQIAPGQTGKIADYNYKLPDDFTGCVIAWNSNNLDSKVGGNYNYLYRLFRKSNLKPFERDISTEIYQAGSTPCNGVEGFNCYFPLQSYGFQPTNGVGYQPYRVVVLSFELLHAPATVCGPKKSTNLVKNKCVNFNFNGLTGTGVLTESNKKFLPFQQFGRDIADTTDAVRDPQTLEILDITPCSFGGVSVITPGTNTSNQVAVLYQGVNCTEVPVAIHADQLTPTWRVYSTGSNVFQTRAGCLIGAEHVNNSYECDIPIGAGICASYQTQTNSPGSASSVASQSIIAYTMSLGAENSVAYSNNSIAIPTNFTISVTTEILPVSMTKTSVDCTMYICGDSTECSNLLLQYGSFCTQLNRALTGIAVEQDKNTQEVFAQVKQIYKTPPIKDFGGFNFSQILPDPSKPSKRSFIEDLLFNKVTLADAGFIKQYGDCLGDIAARDLICAQKFNGLTVLPPLLTDEMIAQYTSALLAGTITSGWTFGAGAALQIPFAMQMAYRFNGIGVTQNVLYENQKLIANQFNSAIGKIQDSLSSTASALGKLQDVVNQNAQALNTLVKQLSSNFGAISSVLNDILSRLDPPEAEVQIDRLITGRLQSLQTYVTQQLIRAAEIRASANLAATKMSECVLGQSKRVDFCGKGYHLMSFPQSAPHGVVFLHVTYVPAQEKNFTTAPAICHDGKAHFPREGVFVSNGTHWFVTQRNFYEPQIITTDNTFVSGNCDVVIGIVNNTVYDPLQPELDSFKEELDKYFKNHTSPDVDLGDISGINASVVNIQKEIDRLNEVAKNLNESLIDLQELGKYEQEGSYIKWPWYIWLGFIAGLIAIVMVTIMLCCMTSCCSCLKGCCSCGSCCKFDEDDSEPVLKGVALAYT

SEQ ID NO: 132 - protein, 419 aa, SARS-CoV-2
MSDNGPQNQRNAPRITFGGPSDSTGSNQNGERSGARSKQRRPQGLPNNTASWFTALTQHGKEDLKFPRGQGVPINTNSSPDDQIGYYRRATRRIRGGDGKMKDLSPRWYFYYLGTGPEAGLPYGANKDGIIWVATEGALNTPKDHIGTRNPANNAAIVLQLPQGTTLPKGFYAEGSRGGSQASSRSSSRSRNSSRNSTPGSSRGTSPARMAGNGGDAALALLLLDRLNQLESKMSGKGQQQQGQTVTKKSAAEASKKPRQKRTATKAYNVTQAFGRRGPEQTQGNFGDQELIRQGTDYKHWPQIAQFAPSASAFFGMSRIGMEVTPSGTWLTYTGAIKLDDKDPNFKDQVILLNKHIDAYKTFPPTEPKKDKKKKADETQALPQRQKKQQTVTLLPAADLDDFSKQLQQSMSSADSTQA

SEQ ID NO: 133 - protein, 222 aa, SARS-CoV-2
MADSNGTITVEELKKLLEQWNLVIGFLFLTWICLLQFAYANRNRFLYIIKLIFLWLLWPVTLACFVLAAVYRINWITGGIAIAMACLVGLMWLSYFIASFRLFARTRSMWSFNPETNILLNVPLHGTILTRPLLESELVIGAVILRGHLRIAGHHLGRCDIKDLPKEITVATSRTLSYYKLGASQRVAGDSGFAAYSRYRIGNYKLNTDHSSSSDNIALLVQ